European Patent Application EP 4 807 006 A2, published September 16, 2026. Title: Synthetic Gene Clusters. Applicant: The Regents of the University of California. The sequence listing filed with the application follows.

SEQUENCE LISTING (345 sequences)

SEQ ID NO: 1 - DNA, 3504 bp, Klebsiella pneumoniae
  misc_feature 1..3504: note = wild type Gene J, nifJ
  source 1..3504: mol_type = genomic DNA
atgaaaacaatggatggcaacgccgcggcggcctggatctcttatgcctttaccgaggtcgcggcgatttaccccataaccccctccacgccgatggcggaaaacgtcgacgagtgggcggcgcaggggaaaaagaacctttttggccagccggtgcgcttaatggagatgcagtcggaggccggcgcggcaggcgcggtccacggcgcgctgcaggccggggcgctcaccaccacctatacggcctcccaggggctgctgctgatgatccccaacatgtacaaaatcgccggtgaactgctgccgggcgtctttcacgtcagcgcccgggcgctggcgaccaattcgctgaatatttttggcgatcaccaggatgtgatggcggtccgccagaccggctgcgcgatgctggcggagaacaacgtgcagcaggtgatggatttgtcggcggtggcgcatctggcggcgattaagggacgcatcccgtttgttaacttcttcgacggttttcgcacctcgcacgaaattcaaaaaatcgaggtgttggaatatgagcagctggcgacgctgctggaccggcccgcgctcgacagcttccgccgtaacgcgctgcatccggatcatccggtcatccgcggaacggcgcagaacccggatatctacttccaggagcgggaggcgggcaaccgtttttatcaggcgctgcccgacattgtcgaaagctatatgacgcaaatcagcgcgctcaccggccgggagtatcatctgtttaactataccggcgcggcggatgccgaacgggtgattatcgcaatgggatcggtctgcgataccgttcaggaagtggtggatacgctgaacgcggcgggagagaaggtcgggctgctcagcgtgcatctgtttcgccctttttcgctggcccacttcttcgcccagctgccgaaaaccgtgcagcggattgccgtccttgaccgtaccaaagagcccggcgctcaggctgaaccgctgtgcctggatgtgaaaaacgccttctaccaccacgacgatgcgccgctaatcgtcggcggccgctatgcgcttggcgggaaggatgttctgcccaacgatatcgcggccgtctttgataacctcaataaaccgctgccgatggacgggtttaccctcgggattgtcgatgatgtaacctttacttcgttaccgccggcccagcagacgctggcggtctcgcatgacggcatcaccgcctgtaaattttggggcatgggctcggacggcaccgtcggggccaataaaagcgcgatcaaaattatcggcgataaaacgccgctctacgcgcaggcctacttttcttatgactcgaaaaaatccggcggcattaccgtttcacatttacgcttcggcgaccggccgatcaattcgccctacctgatccatcgggccgattttatctcctgttcgcagcagtcctacgttgagcgctacgatctgctggacggattaaagccgggcgggacctttttactcaactgcagctggtccgatgcggagctggagcagcatctgccggtcggctttaaacgctatctggcgcgggaaaatatccatttttataccctgaacgccgtggatatcgcccgcgagctcgggctgggcgggcgctttaatatgctgatgcaggcggcgttctttaagctggcggcgattatcgacccgcagaccgcggcggattacctcaagcaggcggttgaaaaaagctacggcagcaaaggggcggcggtgattgagatgaaccagcgggcgatcgagctgggcatggcctcgctgcatcaggtgacgattccggcgcactgggcgacgctggatgaacccgcggcgcaagcatcagccatgatgccggatttcatccgcgatattctgcagccgatgaaccgccagtgcggcgaccagctgccggtgagcgcgttcgtcggtatggaggacgggacctttccttcgggcaccgccgcgtgggagaaacgcgggatcgcgctggaagtgccggtctggcagccggagggctgcacgcagtgtaaccagtgcgcctttatctgcccgcatgcggcgatccgcccggcgctgctcaacggcgaagagcatgacgccgcgccggttgggctgctgagcaaacccgcgcagggagcgaaggagtatcactaccatctggctatctcgccgctggattgttccggctgcggcaactgcgtggatatctgtcccgcgcgcggcaaggcgttaaaaatgcagtctctcgatagccagcgtcagatggcgccggtctgggactatgcgctggcgctgacgccgaagagcaatccgtttcgtaagacgacggtcaaaggcagccagtttgaaaccccgctgctggagttttccggcgcctgcgcgggatgcggtgaaacgccttatgcccgcctgataacccagctgtttggcgaccggatgctgatcgctaacgccaccggctgctcttctatctggggagccagcgcgccgtcgattccctataccaccaaccaccgcggccatggcccggcatgggcgaactcgctgtttgaggataatgcggagtttggcctcggcatgatgctcggcggccaggcggtgcgtcaacaaatcgccgatgatatgaccgccgcgctggcgctaccggtcagcgacgaacttagcgacgcaatgcgccagtggctggcgaagcaggatgaaggcgagggcacccgcgagcgcgcggaccggctcagcgaacggctggcggcggaaaaagagggcgtgccgctgttggagcagctgtggcagaaccgcgactattttgttcgtcgttcgcagtggattttcggcggcgacggctgggcctacgatatcggcttcggcggtctcgatcacgtgctggcgagcggggaagacgtcaatattctggtgtttgacaccgaggtttactccaataccggcggccagtcgtctaaatcgaccccggtggcggccatcgcgaagtttgccgcgcagggcaaacgcacgcggaaaaaagatctcggcatgatggcgatgagctacggcaatgtgtacgtggcccaggtcgcgatgggcgctgataaagatcagaccctacgggcgatcgccgaggccgaagcctggccgggaccgtcgctggtgattgcctacgccgcctgcattaaccacgggctgaaagccggtatgcgctgcagccagcgcgaggcgaaacgggcggttgaggcgggatactggcacctgtggcgctatcatccgcagcgggaagcggaaggtaagacgccgtttatgctcgattccgaagagccggaggagagcttccgcgactttttgcttggcgaagtgcgctacgcctcgctgcacaaaacgacgccgcatctggcggatgcgctctttagccgaaccgaggaggacgcgcgggcccgctttgcccagtatcggcggctggccggcgaggagtag

SEQ ID NO: 2 - DNA, 3504 bp, synthetic construct
  misc_feature 1..3504: note = synthetic Gene J
  source 1..3504: mol_type = other DNA
atgaaaactatggacggtaacgctgcggctgcatggattagctacgcctttaccgaagtggctgcgatctacccgattacgccgagcaccccgatggcggaaaatgtggacgaatgggctgcgcagggcaagaagaacctcttcggccagccggtgcgcctgatggagatgcagtcggaagcgggtgcagcaggtgctgtgcatggcgccttgcaagctggcgcactgacgaccacctacaccgcgtcgcagggcctgttgctgatgatcccaaacatgtacaaaatcgcgggtgaactgctgccgggtgtctttcatgtttcggcacgcgcactggccaccaatagcctcaacatctttggcgatcatcaggatgtaatggcggtgcgccaaacgggctgcgcgatgttggccgagaataacgtccagcaagttatggatttgtccgcggtagcccacttggcagcgatcaaaggtcgcattccgttcgtgaacttcttcgatggctttcgcaccagccacgaaatccagaagatcgaggttctggaatatgaacagctggccaccttgttggatcgtccggccctggacagcttccgccgtaacgcccttcacccggaccacccggtcatccgtggcaccgcccagaacccggacatctacttccaggaacgtgaggccggtaaccgtttctatcaggcgctcccggatattgtggaatcttacatgacccagatttctgccctgactggtcgcgagtatcacctgtttaactacactggtgctgcggatgcggagcgcgtgatcatcgcgatgggctctgtctgtgacaccgtccaagaggtggttgacacgctgaatgcagcgggtgagaaagttggtctgctctccgttcatcttttccgcccgttttcgttagcgcacttcttcgcccaactgccgaaaactgtacagcgtatcgcagtattggaccgtacgaaagagccaggtgctcaagcagagccgctgtgcctcgatgtgaagaatgccttttaccaccatgacgatgccccgttgattgtgggtggtcgctatgccttgggcggtaaggacgtgttgccgaacgatattgcggccgtgtttgataacctgaacaaaccgctgccgatggacggcttcacgctgggtatcgtggacgatgttaccttcacctctctcccgccagcgcagcagaccctggcggtttctcacgacggcatcacggcatgtaagttttggggcatgggctccgacggcacggttggtgcgaacaagtccgcgatcaagattatcggcgacaaaacgccactgtatgcgcaagcgtacttttcctacgactcgaagaagagcggtggtattaccgtcagccatctgcgttttggtgatcgcccgatcaactccccgtatttgatccatcgcgcggatttcatctcgtgcagccagcaaagctatgttgaacgctacgatctgctggatggccttaaaccgggtggcacctttctgctgaactgctcctggagcgatgccgaactggagcaacatctgccggtcggtttcaaacgttatctggcacgcgagaatatccacttctacactctcaacgctgtggacatcgcccgtgagcttggtttgggtggccgtttcaacatgctgatgcaggctgccttcttcaaactggccgcgatcattgacccgcagactgctgcggactatctgaagcaggctgttgagaaaagctatggcagcaaaggtgcggcggtcatcgagatgaaccagcgtgccatcgagcttggcatggccagcctgcaccaggtgacgatcccggcacattgggccaccctggatgagccagcggcgcaggcgtccgcgatgatgccggactttatccgcgacatcctgcaaccgatgaaccgtcagtgcggcgaccagcttccggtgtcggcttttgtcggcatggaagatggcaccttcccgtccggcacggccgcatgggagaaacgtggcatcgcccttgaggtgccagtctggcagccggaaggctgcacgcagtgcaaccagtgcgccttcatttgtccgcacgccgcgattcgtccggcgttgttgaatggcgaagagcatgatgctgccccggttggcctgctgagcaaaccggcacaaggcgctaaagaatatcactatcatctggcgattagcccgctggactgctccggctgtggcaactgcgttgacatttgtccagctcgtggcaaagcgttgaagatgcagtctctggatagccaacgccagatggctccggtgtgggattatgcgctggcgctgaccccgaagtctaacccgtttcgtaaaaccaccgtcaaaggctcgcagttcgaaaccccgctgctggagtttagcggtgcgtgcgctggttgtggcgaaacgccgtatgcgcgcctcattacccagctgtttggcgaccgcatgctgattgccaatgccaccggctgttccagcatctggggcgcatctgcgccgagcatcccgtataccaccaatcatcgtggtcatggtccggcctgggcgaatagcctgtttgaggacaatgccgaatttggtttaggtatgatgctgggcggtcaagctgtgcgtcaacagatcgcggacgatatgacggctgcgttagcgctcccggtttccgatgagctgagcgacgcgatgcgccagtggttggcgaaacaggacgagggtgaaggcacgcgtgagcgtgcggaccgtctgagcgagcgcttagccgcggagaaagagggcgttccgctgttagagcagctgtggcaaaatcgtgattactttgtgcgtcgcagccagtggattttcggcggtgacggctgggcctatgatattggcttcggtggcctggaccacgtcctcgccagcggtgaggatgtgaacattctggtatttgacaccgaagtctactcgaacaccggcggtcaaagcagcaaatcgaccccggtcgcggccatcgccaagttcgcggctcagggcaagcgcacccgcaagaaagacctgggtatgatggcgatgagctacggcaacgtctatgtagcccaggtggcgatgggtgcggataaagatcaaactctgcgcgccattgcggaagctgaagcgtggccaggcccgtcgctggtgattgcgtatgcggcctgcatcaatcatggcctgaaggccggtatgcgttgcagccaacgtgaggcgaagcgcgctgttgaggcgggctactggcacctgtggcgttatcacccgcagcgcgaagcggaaggcaagacgccgtttatgttagatagcgaagaaccggaagagtcgttccgtgactttctgttgggtgaggtgcgctacgcatccctgcacaagaccaccccgcacctcgccgatgcccttttcagccgtaccgaagaagatgcgcgtgcgcgctttgcgcaataccgtcgcctggctggcgaagagtaa

SEQ ID NO: 3 - DNA, 882 bp, Klebsiella pneumoniae
  misc_feature 1..882: note = wild type Gene H, nifH
  source 1..882: mol_type = genomic DNA
atgaccatgcgtcaatgcgctatttacggtaaaggcggtatcggtaaatccaccaccacgcagaacctcgtcgccgcgctggcggagatgggtaagaaagtgatgatcgtcggctgcgatccgaaggcggactccacccgtctgattctgcacgccaaagcacagaacaccattatggagatggccgcggaagtcggctcggtcgaggacctcgaactcgaagacgtgctgcaaattggctacggcgatgtgcgctgcgcggaatccggcggcccggagccaggcgtcggctgcgcgggacgcggcgtgatcacggcgatcaactttcttgaagaagaaggcgcctacgaggacgatctcgatttcgtgttctatgacgtgctcggcgacgtggtctgcggcggcttcgccatgccgatccgcgaaaacaaagcccaggagatctacatcgtctgctccggcgaaatgatggcgatgtacgcggccaacaatatctccaaagggatcgttaaatacgccaaatccggcaaggtgcgcctcggcggcctgatctgtaactcacgtcagaccgaccgtgaagacgaactgattattgccctggcggaaaagctcggtacccagatgatccactttgtgccccgcgacaacatcgtgcagcgcgcggagatccgccgcatgacggttatcgagtacgaccccgcctgtaaacaggccaacgaataccgcaccctggcgcagaagatcgtcaacaacaccatgaaagtggtgccgacgccctgcaccatggatgagctggaatcgctgctgatggagttcggcatcatggaagaggaagacaccagcatcattggcaaaaccgccgccgaagaaaacgcggcctga

SEQ ID NO: 4 - DNA, 882 bp, synthetic construct
  misc_feature 1..882: note = synthetic Gene H
  source 1..882: mol_type = other DNA
atgaccatgcgtcagtgcgcgatttatggcaaaggtggtattggcaaaagcacgacgacccagaacttggtggcggccctggccgagatgggtaaaaaggttatgattgtgggttgcgacccgaaggccgacagcacgcgcctgattctgcacgcgaaagcacaaaacacgattatggagatggctgccgaggttggtagcgtggaggatctggagctggaggacgttctgcaaattggttacggtgatgttcgttgcgcagagagcggtggtccggaaccaggtgtcggctgtgcgggtcgtggtgtgattaccgctatcaatttcctggaagaagagggtgcgtacgaagatgatctggatttcgttttctacgatgtgctgggtgatgtcgtgtgcggtggttttgcaatgccgattcgcgagaataaggcacaagaaatttacattgtctgtagcggcgagatgatggcaatgtacgctgctaacaacatcagcaagggtattgttaaatacgcaaaaagcggtaaggttcgcttgggtggtttgatttgcaacagccgtcagaccgaccgtgaggacgaactgatcatcgccctggctgagaaactgggcacccaaatgatccacttcgtgccacgcgataatattgttcaacgtgcagaaatccgccgtatgaccgtcattgagtatgacccggcatgcaagcaagcgaacgagtaccgcaccttggcacagaaaatcgtgaacaacaccatgaaggttgttccgacgccgtgtacgatggacgagctggagagcctgctgatggagttcggcattatggaggaggaggacaccagcattatcggtaagaccgcagcggaggagaatgcggcataa

SEQ ID NO: 5 - DNA, 1452 bp, Klebsiella pneumoniae
  misc_feature 1..1452: note = wild type Gene D, nifD
  source 1..1452: mol_type = genomic DNA
atgatgaccaacgcaacgggcgaacgtaatctggcgctgatccaggaagtcctggaggtgttcccggaaaccgcgcgaaaagagcgcagaaagcacatgatggtcagcgatccgaaaatgaagagcgtcggcaagtgcattatctctaaccgcaaatcacaacccggcgtaatgaccgtacgcggctgcgcctacgccggttccaaaggggtggtatttgggccgattaaggatatggcccatatttcgcacggaccggctggctgcggccagtattcccgcgccgaacgacgcaactactacaccggagtcagcggcgtcgatagcttcggcacgctgaacttcacctctgattttcaggagcgcgacatcgtcttcggcggcgataaaaagctcagcaagctgattgaagagatggagttgctgttcccgctcaccaaagggatcaccattcagtcggaatgcccggtggggctgatcggtgatgatatcagcgcggtggccaacgccagcagcaaggcgctggataaaccggtgatcccggtacgctgcgaaggctttcgcggcgtgtcgcagtctctggggcaccatatcgccaacgacgtggtgcgcgactggatcctgaacaatcgcgaaggacagccgtttgaaaccaccccttacgatgtggcgatcatcggcgactacaacatcggcggcgacgcctgggcctcgcgcattctgctggaagagatggggctacgggtagtcgcgcagtggtccggcgacggcacgctggtggagatggagaataccccattcgtcaagctgaacctggttcactgctaccgttcgatgaactatatcgcccgccatatggaggagaaacatcagattccgtggatggagtacaacttcttcgggccgaccaaaatcgccgaatcgctgcgcaaaatcgccgaccagttcgacgataccattcgcgcgaacgccgaagcggtgatcgcccggtatgaggggcagatggcggcgattatcgccaaatatcgcccgcgcctggaggggcgtaaggtgctgctctatatcggaggcctgcggccgcgccacgttattggcgcctatgaggatctcgggatggagatcatcgccgccggctacgagtttgcccataacgatgattacgaccgcaccctgccggatctgaaagagggcacgctgctgttcgatgacgccagcagctacgagctggaagcgttcgtcaaggcgctgaagcccgaccttatcggctccggcatcaaggaaaaatatatcttccagaaaatgggcgtgccgttccgccagatgcactcgtgggactattccggcccgtaccacggctacgatggtttcgccattttcgcccgcgatatggatatgaccctgaacaacccggcgtggaacgaactgaccgctccgtggctgaagtctgcgtga

SEQ ID NO: 6 - DNA, 1452 bp, synthetic construct
  misc_feature 1..1452: note = synthetic Gene D
  source 1..1452: mol_type = other DNA
atgatgactaatgctactggcgaacgtaacctggcactgattcaagaagtactggaagtgttcccggaaaccgcgcgcaaagagcgccgtaaacacatgatggtttctgacccgaaaatgaaatctgtgggtaaatgcatcatctctaatcgcaaatctcagccgggtgtcatgactgttcgtggctgtgcgtacgcaggttctaaaggtgtcgtattcggcccgatcaaagatatggcgcatatctctcatggcccggcaggctgtggccagtactctcgcgcggaacgtcgtaactactacacgggcgtttctggcgttgactctttcggcacgctgaacttcacctctgacttccaggaacgtgacatcgttttcggtggcgataaaaagctgtccaaactgatcgaagaaatggaactgctgttcccgctgactaaaggcattactatccaaagcgaatgtccggtgggtctgatcggtgatgacatcagcgcggtcgcaaacgcatcttccaaagccctggataagccggtgatcccggttcgttgcgagggcttccgcggcgtttctcagtctctgggtcatcacatcgcaaacgatgttgtgcgtgactggattctgaacaaccgtgaaggtcagccttttgaaaccaccccttatgacgttgcgattattggcgactataacatcggcggcgacgcctgggcatcccgcatcctgctggaggagatgggtctgcgtgttgtcgcacagtggtctggcgatggcaccctggttgaaatggaaaacaccccgtttgttaaactgaacctggttcactgctaccgctccatgaactacattgcccgtcacatggaagaaaaacatcagatcccttggatggaatacaacttcttcggtccgactaaaatcgcagaatccctgcgtaaaatcgccgatcagtttgatgataccattcgcgcgaacgctgaagcagtaattgcgcgctacgaaggccagatggcagcaatcattgctaagtaccgtccgcgcctggaaggtcgtaaagtgctgctgtacatgggtggtctgcgtccacgtcatgtgatcggtgcctacgaggacctgggcatggagatcatcgcagcgggttacgaatttgcacacaacgacgactatgatcgtacgctgccagacctgaaagaaggtacgctgctgtttgacgacgccagctcttatgaactggaagccttcgtgaaagcgctgaaaccagacctgatcggctccggcatcaaggaaaaatacattttccagaaaatgggcgtgccgttccgccagatgcactcctgggactactccggtccgtaccacggctacgacggtttcgctatcttcgctcgtgacatggatatgaccctgaataacccagcgtggaatgaactgaccgcaccgtggctgaaatctgcataa

SEQ ID NO: 7 - DNA, 1563 bp, Klebsiella pneumoniae
  misc_feature 1..1563: note = wild type Gene K, nifK
  source 1..1563: mol_type = genomic DNA
atgagccaaacgattgataaaattaatagctgttatccgctattcgaacaggatgaataccaggagctgttccgcaataagcggcagctggaagaggcgcacgatgcgcagcgcgtgcaggaggtctttgcctggaccaccaccgccgagtatgaagcgctgaatttccgacgcgaggcgctgaccgttgacccggcgaaagcctgccagccgcttggcgcggtgctttgctcgctgggatttgccaacaccctgccgtatgtgcacggctctcaggggtgcgtggcctactttcgcacctattttaaccgccatttcaaagagccgatcgcctgcgtctccgactcgatgaccgaagacgcggcggtcttcggcggcaacaacaatatgaacctgggcctgcagaacgccagcgcgctgtacaaaccggagatcattgcggtgtccaccacctgcatggcggaagttatcggcgatgacctgcaggcgtttatcgccaacgctaaaaaagatggcttcgtcgacagcagcatcgccgtgccccacgcccatacgccaagctttatcggcagccacgtcaccggctgggataacatgtttgaaggcttcgccaaaaccttcactgcggactaccaggggcagccgggcaaattgccgaagctcaatctggtgaccggctttgaaacctatctcggcaacttccgcgtattaaagcggatgatggaacagatggcggtgccgtgcagcctgctctccgatccgtcggaagttctcgacacgcccgccgacggtcactatcggatgtattccggcggcaccacgcagcaggagatgaaagaggcccctgacgccatcgatacgctgctcctgcagccgtggcagctgctgaagagcaaaaaagtggtgcaggagatgtggaaccagcccgccaccgaggtcgccattccgctggggctggccgccaccgatgaactgctgatgaccgtcagccagcttagcggcaagccgattgccgacgccctcacccttgagcgcggccggctggttgacatgatgctcgactcccacacctggctgcacggcaagaagtttggcctgtacggcgatccggacttcgtgatgggcctcacccgcttcctgctggagctgggctgcgagccaacggtgatcctgagccataacgccaacaaacgctggcaaaaagcgatgaacaaaatgctcgatgcctcgccgtacgggcgcgatagcgaagtgtttatcaactgcgatttgtggcacttccgttcgctgatgttcacccgtcagccggactttatgatcggcaactcctacggcaagtttatccagcgcgataccctggcgaagggtaaagcctttgaagtgccgcttatccgcctcggctttccgctgttcgaccgccaccatctgcaccgccagacaacctggggttatgaaggggcgatgaacattgtgacgacgctggtgaacgccgtgctggagaaactggatagcgataccagccagctgggcaaaaccgattacagcttcgatctcgtccgttaa

SEQ ID NO: 8 - DNA, 1563 bp, synthetic construct
  misc_feature 1..1563: note = synthetic Gene K
  source 1..1563: mol_type = other DNA
atgtctcaaactatcgataaaatcaactcttgttacccgctgttcgagcaggacgaatatcaggaactgttccgtaacaaacgtcagctggaagaagcgcacgacgcacagcgcgtgcaggaagtgttcgcatggaccaccaccgcggaatacgaagctctgaacttccgtcgcgaagccctgacggttgatccggcgaaagcgtgccagcctctgggtgcggttctgtgcagcctgggttttgccaacaccctgccgtatgtccacggttcccagggctgcgtagcctacttccgtacctatttcaaccgccactttaaagaaccaatcgcgtgcgtgtccgacagcatgacggaggacgcggcagttttcggtggtaacaacaacatgaacctgggcctgcaaaatgcttccgcactgtacaaaccggaaatcatcgcagtgtctaccacctgcatggcagaggttattggtgatgatctgcaagcatttattgccaacgcaaagaaagacggtttcgttgacagctctatcgcggttccgcacgctcataccccgtccttcatcggttctcacgtaactggttgggacaacatgttcgaaggcttcgcaaaaacttttaccgcagactatcaaggccaaccgggtaaactgccgaagctgaacctggtgaccggctttgaaacctacctgggcaactttcgtgtcctgaagcgcatgatggagcagatggcggttccgtgttctctgctgtctgacccgtctgaggttctggacactccagcggacggccactatcgcatgtattctggtggcaccactcagcaggaaatgaaagaggccccagacgcgattgacaccctgctgctgcaaccgtggcagctgctgaaaagcaagaaagttgttcaggaaatgtggaaccagccggcaacggaagttgcaatcccgctgggtctggcagctactgacgaactgctgatgaccgtgtcccaactgagcggcaaaccaatcgcggatgctctgaccctggaacgcggtcgcctggtggacatgatgctggacagccacacgtggctgcatggcaagaaatttggcctgtacggtgacccggacttcgtaatgggcctgacccgtttcctgctggaactgggctgcgagccgactgttatcctgtctcacaacgctaacaaacgttggcagaaggccatgaacaaaatgctggatgcgagcccatacggccgtgatagcgaagtgttcatcaactgcgacctgtggcatttccgctctctgatgtttacgcgtcagccggatttcatgatcggtaactcttacggcaaattcatccagcgtgacactctggccaaaggcaaagcgtttgaagtgccgctgattcgtctgggctttccgctgttcgaccgtcaccacctgcaccgccagaccacctggggttacgaaggcgcgatgaacatcgtaactactctggtaaacgcagtactggaaaagctggacagcgatacttcccagctgggcaaaaccgactattctttcgatctggttcgttaa

SEQ ID NO: 9 - DNA, 663 bp, Klebsiella pneumoniae
  misc_feature 1..663: note = wild type Gene Y, nifY
  source 1..663: mol_type = genomic DNA
atgtccgacaacgataccctattctggcgtatgctggcgctgtttcagtctctgccggacctacagccggcgcaaatcgtcgactggctggcgcaggagagcggcgagacgctgacgccagagcgtctggcgaccctgacccagccgcagctggccgccagctttccctccgcgacggcggtgatgtcccccgctcgctggtcgcgggtgatggcgagcctgcagggcgcgctgcccgcccatttacgcatcgttcgccctgcccagcgcacgccgcagctgctggcggcattttgctcccaggatgggctggtgattaacggccatttcggccagggacgactgttttttatctacgcgttcgatgaacaaggcggctggttgtacgatctgcgccgctatccctccgccccccaccagcaggaggccaacgaagtgcgcgcccggcttattgaggactgtcagctgctgttttgccaggagataggcgggcccgccgccgcgcggctgatccgccatcgcatccacccgatgaaagcgcagcccgggacgacgattcaggcacagtgcgaggcgatcaatacgctgctggccggccgtttgccgccgtggctggcgaagcggcttaacagggataaccctctggaagaacgcgttttttaa

SEQ ID NO: 10 - DNA, 663 bp, synthetic construct
  misc_feature 1..663: note = synthetic Gene Y
  source 1..663: mol_type = other DNA
atgtctgacaatgataccctgttttggcgcatgctggcgctgtttcagtcgctgccggatttgcagccggctcaaatcgtcgattggctggcgcaggaatccggcgaaaccctgacgccggagcgccttgccaccctgacccaaccgcaactcgcggcgtcgttcccatccgcgacggcagtgatgagcccggctcgctggagccgcgttatggcttctctgcaaggcgccctcccagcccacttgcgcatcgtacgtccggcgcagcgtaccccgcaactgctcgccgcgttttgcagccaagacggccttgttatcaatggtcatttcggccagggtcgtctgttcttcatttacgcctttgacgagcagggcggctggctgtatgacttgcgccgctatccgagcgcaccgcaccagcaggaagcgaatgaggtgcgtgctcgtctgattgaagattgccagctgctgttctgccaggagattggcggtccggcagcagcgcgtccgatccgccaccgcatccatccgatgaaggcgcagccgggtactacgattcaggcgcagtgtgaagctatcaacaccctgctggccggtcgcctgccgccgtggctcgccaaacgtttgaaccgtgataacccgctggaagagcgtgtgttttaa

SEQ ID NO: 11 - DNA, 1374 bp, Klebsiella pneumoniae
  misc_feature 1..1374: note = wild type Gene E, nifE
  source 1..1374: mol_type = genomic DNA
atgaagggaaatgaaattctggcgctgctggatgaaccggcctgtgaacacaaccataaacaaaaatccggctgcagcgcgcccaaacccggcgccaccgccgcgggctgcgcgttcgacggcgcgcagataaccctgctgcccatcgccgacgtggcgcatctggtccacggccccatcggctgcgccggaagctcatgggataaccgcggcagcgccagctccggccccacccttaatcggctcgggttcaccaccgatctcaacgaacaggacgtgattatgggccgcggcgaacgccgactgtttcacgccgtgcgccatatcgtcacccgctatcatccggcggcggtctttatctacaacacctgcgtaccggccatggagggcgatgacctggaagcggtatgccaggccgcgcagaccgccaccggcgtaccggttatcgctattgacgccgccggtttctacggcagtaaaaatctcggtaaccggccggcgggcgacgtcatggtcaaacgggtcatcggccagcgcgagcccgccccctggccggagagcacgctctttgccccggagcagcgtcacgatattggcctgattggcgaattcaatattgccggcgagttctggcatattcagccgctgctcgacgaactggggatccgcgtgctcggcagcctctccggtgatggccgcttcgccgagatccagaccatgcaccgggcgcaggccaatatgctggtctgctcgcgggcgttaattaacgtcgccagagccctggagcagcgctacggcacgccgtggttcgaaggcagcttttacgggatccgcgccacctctgacgccctgcgccagctggcggcgctgctgggcgacgacgaccttcgccagcgcaccgaagcgctgattgcgcgggaggaacaggcggcggaactggcgctacagccgtggcgcgaacagctgcgcggccgcaaagcgctgctctataccggcggggtgaaatcctggtcggtggtatcggcgctgcaggatttgggcatgaccgtggtggcaaccggcacgcgtaaatccaccgaagaggataaacagcggatccgcgagctgatgggcgaagaggcggtaatgctggaagagggcaacgcccgcacgctgctggatgtggtctatcgctatcaggccgacctgatgattgccggcggacgcaatatgtacaccgcctataaagccaggctgccgtttctcgatatcaatcaggagcgcgaacacgccttcgctggctatcaggggatcgtcaccctcgcccgccagctgtgtcagaccatcaacagccccatctggccgcaaacccattctcgcgccccgtggcgctaa

SEQ ID NO: 12 - DNA, 1374 bp, synthetic construct
  misc_feature 1..1374: note = synthetic Gene E
  source 1..1374: mol_type = other DNA
atgaagggtaacgagattcttgctctgctggacgaaccggcctgtgaacacaaccataaacagaaatccggctgtagcgccccaaagccgggtgcgacggcggctggctgcgctttcgatggtgcgcagatcaccctgctcccgattgcggacgttgcccacctcgtgcatggcccaatcggttgcgcaggtagctcttgggacaaccgtggcagcgcctccagcggtccgaccctgaatcgtttgggctttaccactgacttgaatgaacaagatgtgatcatgggtcgcggcgagcgtcgcctgttccacgctgtgcgccatattgtcacccgttaccacccagcggcagtattcatctacaatacgtgcgtgccggctatggaaggcgatgacctggaggccgtgtgtcaggcagcccagactgcgaccggcgtcccggtaatcgcaattgatgcggctggcttctacggttcgaagaacctgggcaaccgtccggcaggcgatgtcatggttaaacgcgtcattggccaacgtgagccagcgccgtggccggagagcaccctgtttgccccggagcaacgtcatgacattggcttgatcggtgagttcaacattgcgggcgagttttggcacattcagccgctgcttgatgagctgggtatccgcgttttgggttcgctcagcggcgatggtcgtttcgccgagattcaaaccatgcaccgtgcccaggcgaacatgctggtgtgcagccgtgctctgatcaatgttgcgcgtgctctggaacagcgctatggcaccccgtggtttgaaggctcgttctatggtatccgcgcgaccagcgacgccctgcgccagttagcggcgctgctgggcgatgacgacctccgtcagcgcaccgaggcgctgatcgcgcgtgaagaacaggcggctgagctggccctgcaaccgtggcgtgaacagctgcgtggccgcaaggccctgctctacacgggtggtgtcaaaagctggtctgtggtgtccgcgcttcaggatctgggtatgaccgtggttgccacgggcacgcgtaagagcacggaagaggataaacagcgcatccgcgaattgatgggcgaagaggccgtgatgcttgaagaaggcaacgcacgtaccttattggatgtagtttatcgctatcaagcagacctgatgattgccggtggccgcaacatgtataccgcctacaaagcgcgcttgccgttcctggacatcaaccaggaacgcgagcacgcgtttgcgggctaccaaggcatcgtgaccttagcgcgccagctgtgccaaacgattaacagcccgatctggccgcagactcattcccgcgcaccgtggcgctaa

SEQ ID NO: 13 - DNA, 1386 bp, Klebsiella pneumoniae
  misc_feature 1..1386: note = wild type Gene N, nifN
  source 1..1386: mol_type = genomic DNA
atggcagacattttccgcaccgataagccgctggcggtcagccccatcaaaaccggccagccgctcggcgcaatcctcgccagcctcgggatcgaacacagcatccctctggtccacggcgcgcaggggtgcagcgccttcgccaaagtcttttttattcaacatttccacgacccggttcccctgcagtcgacggcgatggaccccacgtcgacgattatgggcgcggacggcaatatttttaccgccctggataccctctgccagcgcaacaatccgcaggctatcgtactgctcagcaccgggctgtcggaggcccagggcagcgatatttcccgcgtggttcgccagtttcgcgaagagtatccccggcataagggggtggcgatattgacggttaacacgccggatttttatggctccatggagaacggcttcagcgcggtgttagagagcgtcattgagcagtgggtgccgccggcgccgcgcccggctcagcgcaatcgccgggtcaatctgctggtcagccatctctgttcgccgggcgatatcgagtggctgcgccgatgcgtcgaagcctttggtctgcagccgataatcctgccggacctggcgcaatcgatggacggccacctggcgcagggcgatttctcgccgctgacccagggcgggacgccgctgcgccagatagagcagatggggcaaagcctgtgcagcttcgccattggcgtctcccttcatcgcgcctcatcgctgctggccccgcgctgccgcggcgaggttatcgccctgccgcacctgatgaccctcgaacgctgcgacgcctttattcatcaactggcgaaaatttccggacgcgccgttcccgagtggctggaacgccagcgcggccagctacaggatgcgatgatcgactgccatatgtggctccagggccagcgcatggcgatagcggcggaaggcgatttgctggcggcgtggtgtgatttcgccaacagccaggggatgcagcccggcccgctggtggcccctaccggtcatcccagcctgcgccagctgccggtggaacgggtggtgccgggggatctggaggatctgcaaaccctgctgtgcgcgcatcccgccgacctgctggtggcgaactcgcacgcccgcgacctggcggagcagtttgcgctgccgctggtgcgcgcgggttttccgctctttgacaagctcggcgaattccgccgggtgcgacaggggtatagcgggatgcgcgatacgctgtttgagctggcaaacctgatacgcgagcgtcaccaccacctcgcccactaccgatcgccgctgcgccagaaccccgaatcgtcactctccacaggaggcgcttatgccgccgattaa

SEQ ID NO: 14 - DNA, 1386 bp, synthetic construct
  misc_feature 1..1386: note = synthetic Gene N
  source 1..1386: mol_type = other DNA
atggcagacattttccgcactgataagccgttggctgtgtcgccgatcaagaccggccagccgctgggtgcgatcctggcgtccctgggtatcgagcactcgattccgctggtacatggcgcgcagggctgttcggcttttgccaaggttttctttatccagcacttccacgatccggtcccgctgcaaagcacggcaatggacccgaccagcaccatcatgggcgctgatggtaacatcttcaccgcgctggacactctctgccaacgcaataacccgcaagcaattgtgctgctgagcaccggcctctccgaggcgcagggcagcgacatttcccgtgtagtgcgtcagttccgtgaagaatatccgcgtcataaaggcgtggcgattctgactgttaacaccccggacttttacggtagcatggagaacggcttttccgctgtcctggagtctgtgattgaacagtgggttccgccagccccacgtccggcgcagcgcaatcgtcgcgtcaatcttttggtgagccatctctgtagcccaggcgatattgagtggctgcgccgttgcgtcgaggccttcggtctgcaaccgatcattctgccggatctggctcagagcatggacggccaccttgctcagggtgacttttcgccgctgacgcagggcggcacgccgttgcgccaaatcgagcagatgggccagagcctttgctcttttgcgattggcgtcagcctgcaccgtgcgagcagcctgctggctccgcgttgtcgtggcgaagtcatcgccttgccgcacctcatgaccttggaacgctgcgacgcctttatccatcagttggcgaaaatcagcggtcgcgccgttccggagtggctggaacgccagcgcggtcagctgcaagacgccatgatcgattgccacatgtggctgcaaggccagcgcatggcgattgccgccgaaggcgacctgctggcagcgtggtgcgatttcgcgaactctcaaggtatgcagccgggtccactggttgctccgacgggtcatccgagcctgcgtcagttgccggtggagcgcgtggtgccgggtgatctggaggatcttcagaccctcttatgcgcacatccggccgacttactggtggcgaactcccacgcccgtgatttagcagagcaattcgccctgccgctggtgcgcgcaggcttcccgctgtttgacaaactgggcgaatttcgtcgtgttcgccagggttatagcggtatgcgtgataccctgttcgagttggcgaacctgatccgtgaacgccatcatcatctggctcattatcgcagcccgctgcgccagaacccagaatcctcgttgtctacgggtggcgcgtacgcagcggattaa

SEQ ID NO: 15 - DNA, 825 bp, Klebsiella pneumoniae
  misc_feature 1..825: note = wild type Gene U, nifU
  source 1..825: mol_type = genomic DNA
atgtggaattactccgagaaagtgaaagaccatttttttaacccccgcaatgcgcgcgtggtggacaacgccaacgcggtaggcgacgtcggttcgttaagctgcggcgacgccctgcgcctgatgctgcgcgtcgacccgcaaagcgaaatcattgaggaggcgggcttccagaccttcggctgcggcagcgccatcgcctcctcctccgcgctgacggagctgattatcggccataccctcgccgaagccgggcagataaccaatcagcagattgccgattatctcgacggactgccgccggagaaaatgcactgctcggtgatgggccaggaggccctgcgcgcggccatcgccaactttcgcggcgaaagccttgaagaggagcacgacgagggcaagctgatctgcaaatgcttcggcgtcgatgaagggcatattcgccgcgcggtacagaacaacgggctgaccacccttgccgaggtgatcaactacaccaaagcgggcggcggctgcacctcttgccacgaaaaaatcgagctggccctggcggagatcctcgcccagcagccgcagacgacgccagccgtggccagcggcaaagatccgcactggcagagcgtcgtcgataccatcgcagaactgcggccgcatattcaggccgacggcggcgatatggcgctactcagcgtcaccaaccaccaggtgaccgtcagcctctccggcagctgtagcggctgcatgatgaccgatatgaccctggcctggctgcagcaaaaactgatggaacgtaccggctgttatatggaagtggtggcggcctga

SEQ ID NO: 16 - DNA, 825 bp, synthetic construct
  misc_feature 1..825: note = synthetic Gene U
  source 1..825: mol_type = other DNA
atgtggaactacagcgagaaagtcaaggaccatttcttcaatccgcgcaacgcgcgtgttgtggataacgcaaatgcggtgggcgacgtcggcagcttatcttgtggcgatgctctccgcttgatgctgcgcgtggacccgcagagcgaaatcatcgaagaagcgggctttcagaccttcggctgcggcagcgcgattgcgtcgtccagcgcactgacggagctgatcatcggtcacaccctggcggaagcgggtcagatcaccaaccagcagatcgccgactatctggacggcttaccgccggaaaagatgcactgctctgtaatgggccaggaagctcttcgtgcggccattgctaactttcgcggtgaatcgctggaagaggagcatgacgagggtaagctgatctgcaagtgcttcggcgtcgatgaaggccatattcgccgtgctgtccagaacaacggtcttacgactctggccgaggtgatcaattacaccaaggcaggtggcggttgtaccagctgccatgagaaaatcgagctggccctggccgagattctcgcccaacagccgcaaaccaccccggcagttgcgtccggtaaagatccgcactggcagagcgtcgtggataccatcgctgaactgcgtccacatatccaagcggacggtggtgacatggcgctgttgtccgtgacgaaccaccaagtgactgtttcgctgtcgggcagctgttctggctgcatgatgaccgacatgaccctggcgtggctgcaacagaaattgatggagcgtaccggctgctatatggaagttgttgccgcctaa

SEQ ID NO: 17 - DNA, 1203 bp, Klebsiella pneumoniae
  misc_feature 1..1203: note = wild type Gene S, nifS
  source 1..1203: mol_type = genomic DNA
atgaaacaggtttatctcgataacaacgccaccacccgtctggacccgatggtcctggaagcgatgatgccctttttgaccgatttttacggcaacccctcgtcgatacacgattttggcattccggcccaggcggctctggaacgcgcgcatcagcaggctgcggcgctgctgggcgcggagtatcccagcgagatcatctttacctcctgcgccaccgaagccaccgccaccgccatcgcctcggcgatcgccctgctgcctgagcgtcgcgaaatcatcaccagcgtggtcgaacatccggcgacgctggcggcctgcgagcacatggagcgcgagggctaccggattcatcgcatcgcggtagatggcgagggggcgctggacatggcgcagttccgcgcggcgctcagcccgcgcgtcgcgttggtcagcgtgatgtgggcgaataacgaaaccggggtgcttttcccgatcggcgaaatggcggagctggcccatgaacaaggggcgctgtttcactgcgatgcggtgcaggtggtcgggaaaataccgatcgccgtgggccagacccgcatcgatatgctctcctgctcggcgcataagttccacgggccaaaaggcgtaggctgtctttatctgcggcggggaacgcgctttcgcccgctgctgcgcggcggtcaccaggagtacggtcggcgagccgggacagaaaatatctgcggaatcgtcggcatgggcgcggcctgcgagctggcgaatattcatctgccgggaatgacgcatatcggccaattgcgcaacaggctggagcatcgcctgctggccagcgtgccgtcggtcatggtgatgggcggcggccagccggcggtgcccggcacggtgaatctggcctttgagtttattgaaggtgaagccattctgctgctgttaaaccaggccgggatcgccgcctccagcggcagcgcctgcacctcaggctcgctggaaccctcccacgtgatgcgggcgatgaatatcccctacaccgccgcccacggcaccatccgcttttctctctcgcgctacacccgggagaaagagatcgattacgtcgtcgccacgctgccgccgattatcgaccggctgcgcgcgctgtcgccctactggcagaacggcaagccgcgcccggcggacgccgtattcacgccggtttacggctaa

SEQ ID NO: 18 - DNA, 1203 bp, synthetic construct
  misc_feature 1..1203: note = synthetic Gene S
  source 1..1203: mol_type = other DNA
atgaaacaagtgtacctggacaacaacgcgaccacccgcctggacccgatggttctggaagcgatgatgccgtttctcacggatttctatggcaatccgtccagcatccatgacttcggcatcccggcacaagcggcgctggaacgtgcgcaccagcaagctgcggcactgctgggcgcagagtacccgtctgaaatcattttcacgagctgtgcgaccgaggccactgcaaccgccattgcgtcggccatcgcgttattgccggaacgccgcgaaatcatcacctcggtagtggagcacccggctacgctggcggcgtgcgagcacatggaacgcgaaggctatcgcatccatcgcattgcggtggatggcgaaggtgcgctggacatggcccagttccgtgcagcgctctcgccgcgtgtcgcgttggtgagcgtgatgtgggccaacaacgaaaccggcgtgctgttcccgattggcgaaatggccgagcttgcccacgagcagggcgctctgttccactgcgatgccgttcaggtcgttggcaaaatcccaattgctgttggccagacgcgcatcgacatgctgtcttgctccgcgcacaagtttcatggtccgaagggtgttggttgcttgtacttacgtcgtggcacgcgctttcgtccgctgcttcgcggtggccatcaagaatatggtcgccgtgccggcactgagaatatctgtggcatcgtcggcatgggcgctgcgtgcgaactggcgaacatccatctgccgggtatgacccatattggccagttacgcaatcgcctggagcaccgtctgctcgccagcgtgccgtccgtgatggttatgggcggtggtcagccggctgtaccgggtactgtcaacctggcgttcgagtttatcgaaggtgaagcgatcctgctcttgctgaaccaggctggcattgccgcaagctccggctccgcgtgtacctctggcagcttggagccgagccatgtgatgcgcgccatgaacattccatacaccgcggctcacggcaccattcgttttagcctgagccgttatacgcgcgagaaagagatcgactacgtcgttgcgaccctcccgccaatcattgatcgtctgcgtgccttgtccccgtattggcagaatggtaagccgcgtccggcagatgcagtctttaccccggtttacggttaa

SEQ ID NO: 19 - DNA, 1143 bp, Klebsiella pneumoniae
  misc_feature 1..1143: note = wild type Gene V, nifV
  source 1..1143: mol_type = genomic DNA
atggaacgcgtgctgattaacgataccaccctgcgcgacggcgagcagagccccggcgtcgcctttcgcaccagcgaaaaggtcgccattgccgaggcgctttacgccgcaggaataacggcgatggaggtcggcaccccggcgatgggcgacgaggagatcgcgcggatccagctggtgcgtcgccagctgcccgacgcgaccctgatgacctggtgtcggatgaacgcgctggagatccgccagagcgccgatctgggcatcgactgggtggatatctcgattccggcttcggataagctgcggcagtacaaactgcgcgagccgctggcggtgctgctggagcggctggcgatgtttatccatcttgcgcataccctcggcctgaaggtatgcatcggctgcgaggacgcctcgcgggccagcggccagaccctgcgcgctatcgccgaggtcgcgcagcaatgcgccgccgcccgcctgcgctatgccgatacggtcggcctgctcgacccttttaccaccgcggcgcaaatctcggccctgcgcgacgtctggtccggcgaaatcgaaatgcatgcccataacgatctgggtatggcgaccgccaatacgctggcggcggtaagcgccggggccaccagcgtgaatacgacggtcctcggtctcggcgagcgggcgggcaacgcggcgctggaaaccgtcgcgctgggccttgaacgctgcctgggcgtggagaccggcgtgcatttttcggcgctgcccgcgtcctgtcagagggtcgcggaagccgcgcagcgcgccatcgacccgcagcagccgctggtcggcgagctggtgtttacccatgagtcaggtgtccacgtggcggcgctgctgcggcacagcgagagctaccagtccatcgccccttccctgatgggccgcagctaccggctggtgctgggcaaacactccgggcgtcaggcggtcaacggcgtttttgaccagatgggctatcacctcaacgccgcgcagattaaccagctgctgcccgccatccgccgcttcgccgagaactggaagcgcagcccgaaagattacgagctggtggctatctacgacgagctgtgcggtgaatccgctctgcgggcgagggggtaa

SEQ ID NO: 20 - DNA, 1143 bp, synthetic construct
  misc_feature 1..1143: note = synthetic Gene V
  source 1..1143: mol_type = other DNA
atggagcgcgtcttgatcaacgatactaccctgcgtgatggcgaacaatctccgggcgtagcgtttcgtacctccgagaaagttgccatcgcggaggcactgtacgctgcgggtatcaccgcgatggaagtcggcactccggcgatgggtgatgaagagatcgcccgcattcagctggtgcgtcgtcaactgccggacgcgacgcttatgacctggtgccgtatgaacgctctggaaatccgtcagagcgcggatctgggtattgactgggtggatatctcgatcccagcatccgacaagctgcgtcagtacaagctgcgtgagccgctggccgtgctgctggagcgccttgcgatgtttatccatctggcccacacgttaggcctcaaagtatgtattggttgcgaggatgcgagccgtgcgtctggtcagaccctgcgcgccattgccgaggtggcccagcaatgcgcggctgcgcgcttgcgttacgctgacaccgtgggcctgctggacccgttcaccaccgcagcccagatcagcgccctgcgtgacgtttggtcgggcgagatcgagatgcatgctcacaatgatctgggcatggctaccgcgaacacgctggcggcagtttcggctggcgccacgtcggtgaacactaccgtcctcggtctgggtgaacgtgcaggcaacgcagccctggaaaccgttgcgctgggcctggaacgctgcctgggcgtggaaaccggcgtccatttcagcgcgctcccagcgagctgtcagcgcgtcgcggaggctgcacagcgcgcaatcgacccgcaacagccgctggtgggtgaattggttttcacccacgagtctggtgttcacgttgcggcgctgctgcgccacagcgaatcctatcaatctattgccccaagcctcatgggccgtagctaccgtctggtgctcggcaagcattcgggtcgtcaggctgtcaacggtgttttcgaccagatgggttaccacctgaatgcggcgcagatcaatcagttgctgccggccattcgccgcttcgccgagaattggaaacgctctccgaaagactacgaactggttgcgatctatgacgaattgtgcggtgaatccgcccttcgtgctcgcggctaa

SEQ ID NO: 21 - DNA, 258 bp, Klebsiella pneumoniae
  misc_feature 1..258: note = wild type Gene W, nifW
  source 1..258: mol_type = genomic DNA
atggagtggttttatcaaattcccggcgtggacgaacttcgctccgccgaatctttttttcagtttttcgccgtcccctatcagcccgagctgcttggccgctgcagcctgccggtgctggcaacgtttcatcgcaaactccgcgcggaggtgccgctgcaaaaccggctcgaggataacgaccgcgcgccctggctgctggcgcgaagactgctcgcggagagctatcagcaacagtttcaggagagcggaacatga

SEQ ID NO: 22 - DNA, 258 bp, synthetic construct
  misc_feature 1..258: note = synthetic Gene W
  source 1..258: mol_type = other DNA
atggagtggttttaccagattccgggtgtagacgaattgcgcagcgctgaatccttctttcagttcttcgcggttccataccagccggaactgctgggccgctgctcgcttccggtgttagcgacgttccaccgtaaactgcgtgcggaggtcccgctgcaaaaccgtctggaggacaatgatcgtgcgccgtggctcttggcgcgccgcctcctggccgaatcttatcagcagcaatttcaggagagcggcacctaa

SEQ ID NO: 23 - DNA, 447 bp, Klebsiella pneumoniae
  misc_feature 1..447: note = wild type Gene Z, nifZ
  source 1..447: mol_type = genomic DNA
atgagaccgaaattcacctttagcgaagaggtccgcgtcgtacgcgcgattcgtaacgacggcaccgtggcgggcttcgcgcccggcgcgctgctggtcaggcgcggcagcaccggctttgtgcgcgactggggcgtttttttgcaagatcagattatctaccagatccactttccggaaaccgatcggatcatcggctgccgcgagcaggagctgatccccatcacccagccgtggctggccggaaatttgcaatacagggatagcgtgacctgccagatggcgctcgcggtcaacggcgatgtggtcgtgagcgccggccagcggggacgcgttgaggctaccgatcggggagagctcggcgacagctacaccgtcgactttagcggccgctggttcagggtcccggtgcaggccatcgcccttatagaggaaagagaagaatga

SEQ ID NO: 24 - DNA, 447 bp, synthetic construct
  misc_feature 1..447: note = synthetic Gene Z
  source 1..447: mol_type = other DNA
atgcgcccgaaattcaccttctctgaagaggtccgcgtagttcgcgcgattcgtaatgatggcaccgtggcgggttttgcgccaggtgcgctgctggttcgtcgcggttcgacgggctttgtgcgtgactggggtgtgttcctgcaagaccagatcatctatcaaatccactttccggaaaccgaccgcattatcggctgtcgcgagcaggagttaatcccgattacccagccgtggttggctggtaacctccagtatcgtgacagcgtcacgtgccaaatggcactggctgtcaacggtgacgtggttgtgagcgccggtcaacgtggccgtgtggaggccactgatcgtggcgaacttggcgattcctacaccgtggacttcagcggccgttggttccgcgttccggtccaggccatcgcgctgattgaagagcgcgaagaataa

SEQ ID NO: 25 - DNA, 801 bp, Klebsiella pneumoniae
  misc_feature 1..801: note = wild type Gene M, nifM
  source 1..801: mol_type = genomic DNA
atgaacccgtggcaacgttttgcccggcagcggctggcgcgcagccgctggaatcgcgatccggcggccctggatccggccgacacgccggcttttgaacaggcctggcaacgccagtgccatatggagcagacgatcgtcgcgcgggtccctgaaggcgatattccggcggcgttgctggagaatatcgctgcctcccttgccatctggctcgacgagggggattttgcgccgcccgagcgcgctgccatcgtgcgccatcacgcccggctggaactcgccttcgccgatatcgcccgccaggcgccgcagccggatctctccacggtacaggcatggtatctgcgccaccagacgcagtttatgcgcccggaacagcgtctgacccgccatttactgctgacggtcgataacgaccgcgaagccgtgcaccagcggatcctcggcctgtatcggcaaatcaacgcctcgcgggacgctttcgcgccgctggcccagcgccattcccactgcccgagcgcgctggaagagggtcgtttaggctggattagccgtggcctgctctatccgcagctcgagaccgcgctgttttcactggcggaaaacgcgctaagccttcccatcgccagcgaactgggctggcatcttttatggtgcgaagcgattcgccccgccgcgcccatggagccgcagcaggcgctggagagcgcgcgcgattatctttggcagcagagccagcagcgccatcagcgccagtggctggaacagatgatttcccgtcagccgggactgtgcgggtag

SEQ ID NO: 26 - DNA, 801 bp, synthetic construct
  misc_feature 1..801: note = synthetic Gene M
  source 1..801: mol_type = other DNA
atgaatccgtggcagcgctttgcccgtcaacgccttgctcgcagccgctggaaccgtgatccggctgctctcgacccagccgataccccagcgttcgagcaggcgtggcagcgtcaatgccatatggaacaaaccatcgtagcgcgtgtcccggaaggcgatattccggctgccttactggaaaacatcgcggccagcctggcgatctggctggacgagggtgacttcgctccgccggagcgcgctgcgattgtgcgtcatcatgcacgtctggagctggcgtttgccgacattgcccgccaggcaccgcaaccggatctgagcacggttcaagcgtggtatctgcgtcaccagactcaattcatgcgtccggagcagcgtctgacccgtcacctgctcctgacggtcgataatgatcgcgaggcggtgcatcaacgcatccttggcctgtatcgtcagatcaacgcgagccgtgacgccttcgccccactggcacagcgccactctcattgcccgtccgccttggaagaaggccgtctgggctggatctcccgtggtctgctgtacccgcagctcgaaaccgcgttgtttagcctggcggaaaacgcactgtcgctgccgattgcgtcggaattgggttggcacctgttatggtgcgaggccattcgtccggcagccccgatggagccgcaacaggcccttgaatctgcgcgcgactacttgtggcagcagagccagcagcgccaccagcgtcaatggctggagcagatgatttcccgccaaccgggcctgtgtggttaa

SEQ ID NO: 27 - DNA, 531 bp, Klebsiella pneumoniae
  misc_feature 1..531: note = wild type Gene F, nifF
  source 1..531: mol_type = genomic DNA
atggcgaacattggtattttctttggcaccgataccggtaaaacccgcaaaatcgcgaaaatgatccataagcaactgggcgagctggcggatgccccggtcaacattaaccgcacgacgctggacgactttatggcctatccggtgctgctgctgggcacgccgacgctcggcgacggccagctgccggggctggaggccggatgcgaaagcgagtcatggagcgaatttatcagcggcctcgacgacgccagcctgaaagggaaaaccgtggcgctgttcggcctcggcgatcagagaggctatccggacaacttcgtcagcgggatgcgcccgctgttcgacgccctgagcgcgcgcggcgcgcagatgattggcagctggccaaatgagggttatgaattcagcgcgtcctcggcgctggaaggcgaccgctttgttgggctggtgctggatcaggataaccagttcgaccagaccgaagcgcgtctggcgagctggcttgaggagattaaacgcaccgtgctgtag

SEQ ID NO: 28 - DNA, 531 bp, synthetic construct
  misc_feature 1..531: note = synthetic Gene F
  source 1..531: mol_type = other DNA
atggcgaacatcggcatcttctttggtacggataccggcaaaacccgcaagattgcgaagatgattcacaaacagctgggcgagctggccgatgccccggttaacatcaatcgtaccactttggatgactttatggcttacccagtcctgttgctcggcacgccgacgcttggtgatggtcaactgccgggcttagaggcgggctgcgagagcgaaagctggtctgagtttatctccggtctggatgacgcttccctgaagggcaaaaccgtggcgctgtttggcctgggcgaccagcgtggttacccggacaacttcgtgtcgggtatgcgtccgctgttcgacgcgctgagcgcccgtggcgcccagatgattggtagctggccgaacgaaggttatgagtttagcgcatcgtccgcgctggaaggcgaccgcttcgtcggcttggtgctggatcaagacaatcagttcgaccagaccgaagcgcgcctggcgtcttggcttgaagagatcaaacgcaccgttctgtaa

SEQ ID NO: 29 - DNA, 1407 bp, Klebsiella pneumoniae
  misc_feature 1..1407: note = wild type Gene B, nifB
  source 1..1407: mol_type = genomic DNA
atgacttcctgctcctctttttctggcggcaaagcctgccgcccggcggatgacagcgcattgacgccgcttgtggccgataaagctgccgcgcacccctgctactctcgccatgggcatcaccgtttcgcgcggatgcatctgcccgtcgcgcccgcctgcaatttgcagtgcaactactgtaatcgcaaattcgattgcagcaacgagtcccgccccggggtatcgtcaacgctgctgacgcctgaacaggcggtcgtgaaagtgcgtcaggtcgcgcaggcgatcccgcagctttcggtggtgggcatcgccgggcccggcgatccgctcgccaatatcgcccgcacctttcgcaccctggagctgatccgcgaacagctgccggacctgaaattatgcctgtcgaccaacggactggtgctgcctgacgcggtggaccgcctgctggatgtcggcgttgaccacgtcacggtcaccattaacaccctcgacgcggagattgccgcgcaaatctacgcctggctatggctggacggcgaacgctacagcgggcgcgaagcgggagagatcctgattgcccgtcagcttgagggcgtacgcaggctgaccgccaaaggcgtgctggtgaaaataaattcggtgctgatccccggtatcaacgatagcggcatggccggcgtgagccgcgcgctgcgggccagcggcgcgtttatccataatattatgccgctgatcgccaggccggagcacggcacggtgtttggcctcaacggccagccggagccggacgccgagacgctcgccgccacccgcagccggtgcggcgaagtgatgccgcagatgacccactgccaccagtgtcgcgccgacgccattgggatgctcggcgaagaccgcagccagcagtttacccagcttccggcgccagagagtctcccggcctggctgccgatcctccaccagcgcgcgcagctgcacgccagcattgcgacccgcggcgaatctgaagccgatgacgcctgcctggtcgccgtggcgtcaagccgcggggacgtcattgattgtcactttggtcacgccgaccggttctacatttacagcctctcggccgccggtatggtgctggtcaacgagcgctttacgcccaaatattgtcaggggcgcgatgactgcgagccgcaggataacgcagcccggtttgcggcgatcctcgaactgctggcggacgttaaagccgtattctgcgtgcgtatcggccatacgccgtggcaacagctggaacaggaaggcattgaaccctgcgttgacggcgcgtggcggccggtctccgaagtgctgcccgcgtggtggcaacagcgtcgggggagctggcctgccgcgttgccgcataagggggtcgcctga

SEQ ID NO: 30 - DNA, 1407 bp, synthetic construct
  misc_feature 1..1407: note = synthetic Gene B
  source 1..1407: mol_type = other DNA
atgacctcttgttcgtcgttttctggcggtaaagcgtgccgtccggccgatgactccgcgctgactccgctggtggccgacaaggcagctgcgcacccgtgctatagccgccacggccatcaccgcttcgcgcgtatgcacctgccagtcgctccggcctgcaacttacaatgcaactactgcaaccgcaagttcgattgcagcaatgaaagccgtccgggcgtgtcctctaccctgctgacgccggaacaggctgtggtgaaggtgcgccaggtcgcccaagctatcccgcagctgtcggtggtcggtattgctggtccgggcgatccgcttgcgaatatcgcccgcaccttccgtaccttggagcttattcgcgaacagttgccggacctgaaactgtgcctgagcaccaacggcttggtgctgccagatgccgttgatcgtctgctcgatgtgggcgtggatcacgttaccgtcaccattaacaccctggacgcagaaatcgcagcgcaaatctacgcgtggttgtggctggatggcgaacgctactccggtcgcgaagccggcgaaattctcattgcccgccagctggaaggcgtacgtcgcctgaccgcgaaaggtgtgctcgtcaagatcaacagcgtattgattccgggcatcaatgacagcggcatggcgggtgttagccgtgcgctgcgcgcgtctggtgcgttcatccacaacatcatgccactgattgcgcgtccggagcatggcactgttttcggtctgaacggccagccggaaccggacgcggaaaccctggcggcgacgcgctcccgctgcggcgaggttatgccacaaatgacccactgccaccagtgccgtgccgacgcgattggcatgcttggtgaggatcgctcgcaacagtttacgcaattaccggctccggagtccctcccggcctggctgccgatcctgcatcagcgtgctcagttgcatgcgagcatcgccacgcgcggtgagagcgaagccgatgacgcctgcctggtggccgttgcgtcgagccgtggcgatgtaattgactgccatttcggccatgccgaccgtttctatatctatagcctgtctgcggctggtatggttctggttaacgaacgtttcaccccgaaatactgccagggtcgcgatgactgcgagccgcaggacaatgccgcacgctttgctgccatccttgagttgctggcggacgtcaaagcggtgttttgtgtgcgtatcggccataccccgtggcaacagctggagcaggaaggcatcgaaccgtgcgtggatggcgcctggcgtccggtatccgaggtcctgccggcatggtggcagcagcgccgtggtagctggccggctgcattgccgcacaaaggcgttgcgtaa

SEQ ID NO: 31 - DNA, 504 bp, Klebsiella pneumoniae
  misc_feature 1..504: note = wild type Gene Q, nifQ
  source 1..504: mol_type = genomic DNA
atgccgccgctcgactggttgcggcgcttatggctgctgtaccacgcggggaaaggcagctttccgctgcgcatggggcttagcccgcgcgattggcaggcgctgcggcggcgcctgggcgaggtggaaacgccgctcgacggcgagacgctcacccgtcgccgcctgatggcggagctcaacgccacccgcgaagaggagcgccagcagctgggcgcctggctggcgggctggatgcagcaggatgccgggccgatggcgcagattatcgccgaggtttcgctggcgtttaaccatctctggcaggatcttggtctggcatcgcgcgccgaattgcgcctgctgatgagcgactgctttccacagctggtggtgatgaacgaacacaatatgcgctggaaaaagttcttttatcgtcagcgctgtttgctgcaacagggggaagttatctgccgttcgccaagctgcgacgagtgctgggaacgcagcgcctgttttgagtag

SEQ ID NO: 32 - DNA, 504 bp, synthetic construct
  misc_feature 1..504: note = synthetic Gene Q
  source 1..504: mol_type = other DNA
atgccgccattggactggttgcgtcgtttgtggttactctatcacgccggcaaaggcagctttccgcttcgtatgggcttgtcgccgcgtgactggcaagctctgcgccgtcgcctgggcgaggtggaaacgccgctggatggcgaaaccctgacccgtcgccgtctgatggcggagctgaatgcgacccgcgaagaagaacgccagcagctgggtgcctggctggccggttggatgcaacaggatgccggtccgatggcgcagattatcgcagaggtgagcctggcgttcaaccatctctggcaggaccttggcctcgcgagccgcgctgaactgcgtctgctgatgtctgactgcttcccgcagctggttgttatgaacgagcacaacatgcgctggaagaaattcttttaccgccagcgttgcctgctgcaacagggcgaagtcatctgtcgcagcccgtcttgcgatgaatgctgggaacgttctgcgtgctttgagtaa

SEQ ID NO: 33 - DNA, 1117 bp, synthetic construct
  misc_feature 1..1117: note = synthetic lacI sequence of Ptac-T7 synthetic controller
  source 1..1117: mol_type = other DNA
caattcgcgctaacttacattaattgcgttgcgctcactgcccgctttccagtcgggaaacctgtcgtgccagctgcattaatgaatcggccaacgcgcggggagaggcggtttgcgtattgggcgccagggtggtttttcttttcaccagtgagacgggcaacagctgattgcccttcaccgcctggccctgagagagttgcagcaagcggtccacgctggtttgccccagcaggcgaaaatcctgtttgatggtggttgacggcgggatataacatgagctgtcttcggtatcgtcgtatcccactaccgagatatccgcaccaacgcgcagcccggactcggtaatggcgcgcattgcgcccagcgccatctgatcgttggcaaccagcatcgcagtgggaacgatgccctcattcagcatttgcatggtttgttgaaaaccggacatggcactccagtcgccttcccgttccgctatcggctgaatttgattgcgagtgagatatttatgccagccagccagacgcagacgcgccgagacagaacttaatgggcccgctaacagcgcgatttgctggtgacccaatgcgaccagatgctccacgcccagtcgcgtaccgtcttcatgggagaaaataatactgttgatgggtgtctggtcagagacatcaagaaataacgccggaacattagtgcaggcagcttccacagcaatggcatcctggtcatccagcggatagttaatgatcagcccactgacgcgttgcgcgagaagattgtgcaccgccgctttacaggcttcgacgccgcttcgttctaccatcgacaccaccacgctggcacccagttgatcggcgcgagatttaatcgccgcgacaatttgcgacggcgcgtgcagggccagactggaggtggcaacgccaatcagcaacgactgtttgcccgccagttgttgtgccacgcggttgggaatgtaattcagctccgccatcgccgcttccactttttcccgcgttttcgcagaaacgtggctggcctggttcaccacgcgggaaacggtctgataagagacaccggcatactctgcgacatcgtataacgttactggtttcac

SEQ ID NO: 34 - DNA, 589 bp, synthetic construct
  misc_feature 1..589: note = synthetic lacI promoter sequence of Ptac-T7 synthetic controller
  source 1..589: mol_type = other DNA
attcaccaccctgaattgactctcttccgggcgctatcatgccataccgcgaaaggttttgcaccattcgatggtgtcaacgtaaatgcatgccgcttcgccttcgcgcgcgaattggccgccatgccggcgataatggcctgcttctcgccgaaacgtttggtggcgggaccagtgacgaaggcttgagcgagggcgtgcaagattccgaataccgcaagcgacaggccgatcatcgtcgcgctccagcgaaagcggtcctcgccgaaaatgacccagagcgctgccggcacctgtcctacgagttgcatgataaagaagacagtcataagtgcggcgacgatagtcatgccccgcgcccaccggaaggagctgactgggttgaaggctctcaagggcatcggcggagcttatcgactgcacggtgcaccaatgcttctggcgtcaggcagccatcggaagctgtggtatggctgtgcaggtcgtaaatcactgcataattcgtgtcgctcaaggcgcactcccgttctggataatgttttttgcgccgacatcataacggttctggcaaatattctgaaatgagctg

SEQ ID NO: 35 - DNA, 55 bp, synthetic construct
  misc_feature 1..55: note = synthetic tac promoter sequence of Ptac-T7 synthetic controller
  source 1..55: mol_type = other DNA
ttgacaattaatcatcggctcgtataatgtgtggaattgtgagcggataacaatt

SEQ ID NO: 36 - DNA, 40 bp, synthetic construct
  misc_feature 1..40: note = synthetic insulator 1 sequence of Ptac-T7 synthetic controller
  source 1..40: mol_type = other DNA
tgcagttttattctctcgccagcactgtaataggcactaa

SEQ ID NO: 37 - DNA, 34 bp, synthetic construct
  misc_feature 1..34: note = synthetic Enterobacteria phage T7 RNA polymerase (RNAP) ribosome binding site (rbs, RBS) sequence of Ptac-T7 synthetic controller
  source 1..34: mol_type = other DNA
tatccaaaccagtagctcaattggagtcgtctat

SEQ ID NO: 38 - DNA, 120 bp, synthetic construct
  misc_feature 1..120: note = synthetic umuD degradatiobn tag sequence of Ptac-T7 synthetic controller
  source 1..120: mol_type = other DNA
gtgttgtttatcaagcctgcggatctccgcgaaattgtgacttttccgctatttagcgatcttgttcagtgtggctttccttcaccggcagcagattacgttgaacagcgcatcgatctg

SEQ ID NO: 39 - DNA, 2568 bp, synthetic construct
  misc_feature 1..2568: note = synthetic Enterobacteria phage T7 RNA polymerase (RNAP) scaffold sequence of Ptac-T7 synthetic controller
  source 1..2568: mol_type = other DNA
ggtggcaacacgattaacatcgctaagaacgacttctctgacatcgaactggctgctatcccgttcaacactctggctgaccattacggtgagcgtttagctcgcgaacagttggcccttgagcatgagtcttacgagatgggtgaagcacgcttccgcaagatgtttgagcgtcaacttaaagctggtgaggttgcggataacgctgccgccaagcctctcatcactaccctactccctaagatgattgcacgcatcaacgactggtttgaggaagtgaaagctaagcgcggcaagcgcccgacagccttccagttcctgcaagaaatcaagccggaagccgtagcgtacatcaccattaagaccactctggcttgcctaaccagtgctgacaatacaaccgttcaggctgtagcaagcgcaatcggtcgggccattgaggacgaggctcgcttcggtcgtatccgtgaccttgaagctaagcacttcaagaaaaacgttgaggaacaactcaacaagcgcgtagggcacgtctacaagaaagcatttatgcaagttgtcgaggctgacatgctctctaagggtctactcggtggcgaggcgtggtcttcgtggcataaggaagactctattcatgtaggagtacgctgcatcgagatgctcattgagtcaaccggaatggttagcttacaccgccaaaatgctggcgtagtaggtcaagactctgagactatcgaactcgcacctgaatacgctgaggctatcgcaacccgtgcaggtgcgctggctggcatctctccgatgttccaaccttgcgtagttcctcctaagccgtggactggcattactggtggtggctattgggctaacggtcgtcgtcctctggcgctggtgcgtactcacagtaagaaagcactgatgcgctacgaagacgtttacatgcctgaggtgtacaaagcgattaacattgcgcaaaacaccgcatggaaaatcaacaagaaagtcctagcggtcgccaacgtaatcaccaagtggaagcattgtccggtcgaggacatccctgcgattgagcgtgaagaactcccgatgaaaccggaagacatcgacatgaatcctgaggctctcaccgcgtggaaacgtgctgccgctgctgtgtaccgcaaggacaaggctcgcaagtctcgccgtatcagccttgagttcatgcttgagcaagccaataagtttgctaaccataaggccatctggttcccttacaacatggactggcgcggtcgtgtttacgctgtgtcaatgttcaacccgcaaggtaacgatatgaccaaaggactgcttacgctggcgaaaggtaaaccaatcggtaaggaaggttactactggctgaaaatccacggtgcaaactgtgcgggtgtcgacaaggttccgttccctgagcgcatcaagttcattgaggaaaaccacgagaacatcatggcttgcgctaagtctccactggagaacacttggtgggctgagcaagattctccgttctgcttccttgcgttctgctttgagtacgctggggtacagcaccacggcctgagctataactgctcccttccgctggcgtttgacgggtcttgctctggcatccagcacttctccgcgatgctccgagatgaggtaggtggtcgcgcggttaacttgcttcctagtgaaaccgttcaggacatctacgggattgttgctaagaaagtcaacgagattctacaagcagacgcaatcaatgggaccgataacgaagtagttaccgtgaccgatgagaacactggtgaaatctctgagaaagtcaagctgggcactaaggcactggctggtcaatggctggcttacggtgttactcgcagtgtgactaagagttcagtcatgacgctggcttacgggtccaaagagttcggcttccgtcaacaagtgctggaagataccattcagccagctattgattccggcaagggtctgatgttcactcagccgaatcaggctgctggatacatggctaagctgatttgggaatctgtgagcgtgacggtggtagctgcggttgaagcaatgaactggcttaagtctgctgctaagctgctggctgctgaggtcaaagataagaagactggagagattcttcgcaagcgttgcgctgtgcattgggtaactcctgatggtttccctgtgtggcaggaatacaagaagcctattcagacgcgcttgaacctgatgttcctcggtcagttccgcttacagcctaccattaacaccaacaaagatagcgagattgatgcacacaaacaggagtctggtatcgctcctaactttgtacacagccaagacggtagccaccttcgtaagactgtagtgtgggcacacgagaagtacggaatcgaatcttttgcactgattcacgactccttcggtacgattccggctgacgctgcgaacctgttcaaagcagtgcgcgaaactatggttgacacatatgagtcttgtgatgtactggctgatttctacgaccagttcgctgaccagttgcacgag

SEQ ID NO: 40 - DNA, 21 bp, synthetic construct
  misc_feature 1..21: note = synthetic Biobrick suffix (BBa_G00001) sequence of Ptac-T7 synthetic controller
  source 1..21: mol_type = other DNA
tactagtagcggccgctgcag

SEQ ID NO: 41 - DNA, 12 bp, synthetic construct
  misc_feature 1..12: note = synthetic translational stop (BBa_B0042) sequence of Ptac-T7 synthetic controller
  source 1..12: mol_type = other DNA
ttagttagttag

SEQ ID NO: 42 - DNA, 69 bp, synthetic construct
  misc_feature 1..69: note = synthetic terminator (BBa_B0054) sequence of Ptac-T7 synthetic controller
  source 1..69: mol_type = other DNA
attagcagaaagtcaaaagcctccgaccggaggcttttgactaaaacttcccttggggttatcattggg

SEQ ID NO: 43 - DNA, 20 bp, synthetic construct
  misc_feature 1..20: note = synthetic VR primer (BBa_G00102) sequence of Ptac-T7 synthetic controller
  source 1..20: mol_type = other DNA
gctcactcaaaggcggtaat

SEQ ID NO: 44 - DNA, 41 bp, synthetic construct
  misc_feature 1..41: note = synthetic terminator (BBa_B0062) sequence of Ptac-T7 synthetic controller
  source 1..41: mol_type = other DNA
cagataaaaaaaatccttagctttcgctaaggatgatttct

SEQ ID NO: 45 - DNA, 3671 bp, synthetic construct
  misc_feature 1..3671: note = synthetic pSa origin sequence of Ptac-T7 synthetic controller
  source 1..3671: mol_type = other DNA
gctagagctgtcagaccagagctccaaaccaacgttttatctataccgctacagggtatttaattcctatttaatctgcgctagaatgaggcatgtttaaccgaatctgacgttttccctgcaaatgccaaaatactatgcctatctccgggtttcgcgtgacggccaagacccggaaaaccaaaaatacggtttgctcgaatacgcgaacgccaaaggcttcgcgccgctacagatcgaggaagaaattgccagcagagcaaaggactggcgcaagcgcaagctcggagcaatcatcgaaaaggccgagcgtggcgacgtgctactgacgccggagattacgcgcattgccggttccgccctcgccgccttggaaattctcaaagcggcgagcgagcgcggcctaatcgtccatgtgaccaaacagaagatcatcatggacggcagcctacaaagcgacatcatggcaaccgtgcttggcttggctgcacagatcgagcggcatttcattcaggcacgtaccaccgaggcgctacaagtcgccagagagcgcggcaagacgctcgggcgacccaagggcagcaaatcgagcgccttgaagctggacagccgtattgatgaagtacaggcatacgtgaaccttggcttgccgcaaagtcgcgcagccgagttgttaggcgtcagccctcacaccttgcgcctgttcatcaaacgccggaacatcaaacccacaaacactagaccaaccatcaccatgccggggagggaacaacatgcctaagaacaacaaagcccccggccatcgtatcaacgagatcatcaagacgagcctcgcgctcgaaatggaggatgcccgcgaagctggcttagtcggctacatggcccgttgccttgtgcaagcgaccatgccccacaccgaccccaagaccagctactttgagcgcaccaatggcatcgtcaccttgtcgatcatgggcaagccgagcatcggcctgccctacggttctatgccgcgcaccttgcttgcttggatatgcaccgaggccgtgcgaacgaaagaccccgtgttgaaccttggccggtcgcaatcggaatttctacaaaggctcggaatgcacaccgatggccgttacacggccacccttcgcaatcaggcgcaacgcctgttttcatccatgatttcgcttgccggcgagcaaggcaatgacttcggcattgagaacgtcgtcattgccaagcgcgcttttctattctggaatcccaagcggccagaagatcgggcgctatgggatagcaccctcaccctcacaggcgatttcttcgaggaagtcacccgctcaccggttcctatccgaatcgactacctgcatgccttgcggcagtctccgcttgcgatggacatttacacgtggctgacctatcgcgtgttcctgttgcgggccaagggccgccccttcgtgcaaatcccttgggtcgccctgcaagcgcaattcggctcatcctatggcagccgcgcacgcaactcgcccgaactggacgataaggcccgagagcgggcagagcgggcagcactcgccagcttcaaatacaacttcaaaaagcgcctacgcgaagtgttgattgtctatcccgaggcaagcgactgcatcgaagatgacggcgaatgcctgcgcatcaaatccacacgcctgcatgtcacccgcgcacccggcaagggcgctcgcatcggcccccctccgacttgaccaggccaacgctacgcttggcttggtcaagccttcccatccaacagcccgccgtcgagcgggcttttttatccccggaagcctgtggatagagggtagttatccacgtgaaaccgctaatgccccgcaaagccttgattcacggggctttccggcccgctccaaaaactatccacgtgaaatcgctaatcagggtacgtgaaatcgctaatcggagtacgtgaaatcgctaataaggtcacgtgaaatcgctaatcaaaaaggcacgtgagaacgctaatagccctttcagatcaacagcttgcaaacacccctcgctccggcaagtagttacagcaagtagtatgttcaattagcttttcaattatgaatatatatatcaattattggtcgcccttggcttgtggacaatgcgctacgcgcaccggctccgcccgtggacaaccgcaagcggttgcccaccgtcgagcgccagcgcctttgcccacaacccggcggccgcaacagatcgttttataaatttttttttttgaaaaagaaaaagcccgaaaggcggcaacctctcgggcttctggatttccgatcaacgcaggagtcgttcggaaagtagctgttccagaattataggcgcagagacaccagattccaagatggctctgttaaattgttgtagtatgtagtatcatacaacatactacagtacagaggcccgcaagaatggcaatcactaaacaagacatttggcgagcagccgacgaactggacgccgaaggcatccggcccactttggccgccgtgcgcaagaaactcggaagcggtagcttcacaaccatttccgatgcaatggctgaatggaaaaaccgcaagaccgccaccctgccctcatcagacccattgccggttgcagtcaacgagcatcttgccgagcttggcaatgcgctatgggctatcgccctggcgcacgccaacgcccggtttgacgaagatcggaaacagatcgaggccgacaaagcggccatcagccagcagcttgccgaagcaatcgaactagccgacaccttcacccgcgaaaacgaccagctccgcgaacgagtgaatcagctcgaacctatggaacgcgagcgcgacaagctggccgaccagcttgccgaagtgaaacgccgcagcggcgaagaactaaaccgctgcatggaaaagctcacccaacgcgataacgaggctatcgaggcccgcaaacaggccaaggaggccatcgagcgcgccgccagtctgcaaggtcaggtggaagccctcaaagagcaggtcgccaatctcacagccgtcttgaaaacaggaggcaaacaatgaaaagcgcccttgccgcccttcgcgcggtcgcggccgctgtcgtcctaatcgtcagtgtgcccgcttgggccgacttccggggtgaagtcgtccgaatccttgacggtgacactatcgacgttttggtgaaccgtcagaccatccgcgtgagattggccgatattgacgcaccggaaagcggccaagccttcggctcccgtgctcgccaacggctcgccgacttgacctttcgccaagaggttcaagtgaccgaaaaagaggttgatcggtatggccgcactcttggggtcgtttacgcgccgttgcaataccccggcggccaaacacaactcaccaacatcaatgcgatcatggttcaagaaggcatggcctgggcttaccgttattacggcaaaccaaccgacgcgcagatgtacgagtatgaaaaagaggcccgccgccaacggctcggcctttggtcagacccgaatgctcaggagccttggaaatggcgtcgcgcctcgaaaaatgccacgaactgacaccgggcacgccccttgttcgacgcgccgcaggcacgtcgaatttaccgccgggacg

SEQ ID NO: 46 - DNA, 1175 bp, synthetic construct
  misc_feature 1..1175: note = synthetic spectinomycin resistance sequence of Ptac-T7 synthetic controller
  source 1..1175: mol_type = other DNA
cccctcgtcccgacacttccagatcgccatagcgcacagcgcctcgagcggtggtaacggcgcagtggcggttttcatggcttgttatgactgtttttttggggtacagtctatgcctcgggcatccaagcagcaagcgcgttacgccgtgggtcgatgtttgatgttatggagcagcaacgatgttacgcagcagggcagtcgccctaaaacaaagttaaacatcatgagggaagcggtgatcgccgaagtatcgactcaactatcagaggtagttggcgtcatcgagcgccatctcgaaccgacgttgctggccgtacatttgtacggctccgcagtggatggcggcctgaagccacacagtgatattgatttgctggttacggtgaccgtaaggcttgatgaaacaacgcggcgagctttgatcaacgaccttttggaaacttcggcttcccctggagagagcgagattctccgcgctgtagaagtcaccattgttgtgcacgacgacatcattccgtggcgttatccagctaagcgcgaactgcaatttggagaatggcagcgcaatgacattcttgcaggtatcttcgagccagccacgatcgacattgatctggctatcttgctgacaaaagcaagagaacatagcgttgccttggtaggtccagcggcggaggaactctttgatccggttcctgaacaggatctatttgaggcgctaaatgaaaccttaacgctatggaactcgccgcccgactgggctggcgatgagcgaaatgtagtgcttacgttgtcccgcatttggtacagcgcagtaaccggcaaaatcgcgccgaaggatgtcgctgccgactgggcaatggagcgcctgccggcccagtatcagcccgtcatacttgaagctagacaggcttatcttggacaagaagaagatcgcttggcctcgcgcgcagatcagttggaagaatttgtccactacgtgaaaggcgagatcaccaaggtagtcggcaaataatgtctaacaattcgttcaagccgacgccgcttcgcggcgcggcttaactcaagcgttagatgcactaagcacataattgctcacagccaaactatcaggtcaagtctgcttttattatttttaagcgtgcataataagccctacacaaatggtaccc

SEQ ID NO: 47 - DNA, 72 bp, synthetic construct
  misc_feature 1..72: note = synthetic terminator (BBa_B0053) sequence of Ptac-T7 synthetic controller
  source 1..72: mol_type = other DNA
tccggcaaaaaaacgggcaaggtgtcaccaccctgccctttttctttaaaaccgaaaagattacttcgcgtt

SEQ ID NO: 48 - DNA, 20 bp, synthetic construct
  misc_feature 1..20: note = synthetic VF2 primer (BBa_G000101) sequence of Ptac-T7 synthetic controller
  source 1..20: mol_type = other DNA
tgccacctgacgtctaagaa

SEQ ID NO: 49 - DNA, 78 bp, synthetic construct
  misc_feature 1..78: note = synthetic terminator (BBa_B0055) sequence of Ptac-T7 synthetic controller
  source 1..78: mol_type = other DNA
aaggaatattcagcaatttgcccgtgccgaagaaaggcccacccgtgaaggtgagccagtgagttgattgctacgtaa

SEQ ID NO: 50 - DNA, 12 bp, synthetic construct
  misc_feature 1..12: note = synthetic translational stop (BBa_B0042) sequence of Ptac-T7 synthetic controller
  source 1..12: mol_type = other DNA
ttagttagttag

SEQ ID NO: 51 - DNA, 22 bp, synthetic construct
  misc_feature 1..22: note = synthetic Biobrick prefix (BBa_G00000) sequence of Ptac-T7 synthetic controller
  source 1..22: mol_type = other DNA
gaattcgcggccgcttctagag

SEQ ID NO: 52 - DNA, 23 bp, synthetic construct
  misc_feature 1..23: note = synthetic Enterobacteria phage T7 wild type (WT) promoter of full synthetic cluster
  source 1..23: mol_type = other DNA
taatacgactcactatagggaga

SEQ ID NO: 53 - DNA, 28 bp, synthetic construct
  misc_feature 1..28: note = synthetic nifH ribosome binding site (rbs, RBS) of full synthetic cluster
  source 1..28: mol_type = other DNA
acaataaactaacataaggaggataaat

SEQ ID NO: 54 - DNA, 882 bp, synthetic construct; identical to SEQ ID NO: 4
  misc_feature 1..882: note = synthetic nifH of full synthetic cluster
  source 1..882: mol_type = other DNA

SEQ ID NO: 55 - DNA, 50 bp, synthetic construct
  misc_feature 1..50: note = synthetic insulator 1 of full synthetic cluster
  source 1..50: mol_type = other DNA
gcgtgcgtacaccttaatcaccgcttcatgctaaggtcctggctgcatgc

SEQ ID NO: 56 - DNA, 34 bp, synthetic construct
  misc_feature 1..34: note = synthetic nifD ribosome binding site (rbs, RBS) of full synthetic cluster
  source 1..34: mol_type = other DNA
aaaaattcacatccctatctagcggaggagccgg

SEQ ID NO: 57 - DNA, 1452 bp, synthetic construct; identical to SEQ ID NO: 6
  misc_feature 1..1452: note = synthetic nifD of full synthetic cluster
  source 1..1452: mol_type = other DNA

SEQ ID NO: 58 - DNA, 50 bp, synthetic construct
  misc_feature 1..50: note = synthetic insulator 2 of full synthetic cluster
  source 1..50: mol_type = other DNA
caaacaccccatgtcgatactgaacgaatcgacgcacactcccttccttg

SEQ ID NO: 59 - DNA, 34 bp, synthetic construct
  misc_feature 1..34: note = synthetic nifK ribosome binding site (rbs, RBS) of full synthetic cluster
  source 1..34: mol_type = other DNA
caatctcatactctcaaaaattaggcgaggtaac

SEQ ID NO: 60 - DNA, 1563 bp, synthetic construct; identical to SEQ ID NO: 8
  misc_feature 1..1563: note = synthetic nifK of full synthetic cluster
  source 1..1563: mol_type = other DNA

SEQ ID NO: 61 - DNA, 40 bp, synthetic construct
  misc_feature 1..40: note = synthetic insulator 3 of full synthetic cluster
  source 1..40: mol_type = other DNA
cctgattgtatccgcatctgatgctaccgtggttgagtta

SEQ ID NO: 62 - DNA, 26 bp, synthetic construct
  misc_feature 1..26: note = synthetic nifY ribosome binding site (rbs, RBS) of full synthetic cluster
  source 1..26: mol_type = other DNA
ccatactcactcccggaggtacttct

SEQ ID NO: 63 - DNA, 663 bp, synthetic construct; identical to SEQ ID NO: 10
  misc_feature 1..663: note = synthetic nifY of full synthetic cluster
  source 1..663: mol_type = other DNA

SEQ ID NO: 64 - DNA, 40 bp, synthetic construct
  misc_feature 1..40: note = synthetic insulator 4 of full synthetic cluster
  source 1..40: mol_type = other DNA
catttttgccttgcgacagacctcctacttagattgccac

SEQ ID NO: 65 - DNA, 32 bp, synthetic construct
  misc_feature 1..32: note = synthetic nifE ribosome binding site (rbs, RBS) of full synthetic cluster
  source 1..32: mol_type = other DNA
actattcaatacatcactggaggttattacaa

SEQ ID NO: 66 - DNA, 1374 bp, synthetic construct; identical to SEQ ID NO: 12
  misc_feature 1..1374: note = synthetic nifE of full synthetic cluster
  source 1..1374: mol_type = other DNA

SEQ ID NO: 67 - DNA, 40 bp, synthetic construct
  misc_feature 1..40: note = synthetic insulator 5 of full synthetic cluster
  source 1..40: mol_type = other DNA
tgtcacgctaggaggcaattctataagaatgcacactgca

SEQ ID NO: 68 - DNA, 31 bp, synthetic construct
  misc_feature 1..31: note = synthetic nifN ribosome binding site (rbs, RBS) of full synthetic cluster
  source 1..31: mol_type = other DNA
cctaaacctaccacacctggaagaagtaatt

SEQ ID NO: 69 - DNA, 1386 bp, synthetic construct; identical to SEQ ID NO: 14
  misc_feature 1..1386: note = synthetic nifN of full synthetic cluster
  source 1..1386: mol_type = other DNA

SEQ ID NO: 70 - DNA, 27 bp, synthetic construct
  misc_feature 1..27: note = synthetic nifJ ribosome binding site (rbs, RBS) of full synthetic cluster
  source 1..27: mol_type = other DNA
ctagagattaaagaggagaaattaagc

SEQ ID NO: 71 - DNA, 3507 bp, synthetic construct
  misc_feature 1..3507: note = synthetic nifJ of full synthetic cluster
  source 1..3507: mol_type = other DNA
atgaaaactatggacggtaacgctgcggctgcatggattagctacgcctttaccgaagtggctgcgatctacccgattacgccgagcaccccgatggcggaaaatgtggacgaatgggctgcgcagggcaagaagaacctcttcggccagccggtgcgcctgatggagatgcagtcggaagcgggtgcagcaggtgctgtgcatggcgccttgcaagctggcgcactgacgaccacctacaccgcgtcgcagggcctgttgctgatgatcccaaacatgtacaaaatcgcgggtgaactgctgccgggtgtctttcatgtttcggcacgcgcactggccaccaatagcctcaacatctttggcgatcatcaggatgtaatggcggtgcgccaaacgggctgcgcgatgttggccgagaataacgtccagcaagttatggatttgtccgcggtagcccacttggcagcgatcaaaggtcgcattccgttcgtgaacttcttcgatggctttcgcaccagccacgaaatccagaagatcgaggttctggaatatgaacagctggccaccttgttggatcgtccggccctggacagcttccgccgtaacgcccttcacccggaccacccggtcatccgtggcaccgcccagaacccggacatctacttccaggaacgtgaggccggtaaccgtttctatcaggcgctcccggatattgtggaatcttacatgacccagatttctgccctgactggtcgcgagtatcacctgtttaactacactggtgctgcggatgcggagcgcgtgatcatcgcgatgggctctgtctgtgacaccgtccaagaggtggttgacacgctgaatgcagcgggtgagaaagttggtctgctctccgttcatcttttccgcccgttttcgttagcgcacttcttcgcccaactgccgaaaactgtacagcgtatcgcagtattggaccgtacgaaagagccaggtgctcaagcagagccgctgtgcctcgatgtgaagaatgccttttaccaccatgacgatgccccgttgattgtgggtggtcgctatgccttgggcggtaaggacgtgttgccgaacgatattgcggccgtgtttgataacctgaacaaaccgctgccgatggacggcttcacgctgggtatcgtggacgatgttaccttcacctctctcccgccagcgcagcagaccctggcggtttctcacgacggcatcacggcatgtaagttttggggcatgggctccgacggcacggttggtgcgaacaagtccgcgatcaagattatcggcgacaaaacgccactgtatgcgcaagcgtacttttcctacgactcgaagaagagcggtggtattaccgtcagccatctgcgttttggtgatcgcccgatcaactccccgtatttgatccatcgcgcggatttcatctcgtgcagccagcaaagctatgttgaacgctacgatctgctggatggccttaaaccgggtggcacctttctgctgaactgctcctggagcgatgccgaactggagcaacatctgccggtcggtttcaaacgttatctggcacgcgagaatatccacttctacactctcaacgctgtggacatcgcccgtgagcttggtttgggtggccgtttcaacatgctgatgcaggctgccttcttcaaactggccgcgatcattgacccgcagactgctgcggactatctgaagcaggctgttgagaaaagctatggcagcaaaggtgcggcggtcatcgagatgaaccagcgtgccatcgagcttggcatggccagcctgcaccaggtgacgatcccggcacattgggccaccctggatgagccagcggcgcaggcgtccgcgatgatgccggactttatccgcgacatcctgcaaccgatgaaccgtcagtgcggcgaccagcttccggtgtcggcttttgtcggcatggaagatggcaccttcccgtccggcacggccgcatgggagaaacgtggcatcgcccttgaggtgccagtctggcagccggaaggctgcacgcagtgcaaccagtgcgccttcatttgtccgcacgccgcgattcgtccggcgttgttgaatggcgaagagcatgatgctgccccggttggcctgctgagcaaaccggcacaaggcgctaaagaatatcactatcatctggcgattagcccgctggactgctccggctgtggcaactgcgttgacatttgtccagctcgtggcaaagcgttgaagatgcagtctctggatagccaacgccagatggctccggtgtgggattatgcgctggcgctgaccccgaagtctaacccgtttcgtaaaaccaccgtcaaaggctcgcagttcgaaaccccgctgctggagtttagcggtgcgtgcgctggttgtggcgaaacgccgtatgcgcgcctcattacccagctgtttggcgaccgcatgctgattgccaatgccaccggctgttccagcatctggggcgcatctgcgccgagcatcccgtataccaccaatcatcgtggtcatggtccggcctgggcgaatagcctgtttgaggacaatgccgaatttggtttaggtatgatgctgggcggtcaagctgtgcgtcaacagatcgcggacgatatgacggctgcgttagcgctcccggtttccgatgagctgagcgacgcgatgcgccagtggttggcgaaacaggacgagggtgaaggcacgcgtgagcgtgcggaccgtctgagcgagcgcttagccgcggagaaagagggcgttccgctgttagagcagctgtggcaaaatcgtgattactttgtgcgtcgcagccagtggattttcggcggtgacggctgggcctatgatattggcttcggtggcctggaccacgtcctcgccagcggtgaggatgtgaacattctggtatttgacaccgaagtctactcgaacaccggcggtcaaagcagcaaatcgaccccggtcgcggccatcgccaagttcgcggctcagggcaagcgcacccgcaagaaagacctgggtatgatggcgatgagctacggcaacgtctatgtagcccaggtggcgatgggtgcggataaagatcaaactctgcgcgccattgcggaagctgaagcgtggccaggcccgtcgctggtgattgcgtatgcggcctgcatcaatcatggcctgaaggccggtatgcgttgcagccaacgtgaggcgaagcgcgctgttgaggcgggctactggcacctgtggcgttatcacccgcagcgcgaagcggaaggcaagacgccgtttatgttagatagcgaagaaccggaagagtcgttccgtgactttctgttgggtgaggtgcgctacgcatccctgcacaagaccaccccgcacctcgccgatgcccttttcagccgtaccgaagaagatgcgcgtgcgcgctttgcgcaataccgtcgcctggctggcgaagagtaataa

SEQ ID NO: 72 - DNA, 37 bp, synthetic construct
  misc_feature 1..37: note = synthetic Enterobacteria phage T7 terminator 25 of full synthetic cluster
  source 1..37: mol_type = other DNA
tactctaaccccatcggccgtcttaggggttttttgt

SEQ ID NO: 73 - DNA, 30 bp, synthetic construct
  misc_feature 1..30: note = synthetic insulator 6 of full synthetic cluster
  source 1..30: mol_type = other DNA
ccgtggttgagtcagcgtcgagcacgcggc

SEQ ID NO: 74 - DNA, 23 bp, synthetic construct
  misc_feature 1..23: note = synthetic Enterobacteria phage T7 promoter mut 2 of full synthetic cluster
  source 1..23: mol_type = other DNA
taatacgactcactagagagaga

SEQ ID NO: 75 - DNA, 40 bp, synthetic construct
  misc_feature 1..40: note = synthetic insulator 7 of full synthetic cluster
  source 1..40: mol_type = other DNA
cgcgacttccagagaagaagactactgacttgagcgttcc

SEQ ID NO: 76 - DNA, 39 bp, synthetic construct
  misc_feature 1..39: note = synthetic nifB ribosome binding site (rbs, RBS) of full synthetic cluster
  source 1..39: mol_type = other DNA
ctctctgtaatacatcaaatcaatcataggagggctaaa

SEQ ID NO: 77 - DNA, 1407 bp, synthetic construct; identical to SEQ ID NO: 30
  misc_feature 1..1407: note = synthetic nifB of full synthetic cluster
  source 1..1407: mol_type = other DNA

SEQ ID NO: 78 - DNA, 40 bp, synthetic construct
  misc_feature 1..40: note = synthetic insulator 8 of full synthetic cluster
  source 1..40: mol_type = other DNA
actacgagatttgaggtaaaccaaataagcacgtagtggc

SEQ ID NO: 79 - DNA, 33 bp, synthetic construct
  misc_feature 1..33: note = synthetic nifQ ribosome binding site (rbs, RBS) of full synthetic cluster
  source 1..33: mol_type = other DNA
tgcgtttagcagttcccgtaggaatatttcctt

SEQ ID NO: 80 - DNA, 504 bp, synthetic construct; identical to SEQ ID NO: 32
  misc_feature 1..504: note = synthetic nifQ of full synthetic cluster
  source 1..504: mol_type = other DNA

SEQ ID NO: 81 - DNA, 29 bp, synthetic construct
  misc_feature 1..29: note = synthetic Enterobacteria phage T7 terminator 1 of full synthetic cluster
  source 1..29: mol_type = other DNA
tacatatcgggggggtaggggttttttgt

SEQ ID NO: 82 - DNA, 18 bp, synthetic construct
  misc_feature 1..18: note = synthetic insulator 9 of full synthetic cluster
  source 1..18: mol_type = other DNA
gtctgtagcacgtgcatc

SEQ ID NO: 83 - DNA, 23 bp, synthetic construct
  misc_feature 1..23: note = synthetic Enterobacteria phage T7 promoter mut 3 of full synthetic cluster
  source 1..23: mol_type = other DNA
taatacgactcactaatgggaga

SEQ ID NO: 84 - DNA, 34 bp, synthetic construct
  misc_feature 1..34: note = synthetic nifF ribosome binding site (rbs, RBS) of full synthetic cluster
  source 1..34: mol_type = other DNA
gacaagagtctcaattataaggaggctttactac

SEQ ID NO: 85 - DNA, 534 bp, synthetic construct
  misc_feature 1..534: note = synthetic nifF of full synthetic cluster
  source 1..534: mol_type = other DNA
atggcgaacatcggcatcttctttggtacggataccggcaaaacccgcaagattgcgaagatgattcacaaacagctgggcgagctggccgatgccccggttaacatcaatcgtaccactttggatgactttatggcttacccagtcctgttgctcggcacgccgacgcttggtgatggtcaactgccgggcttagaggcgggctgcgagagcgaaagctggtctgagtttatctccggtctggatgacgcttccctgaagggcaaaaccgtggcgctgtttggcctgggcgaccagcgtggttacccggacaacttcgtgtcgggtatgcgtccgctgttcgacgcgctgagcgcccgtggcgcccagatgattggtagctggccgaacgaaggttatgagtttagcgcatcgtccgcgctggaaggcgaccgcttcgtcggcttggtgctggatcaagacaatcagttcgaccagaccgaagcgcgcctggcgtcttggcttgaagagatcaaacgcaccgttctgtaataa

SEQ ID NO: 86 - DNA, 29 bp, synthetic construct
  misc_feature 1..29: note = synthetic Enterobacteria phage T7 terminator 1 of full synthetic cluster
  source 1..29: mol_type = other DNA
tacatatcgggggggtaggggttttttgt

SEQ ID NO: 87 - DNA, 18 bp, synthetic construct
  misc_feature 1..18: note = synthetic insulator 10 of full synthetic cluster
  source 1..18: mol_type = other DNA
ggtcattacaacggttat

SEQ ID NO: 88 - DNA, 23 bp, synthetic construct
  misc_feature 1..23: note = synthetic Enterobacteria phage T7 promoter mut 2 of full synthetic cluster
  source 1..23: mol_type = other DNA
taatacgactcactagagagaga

SEQ ID NO: 89 - DNA, 40 bp, synthetic construct
  misc_feature 1..40: note = synthetic insulator 11 of full synthetic cluster
  source 1..40: mol_type = other DNA
aacatagcgttccatgagggctagaattacctaccggcct

SEQ ID NO: 90 - DNA, 37 bp, synthetic construct
  misc_feature 1..37: note = synthetic nifU ribosome binding site (rbs, RBS) of full synthetic cluster
  source 1..37: mol_type = other DNA
cagatactgacaaataaaccagcgaaggaggttccta

SEQ ID NO: 91 - DNA, 825 bp, synthetic construct; identical to SEQ ID NO: 16
  misc_feature 1..825: note = synthetic nifU of full synthetic cluster
  source 1..825: mol_type = other DNA

SEQ ID NO: 92 - DNA, 40 bp, synthetic construct
  misc_feature 1..40: note = synthetic insulator 12 of full synthetic cluster
  source 1..40: mol_type = other DNA
cattgtaatagccaccaaaagagtgatgatagtcatgggt

SEQ ID NO: 93 - DNA, 39 bp, synthetic construct
  misc_feature 1..39: note = synthetic nifS ribosome binding site (rbs, RBS) of full synthetic cluster
  source 1..39: mol_type = other DNA
gatacccgtagaccattctgaaatcgaaggaggttttcc

SEQ ID NO: 94 - DNA, 1203 bp, synthetic construct
  misc_feature 1..1203: note = synthetic nifS of full synthetic cluster
  source 1..1203: mol_type = other DNA
atgaaacaagtgtacctggacaacaacgcgaccacccgcctggacccgatggttctggaagcgatgatgccgtttctcacggatttctatggcaatccgtccagcatccatgacttcggcatcccggcacaagcggcgctggaacgtgcgcaccagcaagctgcggcactgctgggcgcagagtacccgtctgaaatcattttcacgagctgtgcgaccgaggccactgcaaccgccattgcgtcggccatcgcgttattgccggaacgccgcgaaatcatcacctcggtagtggagcacccggctacgctggcggcgtgcgagcacctggaacgccaaggctatcgcatccatcgcattgcggtggatagcgaaggtgcgctggacatggcccagttccgtgcagcgctctcgccgcgtgtcgcgttggtgagcgtgatgtgggccaacaacgaaaccggcgtgctgttcccgattggcgaaatggccgagcttgcccacgagcagggcgctctgttccactgcgatgccgttcaggtcgttggcaaaatcccaattgctgttggccagacgcgcatcgacatgctgtcttgctccgcgcacaagtttcatggtccgaagggtgttggttgcttgtacttacgtcgtggcacgcgctttcgtccgctgcttcgcggtggccatcaagaatatggtcgccgtgccggcactgagaatatctgtggcatcgtcggcatgggcgctgcgtgcgaactggcgaacatccatctgccgggtatgacccatattggccagttacgcaatcgcctggagcaccgtctgctcgccagcgtgccgtccgtgatggttatgggcggtggtcagccgcgtgtaccgggtactgtcaacctggcgttcgagtttatcgaaggtgaagcgatcctgctcttgctgaaccaggctggcattgccgcaagctccggctccgcgtgtacctctggcagcttggagccgagccatgtgatgcgcgccatgaacattccatacaccgcggctcacggcaccattcgttttagcctgagccgttatacgcgcgagaaagagatcgactacgtcgttgcgaccctcccgccaatcattgatcgtctgcgtgccttgtccccgtattggcagaatggtaagccgcgtccggcagatgcagtctttaccccggtttacggttaa

SEQ ID NO: 95 - DNA, 40 bp, synthetic construct
  misc_feature 1..40: note = synthetic insulator 13 of full synthetic cluster
  source 1..40: mol_type = other DNA
gagttactggccctgatttctccgcttctaataccgcaca

SEQ ID NO: 96 - DNA, 34 bp, synthetic construct
  misc_feature 1..34: note = synthetic nifV ribosome binding site (rbs, RBS) of full synthetic cluster
  source 1..34: mol_type = other DNA
gcgactaggagcctaactcgccacaaggaaacat

SEQ ID NO: 97 - DNA, 1143 bp, synthetic construct; identical to SEQ ID NO: 20
  misc_feature 1..1143: note = synthetic nifV of full synthetic cluster
  source 1..1143: mol_type = other DNA

SEQ ID NO: 98 - DNA, 40 bp, synthetic construct
  misc_feature 1..40: note = synthetic insulator 14 of full synthetic cluster
  source 1..40: mol_type = other DNA
gactcaacacgctagggacgtgaagtcgattccttcgatg

SEQ ID NO: 99 - DNA, 35 bp, synthetic construct
  misc_feature 1..35: note = synthetic nifW ribosome binding site (rbs, RBS) of full synthetic cluster
  source 1..35: mol_type = other DNA
cagaaggcgagaactagatttaagggccattatag

SEQ ID NO: 100 - DNA, 258 bp, synthetic construct; identical to SEQ ID NO: 22
  misc_feature 1..258: note = synthetic nifW of full synthetic cluster
  source 1..258: mol_type = other DNA

SEQ ID NO: 101 - DNA, 40 bp, synthetic construct
  misc_feature 1..40: note = synthetic insulator 15 of full synthetic cluster
  source 1..40: mol_type = other DNA
tcgagaaacaaggcagttccgggctgaaagtagcgccggg

SEQ ID NO: 102 - DNA, 36 bp, synthetic construct
  misc_feature 1..36: note = synthetic nifZ ribosome binding site (rbs, RBS) of full synthetic cluster
  source 1..36: mol_type = other DNA
acaagtcccgtattataaccgcctaggaggtgttgg

SEQ ID NO: 103 - DNA, 447 bp, synthetic construct; identical to SEQ ID NO: 24
  misc_feature 1..447: note = synthetic nifZ of full synthetic cluster
  source 1..447: mol_type = other DNA

SEQ ID NO: 104 - DNA, 40 bp, synthetic construct
  misc_feature 1..40: note = synthetic insulator 16 of full synthetic cluster
  source 1..40: mol_type = other DNA
acgccacgcgtagtgagacatacacgttcgttgggttcac

SEQ ID NO: 105 - DNA, 34 bp, synthetic construct
  misc_feature 1..34: note = synthetic nifM ribosome binding site (rbs, RBS) of full synthetic cluster
  source 1..34: mol_type = other DNA
tcagagactgaagttattacccaggaggtctata

SEQ ID NO: 106 - DNA, 801 bp, synthetic construct; identical to SEQ ID NO: 26
  misc_feature 1..801: note = synthetic nifM of full synthetic cluster
  source 1..801: mol_type = other DNA

SEQ ID NO: 107 - DNA, 47 bp, synthetic construct
  misc_feature 1..47: note = synthetic Enterobacteria phage T7 wild type (WT) terminator of full synthetic cluster
  source 1..47: mol_type = other DNA
tagcataaccccttggggcctctaaacgggtcttgaggggttttttg

SEQ ID NO: 108 - DNA, 21 bp, synthetic construct
  misc_feature 1..21: note = synthetic Biobrick suffix (BBa_G000001) of full synthetic cluster
  source 1..21: mol_type = other DNA
tactagtagcggccgctgcag

SEQ ID NO: 109 - DNA, 12 bp, synthetic construct
  misc_feature 1..12: note = synthetic translational stop (BBa_B0042) of full synthetic cluster
  source 1..12: mol_type = other DNA
ttagttagttag

SEQ ID NO: 110 - DNA, 69 bp, synthetic construct; identical to SEQ ID NO: 42
  misc_feature 1..69: note = synthetic terminator (BBa_B0054) of full synthetic cluster
  source 1..69: mol_type = other DNA

SEQ ID NO: 111 - DNA, 20 bp, synthetic construct
  misc_feature 1..20: note = synthetic VR primer (BBa_G00102) of full synthetic cluster
  source 1..20: mol_type = other DNA
gctcactcaaaggcggtaat

SEQ ID NO: 112 - DNA, 41 bp, synthetic construct; identical to SEQ ID NO: 44
  misc_feature 1..41: note = synthetic terminator (BBa_B0062) of full synthetic cluster
  source 1..41: mol_type = other DNA

SEQ ID NO: 113 - DNA, 2037 bp, synthetic construct
  misc_feature 1..2037: note = synthetic pSC101 origin (BBa_150042) of full synthetic cluster
  source 1..2037: mol_type = other DNA
ctgtcagaccaagtttacgagctcgcttggactcctgttgatagatccagtaatgacctcagaactccatctggatttgttcagaacgctcggttgccgccgggcgttttttattggtgagaatccaagcactagggacagtaagacgggtaagcctgttgatgataccgctgccttactgggtgcattagccagtctgaatgacctgtcacgggataatccgaagtggtcagactggaaaatcagagggcaggaactgctgaacagcaaaaagtcagatagcaccacatagcagacccgccataaaacgccctgagaagcccgtgacgggcttttcttgtattatgggtagtttccttgcatgaatccataaaaggcgcctgtagtgccatttacccccattcactgccagagccgtgagcgcagcgaactgaatgtcacgaaaaagacagcgactcaggtgcctgatggtcggagacaaaaggaatattcagcgatttgcccgagcttgcgagggtgctacttaagcctttagggttttaaggtctgttttgtagaggagcaaacagcgtttgcgacatccttttgtaatactgcggaactgactaaagtagtgagttatacacagggctgggatctattctttttatctttttttattctttctttattctataaattataaccacttgaatataaacaaaaaaaacacacaaaggtctagcggaatttacagagggtctagcagaatttacaagttttccagcaaaggtctagcagaatttacagatacccacaactcaaaggaaaaggacatgtaattatcattgactagcccatctcaattggtatagtgattaaaatcacctagaccaattgagatgtatgtctgaattagttgttttcaaagcaaatgaactagcgattagtcgctatgacttaacggagcatgaaaccaagctaattttatgctgtgtggcactactcaaccccacgattgaaaaccctacaaggaaagaacggacggtatcgttcacttataaccaatacgctcagatgatgaacatcagtagggaaaatgcttatggtgtattagctaaagcaaccagagagctgatgacgagaactgtggaaatcaggaatcctttggttaaaggctttgagattttccagtggacaaactatgccaagttctcaagcgaaaaattagaattagtttttagtgaagagatattgccttatcttttccagttaaaaaaattcataaaatataatctggaacatgttaagtcttttgaaaacaaatactctatgaggatttatgagtggttattaaaagaactaacacaaaagaaaactcacaaggcaaatatagagattagccttgatgaatttaagttcatgttaatgcttgaaaataactaccatgagtttaaaaggcttaaccaatgggttttgaaaccaataagtaaagatttaaacacttacagcaatatgaaattggtggttgataagcgaggccgcccgactgatacgttgattttccaagttgaactagatagacaaatggatctcgtaaccgaacttgagaacaaccagataaaaatgaatggtgacaaaataccaacaaccattacatcagattcctacctacgtaacggactaagaaaaacactacacgatgctttaactgcaaaaattcagctcaccagttttgaggcaaaatttttgagtgacatgcaaagtaagcatgatctcaatggttcgttctcatggctcacgcaaaaacaacgaaccacactagagaacatactggctaaatacggaaggatctgaggttcttatggctcttgtatctatcagtgaagcatcaagactaacaaacaaaagtagaacaactgttcaccgttagatatcaaagggaaaactgtccatatgcacagatgaaaacggtgtaaaaaagatagatacatcagagcttttacgagtttttggtgcatttaaagctgttcaccatgaacagatcgacaatgtaac

SEQ ID NO: 114 - DNA, 769 bp, synthetic construct
  misc_feature 1..769: note = synthetic chloramphenicol resistance (BBa_P1004) of full synthetic cluster
  source 1..769: mol_type = other DNA
gttgatcgggcacgtaagaggttccaactttcaccataatgaaataagatcactaccgggcgtattttttgagttatcgagattttcaggagctaaggaagctaaaatggagaaaaaaatcacgggatataccaccgttgatatatcccaatggcatcgtaaagaacattttgaggcatttcagtcagttgctcaatgtacctataaccagaccgttcagctggatattacggcctttttaaagaccgtaaagaaaaataagcacaagttttatccggcctttattcacattcttgcccgcctgatgaacgctcacccggagtttcgtatggccatgaaagacggtgagctggtgatctgggatagtgttcacccttgttacaccgttttccatgagcaaactgaaacgttttcgtccctctggagtgaataccacgacgatttccggcagtttctccacatatattcgcaagatgtggcgtgttacggtgaaaacctggcctatttccctaaagggtttattgagaatatgttttttgtctcagccaatccctgggtgagtttcaccagttttgatttaaacgtggccaatatggacaacttcttcgcccccgttttcacgatgggcaaatattatacgcaaggcgacaaggtgctgatgccgctggcgatccaggttcatcatgccgtttgtgatggcttccatgtcggccgcatgcttaatgaattacaacagtactgtgatgagtggcagggcggggcgtaataa

SEQ ID NO: 115 - DNA, 72 bp, synthetic construct; identical to SEQ ID NO: 47
  misc_feature 1..72: note = synthetic terminator (BBa_B0053) of full synthetic cluster
  source 1..72: mol_type = other DNA

SEQ ID NO: 116 - DNA, 20 bp, synthetic construct
  misc_feature 1..20: note = synthetic VF2 primer (BBa_G00101) of full synthetic cluster
  source 1..20: mol_type = other DNA
tgccacctgacgtctaagaa

SEQ ID NO: 117 - DNA, 78 bp, synthetic construct; identical to SEQ ID NO: 49
  misc_feature 1..78: note = synthetic terminator (BBa_B0055) of full synthetic cluster
  source 1..78: mol_type = other DNA

SEQ ID NO: 118 - DNA, 12 bp, synthetic construct
  misc_feature 1..12: note = synthetic translational stop (BBa_B0042) of full synthetic cluster
  source 1..12: mol_type = other DNA
ttagttagttag

SEQ ID NO: 119 - DNA, 19 bp, synthetic construct
  misc_feature 1..19: note = synthetic SynPrgH ribosome binding site (rbs, RBS) of bacterial type III secretion system (T3SS)
  source 1..19: mol_type = other DNA
attaaacaggataataagc

SEQ ID NO: 120 - DNA, 1182 bp, synthetic construct
  misc_feature 1..1182: note = synthetic SynPrgH of bacterial type III secretion system (T3SS)
  source 1..1182: mol_type = other DNA
atggaaactagcaaggagaaaacgattacgtcccctggtccgtatatcgttcgtctgttgaactcgtccctgaacggttgtgaatttccgctgctgactggtcgtacgctgttcgtcgtgggtcagagcgatgctctgaccgcgtctggtcagctgccggacattcctgccgactccttcttcatcccgctggatcatggcggtgttaatttcgagattcaagtggacactgacgcgacggaaatcatcctgcacgaactgaaagagggcaactccgagagccgctccgtgcaactgaacaccccgatccaagttggtgaactgctgattttgattcgtccggagagcgagccgtgggtgccggaacagccggagaagttggaaacttctgcgaaaaagaacgaaccgcgctttaaaaacggcatcgtcgcggcactggcgggtttctttatcctgggtatcggcacggttggcaccctgtggattctgaactcgccgcaacgtcaagcagccgaattggacagcctgttgggtcaggagaaggagcgttttcaggtgctgccgggtcgcgacaagatgctgtatgtcgccgcgcaaaacgaacgcgacaccctgtgggcacgtcaagtcctggcacgcggcgattacgataaaaacgcacgcgttattaatgaaaatgaggagaataaacgtatcagcatctggctggacacgtattatccacaactggcatattaccgtatccattttgatgaaccacgtaagccggtgttttggctgtcccgtcaacgcaacacgatgagcaagaaagagctggaggtgctgtcccagaaattgcgtgcgctgatgccgtacgccgacagcgtcaatattactctgatggatgacgtgaccgcagcaggccaagccgaggcaggtctgaaacaacaggcgctgccatacagccgccgtaaccacaaaggtggtgttacgttcgttattcagggcgccttggacgacgttgagattctgcgtgcgcgccagtttgtcgactcctattatcgtacctggggtggtcgttacgttcaattcgcaattgaattgaaagacgattggctgaaaggccgctcgttccaatacggtgcggaaggctacattaagatgagcccaggtcattggtattttccgtctcctctgtaatag

SEQ ID NO: 121 - DNA, 21 bp, synthetic construct
  misc_feature 1..21: note = synthetic SynPrgI ribosome binding site (rbs, RBS) of bacterial type III secretion system (T3SS)
  source 1..21: mol_type = other DNA
attaaagaggagaaattaagc

SEQ ID NO: 122 - DNA, 21 bp, synthetic construct
  misc_feature 1..21: note = synthetic SynPrgJ ribosome binding site (rbs, RBS) of bacterial type III secretion system (T3SS)
  source 1..21: mol_type = other DNA
attaaggaggataaattaagc

SEQ ID NO: 123 - DNA, 309 bp, synthetic construct
  misc_feature 1..309: note = synthetic SynPrgJ of bacterial type III secretion system (T3SS)
  source 1..309: mol_type = other DNA
atgtctatcgcgactatcgtgcctgaaaatgccgttattggtcaagcggtgaatattcgcagcatggaaacggacatcgtcagcttggacgaccgtttgctgcaagcattttcgggcagcgccatcgctaccgccgtcgataagcagaccattaccaatcgcattgaagaccctaatctggttaccgatccgaaggagctggcgattagccaggaaatgatttccgactacaatctgtacgtcagcatggttagcaccctgacgcgtaagggcgttggcgctgttgagactttgctgcgttcctgatag

SEQ ID NO: 124 - DNA, 19 bp, synthetic construct
  misc_feature 1..19: note = synthetic SynPrgK ribosome binding site (rbs, RBS) of bacterial type III secretion system (T3SS)
  source 1..19: mol_type = other DNA
attaaacaggataataagc

SEQ ID NO: 125 - DNA, 762 bp, synthetic construct
  misc_feature 1..762: note = synthetic SynPrgK of bacterial type III secretion system (T3SS)
  source 1..762: mol_type = other DNA
atgatccgccgttacctgtataccttcttgctggttatgactttggccggctgtaaagataaggatctgctgaaaggcttggaccaagagcaagcgaatgaggtcattgcggttctgcaaatgcacaacattgaggctaacaagattgatagcggcaagctgggttacagcattaccgtcgcggaaccggatttcaccgcggcagtgtattggattaagacctaccagttgccgcctcgcccgcgtgtcgaaatcgcccaaatgtttccggcagacagcctggttagctctccgcgtgcggagaaagcacgtctgtactcggcgattgaacagcgcctggagcagtcgctgcaaacgatggaaggtgttctgtcggcccgtgtccacatcagctatgatattgatgcgggcgagaacggtcgtccgcctaagccggtgcacctgtcggctttggcggtgtatgaacgcggttcccctctggcccatcagatttcggatattaagcgcttcctgaaaaacagcttcgcggatgttgactatgataacatcagcgtggttctgtccgagcgtagcgacgcacagttgcaggcgccgggcacgccggtcaagcgcaatagcttcgctacctcctggattgtgctgattatcctgttgtctgttatgagcgcgggtttcggtgtctggtactacaaaaatcactatgcgcgtaataagaaaggcattactgccgatgacaaggcaaagtccagcaacgagtaataa

SEQ ID NO: 126 - DNA, 19 bp, synthetic construct
  misc_feature 1..19: note = synthetic SynOrgA ribosome binding site (rbs, RBS) of bacterial type III secretion system (T3SS)
  source 1..19: mol_type = other DNA
gaaagaagggacagactag

SEQ ID NO: 127 - DNA, 603 bp, synthetic construct
  misc_feature 1..603: note = synthetic SynOrgA of bacterial type III secretion system (T3SS)
  source 1..603: mol_type = other DNA
atgattcgtcgtaaccgtcaaatgaaccgtcaaccactgccaattatctggcaacgcattattttcgacccactgtcctatattcacccacaacgtctgcaaatcgcgccggagatgatcgtgcgtccggcagcgcgtgcggcagcgaatgagctgattttggcggcgtggcgtttgaagaacggtgagaaggagtgcattcagaatagcctgacgcagctgtggttgcgtcaatggcgccgtctgccgcaggttgcttacctgctgggttgccacaagttgcgtgctgacctggcccgtcaaggtgctttattgggcctgccggactgggcgcaggcattcttggcgatgcaccagggtacgtccttgtcggtttgtaataaggcgccgaaccaccgtttcctgctgtccgttggttacgcccaactgaacgcgctgaatgagttcctgccggagagcttggcccaacgctttcctctgctgtttccaccgttcatcgaggaggcactgaaacaagatgcagtggagatgagcatcctgctgctggccctgcaatacgcgcaaaagtatcctaacaccgtcccggcgtttgcgtgctaataa

SEQ ID NO: 128 - DNA, 19 bp, synthetic construct
  misc_feature 1..19: note = synthetic SynOrgB ribosome binding site (rbs, RBS) of bacterial type III secretion system (T3SS)
  source 1..19: mol_type = other DNA
gaaagaagggacagactag

SEQ ID NO: 129 - DNA, 684 bp, synthetic construct
  misc_feature 1..684: note = synthetic SynOrgB of bacterial type III secretion system (T3SS)
  source 1..684: mol_type = other DNA
atgttgaaaaatatcccgattccatcccctctgtctccggttgaaggtatcctgattaaacgcaagacgttggagcgttacttctcgattgagcgcctggaacaacaggcgcatcagcgtgcaaagcgcattttgcgtgaggcagaagaagaagccaagaccctgcgcatgtatgcgtaccaggagggctacgagcagggcatgattgacgcactgcaacaggtggccgcctatttgaccgacaaccagacgatggcttggaaatggatggagaaaattcaaatctatgcgcgtgagttgttcagcgcggctgtcgatcacccggaaacgttgttgacggtgctggacgagtggctgcgtgatttcgataagccggaaggtcagctgtttttgaccctgccggtgaacgcaaagaaagatcatcagaaactgatggtgctgctgatggaaaattggccgggcaccttcaatctgaagtatcatcaggagcaacgttttatcatgtcctgtggcgatcagattgccgagttttcgccggaacaatttgttgaaacggcggttggtgttatcaagcaccatctggatgagctgcctcaggactgtcgcaccatttcggacaatgcgattaacgcgctgattgatgaatggaagacgaaaacccaagctgaagttattcgctgataa

SEQ ID NO: 130 - DNA, 36 bp, synthetic construct
  misc_feature 1..36: note = synthetic SynInvA ribosome binding site (rbs, RBS) of bacterial type III secretion system (T3SS)
  source 1..36: mol_type = other DNA
cttgggcacgcgtccattaaacaggagtaattaagc

SEQ ID NO: 131 - DNA, 2058 bp, synthetic construct
  misc_feature 1..2058: note = synthetic SynInvA of bacterial type III secretion system (T3SS)
  source 1..2058: mol_type = other DNA
atgctgctgtccctgctgaatagcgcgcgtctgcgtcctgagctgctgattctggttctgatggttatgatcatcagcatgttcgttatcccgttgccgacctatttggttgacttcttgatcgctttgaacattgtcctggcaattctggtgttcatgggctccttctacatcgaccgcattctgagcttcagcacctttccggcggttctgctgatcacgactctgttccgtttggcactgagcatcagcaccagccgcctgatcctgattgaagcagatgcgggtgagatcatcgcgacctttggtcagtttgtgatcggtgacagcctggcggttggtttcgtcgtattctccatcgtgacggtggtgcagtttatcgttattaccaagggcagcgaacgtgtggcggaggtcgccgctcgcttcagcctggacggcatgccgggtaaacagatgtctattgatgcagacctgaaagccggcattattgatgctgatgcagcgcgcgagcgccgcagcgtcctggagcgtgaaagccaactgtacggttccttcgacggtgccatgaagttcattaaaggtgatgcgattgcgggcatcattatcatcttcgttaacttcattggcggtatcagcgtcggtatgacccgtcatggtatggatctgagcagcgccctgagcacctacaccatgctgacgattggtgatggtctggttgcccaaattccggcgttgctgatcgcgatttctgcgggcttcatcgttacccgcgtcaacggtgatagcgataacatgggtcgtaacattatgacccagctgctgaataatccgtttgtcctggttgtaacggcgattttgaccatcagcatgggcacgctgccgggctttccgttgccggttttcgttattctgtctgttgtgctgtccgtcctgttttactttaagttccgcgaggcgaaacgtagcgctgcgaaaccaaaaacgagcaagggcgagcaaccgttgtccatcgaggagaaggaaggtagcagcctgggcctgattggcgacctggataaggttagcacggaaaccgtcccgctgattttgctggtgccgaaatcgcgtcgtgaggatctggagaaagcgcagctggcggaacgtctgcgcagccaattctttattgattatggtgtgcgtctgccagaagtactgctgcgtgacggtgagggtctggatgacaactctatcgtcctgctgattaatgagattcgcgttgaacagtttactgtctattttgacctgatgcgtgtggttaactacagcgacgaggtggtgagctttggcatcaacccgaccattcaccagcaaggttccagccagtacttttgggtgacccatgaggaaggcgaaaagctgcgcgagctgggctacgtcctgcgtaatgcactggacgaactgtaccactgtctggcggtgacgctggcacgcaatgtgaacgagtatttcggtatccaagaaacgaaacacatgctggaccaactggaagcaaagtttcctgacctgctgaaggaggttttgcgccacgccaccgtgcagcgcatttcggaagtgctgcaacgtctgctgtccgaacgcgtgagcgtccgtaacatgaagctgatcatggaagccctggcactgtgggctccgcgtgagaaagatgtgatcaatctggtggagcacatccgtggtgcgatggcgcgttatatctgccacaagttcgcaaatggtggtgaactgcgtgccgttatggtttccgccgaagttgaggatgtcattcgtaaaggcattcgtcaaacttctggctccacctttttgagcttggacccggaggcttcggcaaatctgatggacctgatcacgctgaagctggacgacctgttgattgcgcataaggacctggtcctgttgaccagcgttgacgtgcgtcgttttatcaagaaaatgattgaaggtcgttttccggatctggaggtcctgtccttcggtgagattgcagatagcaaaagcgtgaatgtcatcaaaaccatctga

SEQ ID NO: 132 - DNA, 36 bp, synthetic construct
  misc_feature 1..36: note = synthetic SynInvC ribosome binding site (rbs, RBS) of bacterial type III secretion system (T3SS)
  source 1..36: mol_type = other DNA
cttgggcacgcgtccattaaagaggaccaattaagc

SEQ ID NO: 133 - DNA, 1296 bp, synthetic construct
  misc_feature 1..1296: note = synthetic SynInvC of bacterial type III secretion system (T3SS)
  source 1..1296: mol_type = other DNA
atgaaaaccccacgtctgctgcaatacctggcctacccgcagaaaatcactggccctatcattgaagcagaactgcgtgatgttgcaattggtgaattgtgcgagatccgtcgcggctggcaccagaagcaggttgtggcccgtgcgcaagtggttggtttgcagcgcgaacgtaccgtcctgagcctgatcggcaatgcccaaggcctgagccgtgatgtggtcttgtacccgaccggccgtgctctgagcgcgtgggttggttacagcgttctgggcgcagtactggacccgacgggtaaaatcgttgaacgtttcaccccggaagtcgcaccgatttccgaggagcgcgttatcgacgtggcaccgccgagctacgcaagccgtgtcggtgtgcgcgaaccgctgatcacgggtgtccgcgcaattgatggtctgctgacgtgtggtgtgggccagcgtatgggtattttcgcaagcgcgggttgtggtaagaccatgttgatgcacatgctgatcgagcaaaccgaagcggatgtctttgttattggcctgattggcgagcgtggtcgtgaagttaccgaatttgtagacatgttgcgtgcatctcataagaaagaaaaatgtgtgctggtttttgccacgtccgacttcccaagcgttgaccgctgcaacgctgcccagctggcaacgacggtcgccgagtatttccgcgaccagggtaaacgtgttgtcctgtttatcgacagcatgacccgttatgcacgcgcgttgcgtgatgtcgcgctggcgagcggcgagcgtccggctcgccgtggttatccggcgtctgtgttcgacaatctgccgcgtttgctggagcgtccgggtgcgacgagcgagggtagcattaccgccttctataccgtcctgctggagtcggaagaagaagcggacccgatggcggacgagatccgttctattctggacggtcacctgtacctgtcccgcaaactggcgggtcagggtcattacccggctatcgatgtgctgaagagcgtgagccgtgtgtttggtcaagtgaccaccccgactcacgcggagcaagcgagcgcggtccgtaagctgatgacccgtctggaagagctgcaactgttcattgacctgggcgagtatcgtccgggcgagaacattgacaatgatcgtgcgatgcaaatgcgcgatagcctgaaggcgtggctgtgtcagcctgttgcgcaatacagcagcttcgatgatacgctgtccggcatgaacgcctttgcggatcagaactga

SEQ ID NO: 134 - DNA, 36 bp, synthetic construct
  misc_feature 1..36: note = synthetic SynInvE ribosome binding site (rbs, RBS) of bacterial type III secretion system (T3SS)
  source 1..36: mol_type = other DNA
tacttgggcacgcgtccattaattaggatcaatagc

SEQ ID NO: 135 - DNA, 1119 bp, synthetic construct
  misc_feature 1..1119: note = synthetic SynInvE of bacterial type III secretion system (T3SS)
  source 1..1119: mol_type = other DNA
atgattccgggcagcacctccggtatttcctttagccgtatcctgagccgtcagacctcccaccaggatgcaacccagcataccgacgcacaacaagcggaaattcaacaagcggcggaagatagctcgccgggtgcggaggttcagaaattcgtccagagcacggacgagatgtctgctgcgttggcgcagttccgcaatcgccgtgactatgagaaaaagagcagcaatttgtctaactccttcgagcgcgttctggaggacgaggcactgccgaaagcgaagcagattctgaaactgatcagcgtgcatggcggtgcgttggaggatttcctgcgtcaggcgcgcagcctgttcccggacccaagcgatctggtgctggttctgcgcgagctgttgcgtcgtaaggacctggaggagatcgtgcgtaagaagctggagagcctgctgaagcacgtggaggaacaaaccgacccgaaaaccctgaaggccggtattaactgcgcgctgaaggcgcgtctgtttggcaagacgctgtctctgaaacctggtctgctgcgtgccagctaccgccagttcatccaaagcgaaagccacgaagtcgagatttacagcgattggatcgccagctacggttatcagcgtcgcctggttgttctggatttcattgaaggcagcctgctgactgacatcgatgctaacgatgcaagctgctcccgtctggagtttggccaactgctgcgccgtctgacccagctgaaaatgttgcgtagcgccgacctgctgtttgtctcgacgttgctgtcttacagcttcacgaaagcatttaacgctgaggagagcagctggctgttgctgatgctgtctttgctgcaacagccgcacgaagtggatagcctgctggcggacattatcggtctgaatgcgctgctgttgtcccacaaagagcacgccagcttcctgcaaatcttctatcaggtctgtaaggcaatcccgtctagcctgttttatgaagagtactggcaagaagaactgctgatggcactgcgctccatgacggacattgcttacaaacacgaaatggccgaacaacgtcgtaccatcgaaaagctgtcctaa

SEQ ID NO: 136 - DNA, 36 bp, synthetic construct
  misc_feature 1..36: note = synthetic SynInvF ribosome binding site (rbs, RBS) of bacterial type III secretion system (T3SS)
  source 1..36: mol_type = other DNA
cttgggcacgcgtccattaaaaaggagtaattaagc

SEQ ID NO: 137 - DNA, 651 bp, synthetic construct
  misc_feature 1..651: note = synthetic SynInvF of bacterial type III secretion system (T3SS)
  source 1..651: mol_type = other DNA
atgagcttcagcgagagccgccacaatgaaaactgtctgattcaagaaggcgcactgctgttttgtgagcaagcagtcgtggcgcctgtcagcggtgatctggtttttcgtccgctgaaaatcgaggtcctgagcaagctgctggcgttcatcgacggcgcaggtctggtggatacgacctacgcggagtcggacaaatgggttctgctgtctccggagttccgtgctatttggcaagaccgtaaacgttgcgaatattggtttttgcagcagattatcaccccatctccggcgttcaacaaggttctggcactgttgcgtaagagcgaaagctattggttggtcggctacttgctggcccaaagcaccagcggcaatactatgcgtatgttgggtgaggattacggtgttagctacacgcatttccgccgtctgtgcagccgcgctctgggcggtaaggcgaaaagcgagctgcgcaattggcgcatggcccagtccctgctgaatagcgtggaaggtcatgaaaacatcacccagctggcggtcaaccacggttatagcagcccgtcccactttagctctgaaatcaaggagctgattggtgtttccccgcgtaagctgtctaacatcattcagctggccgacaaatga

SEQ ID NO: 138 - DNA, 36 bp, synthetic construct
  misc_feature 1..36: note = synthetic SynInvG ribosome binding site (rbs, RBS) of bacterial type III secretion system (T3SS)
  source 1..36: mol_type = other DNA
tgggcacgcgtccattaatgaggaaaaattattagc

SEQ ID NO: 139 - DNA, 1689 bp, synthetic construct
  misc_feature 1..1689: note = synthetic SynInvG of bacterial type III secretion system (T3SS)
  source 1..1689: mol_type = other DNA
atgaaaacgcacattctgttggcccgtgtgctggcttgcgcagctctggtgctggtcaccccaggttatagctccgagaagatcccggttacgggcagcggcttcgttgcaaaggacgattctctgcgcacctttttcgatgcgatggcactgcaattgaaggagccggtgattgtcagcaagatggcggctcgcaaaaagattaccggcaatttcgagttccacgatccaaacgcgctgctggagaaactgtccctgcaactgggtctgatctggtactttgatggtcaggcgatctacatctacgacgcgagcgaaatgcgtaatgcggttgtgagcctgcgtaatgtcagcctgaacgagttcaacaattttctgaagcgcagcggcctgtacaataagaactaccctctgcgtggtgataatcgtaaaggcaccttctatgtcagcggtccgccggtgtatgttgatatggttgtaaatgcggccaccatgatggacaaacagaatgatggcatcgagctgggtcgccaaaagatcggtgttatgcgcctgaacaacacttttgtgggcgaccgcacctacaacctgcgtgatcaaaagatggtcattccgggtattgctacggcaattgaacgcctgttgcaaggcgaagaacaaccgctgggtaacattgtaagctccgagcctccggccatgccggcctttagcgcaaacggcgagaaaggtaaggcagcgaattacgcgggtggtatgagcctgcaagaagcgctgaaacagaacgcagcggcaggcaacatcaaaattgtggcctatccggacaccaacagcctgctggtgaaaggtacggcggagcaggtgcatttcatcgagatgctggttaaagccctggacgtggcgaaacgtcacgttgaattgagcctgtggattgtggatttgaataagagcgacctggaacgcttgggcaccagctggagcggtagcatcaccatcggcgacaagctgggtgtgagcctgaaccagagcagcatctccacgctggacggtagccgctttattgcggcggtcaacgctctggaggaaaagaaacaggccactgttgtcagccgtccggttctgctgacccaggagaatgtcccggcgatttttgacaataatcgtactttctataccaaactgatcggtgaacgtaatgttgcattggaacacgtgacctatggcaccatgatccgtgtcctgccgcgtttcagcgcggacggccagattgagatgagcctggacatcgaagatggtaatgacaaaaccccgcagtctgatacgaccacctccgttgatgcgctgccagaagtgggtcgtaccctgatctcgacgattgcacgtgtcccgcatggtaaatctctgctggttggtggctacacgcgtgatgcaaacacggacacggtccaaagcatcccgttcctgggtaagctgccgctgattggctcgttgtttcgctacagcagcaaaaacaagtctaatgtcgtccgtgtctttatgattgagccgaaagaaatcgttgacccgctgaccccggatgccagcgagagcgttaacaacattctgaaacagtccggtgcgtggagcggtgacgataagctgcaaaagtgggttcgtgtgtatttggaccgtggtcaggaggccattaagtaa

SEQ ID NO: 140 - DNA, 36 bp, synthetic construct
  misc_feature 1..36: note = synthetic SynInvI ribosome binding site (rbs, RBS) of bacterial type III secretion system (T3SS)
  source 1..36: mol_type = other DNA
cttgggcacgcgtccattaaaaaggaccaattaagc

SEQ ID NO: 141 - DNA, 444 bp, synthetic construct
  misc_feature 1..444: note = synthetic SynInvI of bacterial type III secretion system (T3SS)
  source 1..444: mol_type = other DNA
atgcactctctgactcgtatcaaggtcctgcaacgtcgttgtaccgtgttccattctcagtgcgagtccattctgttgcgttatcaggacgaagatcgcggcttgcaggcggaggaggaggccatcctggaacagatcgcaggtctgaaactgctgttggacaccctgcgtgctgaaaatcgtcaactgagccgtgaagaaatctatacgctgctgcgcaaacagagcattgttcgtcgccagattaaggatctggagctgcaaatcattcagattcaagaaaagcgtagcgagctggaaaagaaacgtgaggaatttcaaaagaaaagcaaatactggctgcgtaaagaaggtaactaccagcgctggattatccgtcaaaaacgcttctacattcaacgtgagatccagcaagaggaggcggagagcgaagagatcatttaa

SEQ ID NO: 142 - DNA, 36 bp, synthetic construct
  misc_feature 1..36: note = synthetic SynInvJ ribosome binding site (rbs, RBS) of bacterial type III secretion system (T3SS)
  source 1..36: mol_type = other DNA
aaaaaaaagctctaaaagattaagagggggtaacat

SEQ ID NO: 143 - DNA, 1011 bp, synthetic construct
  misc_feature 1..1011: note = synthetic SynInvJ of bacterial type III secretion system (T3SS)
  source 1..1011: mol_type = other DNA
atgggtgacgtgagcgcggtgagcagcagcggtaacattctgctgccgcagcaggacgaggttggtggcctgtccgaagcgctgaagaaagcggttgaaaaacacaaaaccgaatacagcggtgacaagaaagatcgtgattatggtgacgcctttgttatgcacaaggaaaccgcgctgccgttgttgctggcagcttggcgccacggcgcaccggcgaaaagcgagcaccataacggtaacgtaagcggtctgcatcacaacggtaagagcgagctgcgtattgctgagaaactgctgaaggtgacggcggagaagagcgttggtctgattagcgctgaagcgaaggtggataaatctgcggcgctgctgtctagcaagaatcgtccgctggaatcggtcagcggcaaaaagttgtccgccgatctgaaagcagtggagtccgtgtccgaggtcacggataacgccaccggcatttcggatgacaacatcaaagcattgccgggtgacaataaggccatcgccggtgagggtgtgcgtaaagaaggtgcgccgctggcgcgtgacgtggctccggcacgcatggcggcagcaaatacgggcaagccggaggataaagaccacaagaaggtcaaggacgttagccagctgccgctgcaaccgactaccatcgccgatctgtctcaactgacgggtggcgatgaaaagatgccgctggcagcgcagtccaaaccgatgatgaccattttcccaaccgccgacggcgttaaaggtgaggacagctctctgacctatcgtttccagcgctggggcaacgattactccgtcaatatccaggcacgccaagcgggcgaatttagcctgattcctagcaatacccaggttgaacatcgtctgcacgaccaatggcaaaatggcaatccacaacgctggcatttgacgcgtgatgaccagcaaaacccgcaacagcaacagcatcgtcagcagtccggtgaagaggacgacgcgtaa

SEQ ID NO: 144 - DNA, 36 bp, synthetic construct
  misc_feature 1..36: note = synthetic SynSpaO ribosome binding site (rbs, RBS) of bacterial type III secretion system (T3SS)
  source 1..36: mol_type = other DNA
cttgggcacgcgtccatgaaagacaggacccactag

SEQ ID NO: 145 - DNA, 912 bp, synthetic construct
  misc_feature 1..912: note = synthetic SynSpaO of bacterial type III secretion system (T3SS)
  source 1..912: mol_type = other DNA
atgagcttgcgcgtacgccaaattgaccgccgtgaatggctgctggcccagactgcgaccgaatgtcagcgtcacggtcgtgaggccaccctggagtatccgacccgtcagggtatgtgggtccgcctgtctgatgccgaaaaacgctggtctgcgtggatcaaaccgggtgattggttggaacacgttagcccagcactggcgggtgccgcggtcagcgcaggcgcggagcacctggtggttccgtggctggcggcaaccgaacgcccgttcgagctgccggtcccgcacttgagctgccgtcgtctgtgcgtggagaacccggttccgggttccgcactgcctgagggcaagctgctgcacatcatgtcggatcgtggtggcctgtggtttgagcatctgccggagctgccggctgttggcggtggccgtccgaagatgctgcgttggccgctgcgtttcgttattggcagcagcgacacccagcgcagcctgctgggtcgtatcggtatcggtgatgttctgctgatccgcaccagccgtgctgaggtttactgttacgcgaagaaactgggccactttaatcgtgtggaaggtggcattattgtcgaaacgctggacattcaacatatcgaggaggagaacaacacgacggaaacggcggaaaccctgccgggtctgaatcaactgccggtgaagctggagttcgttctgtatcgtaaaaacgtgacgttggccgaactggaagcaatgggtcagcaacaactgctgtccttgccaaccaatgcggaactgaacgtcgaaatcatggcgaatggcgtgctgctgggtaacggcgaactggtgcagatgaatgacaccctgggtgtcgagattcatgagtggttgtccgagagcggtaatggcgagtag

SEQ ID NO: 146 - DNA, 36 bp, synthetic construct
  misc_feature 1..36: note = synthetic SynSpaP ribosome binding site (rbs, RBS) of bacterial type III secretion system (T3SS)
  source 1..36: mol_type = other DNA
cttgggcacgcgtccatgaaagaaacgacatactag

SEQ ID NO: 147 - DNA, 675 bp, synthetic construct
  misc_feature 1..675: note = synthetic SynSpaP of bacterial type III secretion system (T3SS)
  source 1..675: mol_type = other DNA
atgggtaacgatattagcttgattgcattgctggcgttttccaccctgctgccgttcatcatcgcgtctggtacttgcttcgtcaaattcagcatcgtctttgtgatggtgcgcaacgcgctgggtctgcaacaaattccaagcaatatgaccctgaatggcgtcgcactgctgctgtcgatgtttgttatgtggccgattatgcacgacgcgtatgtgtatttcgaggatgaagatgtgacctttaacgacatctccagcctgagcaagcatgttgatgagggcctggacggttatcgcgactacctgatcaagtattccgaccgtgagctggtgcagttctttgagaatgcccagttgaaacgtcagtacggtgaagaaacggaaaccgttaaacgtgacaaggacgagattgaaaagccgagcattttcgcactgttgcctgcttacgccttgagcgagattaagagcgcattcaaaattggtttttacctgtacctgccgttcgttgtggtcgatctggttgtctccagcgttctgctggccctgggcatgatgatgatgtccccggttaccatcagcacgccgatcaaactggtcctgtttgtggccctggatggttggacgctgctgtctaaaggcctgatcctgcaatacatggacatcgcgacctaa

SEQ ID NO: 148 - DNA, 36 bp, synthetic construct
  misc_feature 1..36: note = synthetic SynSpaQ ribosome binding site (rbs, RBS) of bacterial type III secretion system (T3SS)
  source 1..36: mol_type = other DNA
cttgggcacgcgtccattaagaaggaggaattaagc

SEQ ID NO: 149 - DNA, 261 bp, synthetic construct
  misc_feature 1..261: note = synthetic SynSpaQ of bacterial type III secretion system (T3SS)
  source 1..261: mol_type = other DNA
atggacgatctggttttcgccggcaacaaagccctgtacttggtgctgattctgtccggttggccgacgattgtcgcaaccattatcggtctgctggttggtctgtttcaaaccgtgacgcagttgcaggagcaaaccctgccgttcggtatcaagctgctgggtgtgtgtctgtgcctgtttttgctgtctggctggtatggcgaagttctgctgtcctacggccgtcaggtcatcttcctggctctggcgaaaggttaa

SEQ ID NO: 150 - DNA, 36 bp, synthetic construct; identical to SEQ ID NO: 144
  misc_feature 1..36: note = synthetic SynSpaR ribosome binding site (rbs, RBS) of bacterial type III secretion system (T3SS)
  source 1..36: mol_type = other DNA

SEQ ID NO: 151 - DNA, 792 bp, synthetic construct
  misc_feature 1..792: note = synthetic SynSpaR of bacterial type III secretion system (T3SS)
  source 1..792: mol_type = other DNA
atgttctatgcattgtattttgagatccaccatctggtggcgtccgcggctctgggttttgcgcgtgttgctccgatctttttctttctgccgttcctgaatagcggtgtcctgagcggtgctccgcgcaacgcgatcatcattctggtggcgctgggtgtatggccgcacgccctgaatgaggcgccaccgtttctgtctgtggcaatgattccgctggtcctgcaagaggcagccgtgggtgttatgctgggttgcctgttgtcctggccgttttgggttatgcacgcgttgggctgtatcattgataaccaacgcggtgcaaccctgtccagcagcattgatcctgcgaatggcatcgacaccagcgagatggccaatttcctgaacatgttcgcggctgtcgtgtatttgcagaacggtggcttggtcacgatggtggacgtgctgaataagtcttaccagctgtgtgatccgatgaacgagtgtacgccgagcctgcctccgttgctgaccttcattaatcaagtggcccagaacgcactggtgctggcgtccccggtcgttctggttctgctgctgtcggaagttttcctgggcctgctgtctcgttttgcaccgcaaatgaacgcgttcgccattagcctgactgttaaaagcggtattgcggttttgatcatgctgctgtatttcagcccggtcctgccggacaatgttctgcgtctgagctttcaggcgaccggcctgagcagctggttctacgaacgtggcgcaacgcatgtgctggaataa

SEQ ID NO: 152 - DNA, 36 bp, synthetic construct; identical to SEQ ID NO: 144
  misc_feature 1..36: note = synthetic SynSpaS ribosome binding site (rbs, RBS) of bacterial type III secretion system (T3SS)
  source 1..36: mol_type = other DNA

SEQ ID NO: 153 - DNA, 1071 bp, synthetic construct
  misc_feature 1..1071: note = synthetic SynSpaS of bacterial type III secretion system (T3SS)
  source 1..1071: mol_type = other DNA
atgtccagcaacaaaaccgaaaaaccgactaagaaacgtctggaggatagcgcaaagaaaggtcagagcttcaagagcaaggacctgattatcgcgtgcctgaccctgggtggtatcgcttatttggtgagctacggcagcttcaatgagtttatgggtatcattaagattatcatcgctgataactttgatcagtcgatggcagattatagcctggccgtgtttggtattggcctgaaatacctgattccgttcatgctgctgtgtttggtttgttccgcactgccggcactgctgcaagcgggcttcgttctggcaaccgaggccctgaagccgaatctgtccgccctgaacccggttgaaggcgcgaagaaactgttttccatgcgcaccgtcaaagacacggtcaagacgctgctgtatctgtcgagctttgtggttgcggcaatcatttgctggaaaaagtataaagtcgagattttcagccaactgaacggtaatatcgtgggtattgcggttatctggcgtgaattgctgctggcgttggttctgacctgtctggcgtgcgcgctgatcgtgctgttgctggatgctattgccgagtactttctgaccatgaaagatatgaagatggacaaagaagaagttaaacgcgagatgaaagagcaggagggtaacccggaggtgaagtctaaacgtcgtgaagtccacatggaaatcctgagcgaacaagtcaagtctgacattgaaaatagccgtctgattgtggcaaaccctacgcatattaccatcggcatctacttcaaaccggaactgatgccgattccaatgattagcgtctatgaaaccaatcaacgcgcgctggcggtccgtgcgtacgccgagaaagtgggtgttccggttattgtagacatcaagctggcgcgcagcctgttcaaaacgcaccgtcgttacgacctggtgagcctggaggagatcgacgaggttttgcgcctgctggtttggttggaagaggtcgaaaacgcaggcaaggatgtgatccaaccgcaggagaatgaagtgcgtcattaa

SEQ ID NO: 154 - DNA, 4075 bp, synthetic construct
  misc_feature 1..4075: note = synthetic Syn_PrgOrg operon of bacterial type III secretion system (T3SS)
  source 1..4075: mol_type = other DNA
gcatgcattaaagaggagaaattaagcatggctactccgtggtctggttatctggatgatgtttctgcaaaatttgacacgggtgttgacaacttgcaaacccaagttaccgaagccctggacaagctggctgcgaagccgtccgatccggcgctgctggcggcgtatcaatccaaactgtctgagtataacttgtaccgtaatgcgcagtcgaacacggtcaaggtcttcaaagatattgatgcagcgattattcagaactttcgttagtaacctaggattaaggaggataaattaagcatgtctatcgcgactatcgtgcctgaaaatgccgttattggtcaagcggtgaatattcgcagcatggaaacggacatcgtcagcttggacgaccgtttgctgcaagcattttcgggcagcgccatcgctaccgccgtcgataagcagaccattaccaatcgcattgaagaccctaatctggttaccgatccgaaggagctggcgattagccaggaaatgatttccgactacaatctgtacgtcagcatggttagcaccctgacgcgtaagggcgttggcgctgttgagactttgctgcgttcctgataggctagcattaaacaggataataagcatggaaactagcaaggagaaaacgattacgtcccctggtccgtatatcgttcgtctgttgaactcgtccctgaacggttgtgaatttccgctgctgactggtcgtacgctgttcgtcgtgggtcagagcgatgctctgaccgcgtctggtcagctgccggacattcctgccgactccttcttcatcccgctggatcatggcggtgttaatttcgagattcaagtggacactgacgcgacggaaatcatcctgcacgaactgaaagagggcaactccgagagccgctccgtgcaactgaacaccccgatccaagttggtgaactgctgattttgattcgtccggagagcgagccgtgggtgccggaacagccggagaagttggaaacttctgcgaaaaagaacgaaccgcgctttaaaaacggcatcgtcgcggcactggcgggtttctttatcctgggtatcggcacggttggcaccctgtggattctgaactcgccgcaacgtcaagcagccgaattggacagcctgttgggtcaggagaaggagcgttttcaggtgctgccgggtcgcgacaagatgctgtatgtcgccgcgcaaaacgaacgcgacaccctgtgggcacgtcaagtcctggcacgcggcgattacgataaaaacgcacgcgttattaatgaaaatgaggagaataaacgtatcagcatctggctggacacgtattatccacaactggcatattaccgtatccattttgatgaaccacgtaagccggtgttttggctgtcccgtcaacgcaacacgatgagcaagaaagagctggaggtgctgtcccagaaattgcgtgcgctgatgccgtacgccgacagcgtcaatattactctgatggatgacgtgaccgcagcaggccaagccgaggcaggtctgaaacaacaggcgctgccatacagccgccgtaaccacaaaggtggtgttacgttcgttattcagggcgccttggacgacgttgagattctgcgtgcgcgccagtttgtcgactcctattatcgtacctggggtggtcgttacgttcaattcgcaattgaattgaaagacgattggctgaaaggccgctcgttccaatacggtgcggaaggctacattaagatgagcccaggtcattggtattttccgtctcctctgtaatagaagcttattaaacaggataataagcatgatccgccgttacctgtataccttcttgctggttatgactttggccggctgtaaagataaggatctgctgaaaggcttggaccaagagcaagcgaatgaggtcattgcggttctgcaaatgcacaacattgaggctaacaagattgatagcggcaagctgggttacagcattaccgtcgcggaaccggatttcaccgcggcagtgtattggattaagacctaccagttgccgcctcgcccgcgtgtcgaaatcgcccaaatgtttccggcagacagcctggttagctctccgcgtgcggagaaagcacgtctgtactcggcgattgaacagcgcctggagcagtcgctgcaaacgatggaaggtgttctgtcggcccgtgtccacatcagctatgatattgatgcgggcgagaacggtcgtccgcctaagccggtgcacctgtcggctttggcggtgtatgaacgcggttcccctctggcccatcagatttcggatattaagcgcttcctgaaaaacagcttcgcggatgttgactatgataacatcagcgtggttctgtccgagcgtagcgacgcacagttgcaggcgccgggcacgccggtcaagcgcaatagcttcgctacctcctggattgtgctgattatcctgttgtctgttatgagcgcgggtttcggtgtctggtactacaaaaatcactatgcgcgtaataagaaaggcattactgccgatgacaaggcaaagtccagcaacgagtaataaggtaccgaaagaagggacagactagatgattcgtcgtaaccgtcaaatgaaccgtcaaccactgccaattatctggcaacgcattattttcgacccactgtcctatattcacccacaacgtctgcaaatcgcgccggagatgatcgtgcgtccggcagcgcgtgcggcagcgaatgagctgattttggcggcgtggcgtttgaagaacggtgagaaggagtgcattcagaatagcctgacgcagctgtggttgcgtcaatggcgccgtctgccgcaggttgcttacctgctgggttgccacaagttgcgtgctgacctggcccgtcaaggtgctttattgggcctgccggactgggcgcaggcattcttggcgatgcaccagggtacgtccttgtcggtttgtaataaggcgccgaaccaccgtttcctgctgtccgttggttacgcccaactgaacgcgctgaatgagttcctgccggagagcttggcccaacgctttcctctgctgtttccaccgttcatcgaggaggcactgaaacaagatgcagtggagatgagcatcctgctgctggccctgcaatacgcgcaaaagtatcctaacaccgtcccggcgtttgcgtgctaataaagatctgaaagaagggacagactagatgttgaaaaatatcccgattccatcccctctgtctccggttgaaggtatcctgattaaacgcaagacgttggagcgttacttctcgattgagcgcctggaacaacaggcgcatcagcgtgcaaagcgcattttgcgtgaggcagaagaagaagccaagaccctgcgcatgtatgcgtaccaggagggctacgagcagggcatgattgacgcactgcaacaggtggccgcctatttgaccgacaaccagacgatggcttggaaatggatggagaaaattcaaatctatgcgcgtgagttgttcagcgcggctgtcgatcacccggaaacgttgttgacggtgctggacgagtggctgcgtgatttcgataagccggaaggtcagctgtttttgaccctgccggtgaacgcaaagaaagatcatcagaaactgatggtgctgctgatggaaaattggccgggcaccttcaatctgaagtatcatcaggagcaacgttttatcatgtcctgtggcgatcagattgccgagttttcgccggaacaatttgttgaaacggcggttggtgttatcaagcaccatctggatgagctgcctcaggactgtcgcaccatttcggacaatgcgattaacgcgctgattgatgaatggaagacgaaaacccaagctgaagttattcgctgataaggatccggcatcaaataaaacgaaaggctcagtcgaaagactgggcctttcgttttatctgttgtttgtcggtgaacgctctcctgagtaggacaaatccgccgccctagaactagtccataagaatgcggccgc

SEQ ID NO: 155 - DNA, 12614 bp, synthetic construct
  misc_feature 1..12614: note = synthetic Syn_InvSpa operon of bacterial type III secretion system (T3SS)
  source 1..12614: mol_type = other DNA
ctcgagaaaaaaaagctctaaaagattaagagggggtaacatatgggtgacgtgagcgcggtgagcagcagcggtaacattctgctgccgcagcaggacgaggttggtggcctgtccgaagcgctgaagaaagcggttgaaaaacacaaaaccgaatacagcggtgacaagaaagatcgtgattatggtgacgcctttgttatgcacaaggaaaccgcgctgccgttgttgctggcagcttggcgccacggcgcaccggcgaaaagcgagcaccataacggtaacgtaagcggtctgcatcacaacggtaagagcgagctgcgtattgctgagaaactgctgaaggtgacggcggagaagagcgttggtctgattagcgctgaagcgaaggtggataaatctgcggcgctgctgtctagcaagaatcgtccgctggaatcggtcagcggcaaaaagttgtccgccgatctgaaagcagtggagtccgtgtccgaggtcacggataacgccaccggcatttcggatgacaacatcaaagcattgccgggtgacaataaggccatcgccggtgagggtgtgcgtaaagaaggtgcgccgctggcgcgtgacgtggctccggcacgcatggcggcagcaaatacgggcaagccggaggataaagaccacaagaaggtcaaggacgttagccagctgccgctgcaaccgactaccatcgccgatctgtctcaactgacgggtggcgatgaaaagatgccgctggcagcgcagtccaaaccgatgatgaccattttcccaaccgccgacggcgttaaaggtgaggacagctctctgacctatcgtttccagcgctggggcaacgattactccgtcaatatccaggcacgccaagcgggcgaatttagcctgattcctagcaatacccaggttgaacatcgtctgcacgaccaatggcaaaatggcaatccacaacgctggcatttgacgcgtgatgaccagcaaaacccgcaacagcaacagcatcgtcagcagtccggtgaagaggacgacgcgtaacttgggcacgcgtccattaagaaggaggaattaagcatggacgatctggttttcgccggcaacaaagccctgtacttggtgctgattctgtccggttggccgacgattgtcgcaaccattatcggtctgctggttggtctgtttcaaaccgtgacgcagttgcaggagcaaaccctgccgttcggtatcaagctgctgggtgtgtgtctgtgcctgtttttgctgtctggctggtatggcgaagttctgctgtcctacggccgtcaggtcatcttcctggctctggcgaaaggttaagacgtccttgggcacgcgtccattaaacaggagtaattaagcatgctgctgtccctgctgaatagcgcgcgtctgcgtcctgagctgctgattctggttctgatggttatgatcatcagcatgttcgttatcccgttgccgacctatttggttgacttcttgatcgctttgaacattgtcctggcaattctggtgttcatgggctccttctacatcgaccgcattctgagcttcagcacctttccggcggttctgctgatcacgactctgttccgtttggcactgagcatcagcaccagccgcctgatcctgattgaagcagatgcgggtgagatcatcgcgacctttggtcagtttgtgatcggtgacagcctggcggttggtttcgtcgtattctccatcgtgacggtggtgcagtttatcgttattaccaagggcagcgaacgtgtggcggaggtcgccgctcgcttcagcctggacggcatgccgggtaaacagatgtctattgatgcagacctgaaagccggcattattgatgctgatgcagcgcgcgagcgccgcagcgtcctggagcgtgaaagccaactgtacggttccttcgacggtgccatgaagttcattaaaggtgatgcgattgcgggcatcattatcatcttcgttaacttcattggcggtatcagcgtcggtatgacccgtcatggtatggatctgagcagcgccctgagcacctacaccatgctgacgattggtgatggtctggttgcccaaattccggcgttgctgatcgcgatttctgcgggcttcatcgttacccgcgtcaacggtgatagcgataacatgggtcgtaacattatgacccagctgctgaataatccgtttgtcctggttgtaacggcgattttgaccatcagcatgggcacgctgccgggctttccgttgccggttttcgttattctgtctgttgtgctgtccgtcctgttttactttaagttccgcgaggcgaaacgtagcgctgcgaaaccaaaaacgagcaagggcgagcaaccgttgtccatcgaggagaaggaaggtagcagcctgggcctgattggcgacctggataaggttagcacggaaaccgtcccgctgattttgctggtgccgaaatcgcgtcgtgaggatctggagaaagcgcagctggcggaacgtctgcgcagccaattctttattgattatggtgtgcgtctgccagaagtactgctgcgtgacggtgagggtctggatgacaactctatcgtcctgctgattaatgagattcgcgttgaacagtttactgtctattttgacctgatgcgtgtggttaactacagcgacgaggtggtgagctttggcatcaacccgaccattcaccagcaaggttccagccagtacttttgggtgacccatgaggaaggcgaaaagctgcgcgagctgggctacgtcctgcgtaatgcactggacgaactgtaccactgtctggcggtgacgctggcacgcaatgtgaacgagtatttcggtatccaagaaacgaaacacatgctggaccaactggaagcaaagtttcctgacctgctgaaggaggttttgcgccacgccaccgtgcagcgcatttcggaagtgctgcaacgtctgctgtccgaacgcgtgagcgtccgtaacatgaagctgatcatggaagccctggcactgtgggctccgcgtgagaaagatgtgatcaatctggtggagcacatccgtggtgcgatggcgcgttatatctgccacaagttcgcaaatggtggtgaactgcgtgccgttatggtttccgccgaagttgaggatgtcattcgtaaaggcattcgtcaaacttctggctccacctttttgagcttggacccggaggcttcggcaaatctgatggacctgatcacgctgaagctggacgacctgttgattgcgcataaggacctggtcctgttgaccagcgttgacgtgcgtcgttttatcaagaaaatgattgaaggtcgttttccggatctggaggtcctgtccttcggtgagattgcagatagcaaaagcgtgaatgtcatcaaaaccatctgaatttaaatcttgggcacgcgtccattaaaaaggagtaattaagcatgagcttcagcgagagccgccacaatgaaaactgtctgattcaagaaggcgcactgctgttttgtgagcaagcagtcgtggcgcctgtcagcggtgatctggtttttcgtccgctgaaaatcgaggtcctgagcaagctgctggcgttcatcgacggcgcaggtctggtggatacgacctacgcggagtcggacaaatgggttctgctgtctccggagttccgtgctatttggcaagaccgtaaacgttgcgaatattggtttttgcagcagattatcaccccatctccggcgttcaacaaggttctggcactgttgcgtaagagcgaaagctattggttggtcggctacttgctggcccaaagcaccagcggcaatactatgcgtatgttgggtgaggattacggtgttagctacacgcatttccgccgtctgtgcagccgcgctctgggcggtaaggcgaaaagcgagctgcgcaattggcgcatggcccagtccctgctgaatagcgtggaaggtcatgaaaacatcacccagctggcggtcaaccacggttatagcagcccgtcccactttagctctgaaatcaaggagctgattggtgtttccccgcgtaagctgtctaacatcattcagctggccgacaaatgaatttaaatgctagccttgggcacgcgtccattaaagaggaccaattaagcatgaaaaccccacgtctgctgcaatacctggcctacccgcagaaaatcactggccctatcattgaagcagaactgcgtgatgttgcaattggtgaattgtgcgagatccgtcgcggctggcaccagaagcaggttgtggcccgtgcgcaagtggttggtttgcagcgcgaacgtaccgtcctgagcctgatcggcaatgcccaaggcctgagccgtgatgtggtcttgtacccgaccggccgtgctctgagcgcgtgggttggttacagcgttctgggcgcagtactggacccgacgggtaaaatcgttgaacgtttcaccccggaagtcgcaccgatttccgaggagcgcgttatcgacgtggcaccgccgagctacgcaagccgtgtcggtgtgcgcgaaccgctgatcacgggtgtccgcgcaattgatggtctgctgacgtgtggtgtgggccagcgtatgggtattttcgcaagcgcgggttgtggtaagaccatgttgatgcacatgctgatcgagcaaaccgaagcggatgtctttgttattggcctgattggcgagcgtggtcgtgaagttaccgaatttgtagacatgttgcgtgcatctcataagaaagaaaaatgtgtgctggtttttgccacgtccgacttcccaagcgttgaccgctgcaacgctgcccagctggcaacgacggtcgccgagtatttccgcgaccagggtaaacgtgttgtcctgtttatcgacagcatgacccgttatgcacgcgcgttgcgtgatgtcgcgctggcgagcggcgagcgtccggctcgccgtggttatccggcgtctgtgttcgacaatctgccgcgtttgctggagcgtccgggtgcgacgagcgagggtagcattaccgccttctataccgtcctgctggagtcggaagaagaagcggacccgatggcggacgagatccgttctattctggacggtcacctgtacctgtcccgcaaactggcgggtcagggtcattacccggctatcgatgtgctgaagagcgtgagccgtgtgtttggtcaagtgaccaccccgactcacgcggagcaagcgagcgcggtccgtaagctgatgacccgtctggaagagctgcaactgttcattgacctgggcgagtatcgtccgggcgagaacattgacaatgatcgtgcgatgcaaatgcgcgatagcctgaaggcgtggctgtgtcagcctgttgcgcaatacagcagcttcgatgatacgctgtccggcatgaacgcctttgcggatcagaactgacttgggcacgcgtccatgaaagaaacgacatactagatgggtaacgatattagcttgattgcattgctggcgttttccaccctgctgccgttcatcatcgcgtctggtacttgcttcgtcaaattcagcatcgtctttgtgatggtgcgcaacgcgctgggtctgcaacaaattccaagcaatatgaccctgaatggcgtcgcactgctgctgtcgatgtttgttatgtggccgattatgcacgacgcgtatgtgtatttcgaggatgaagatgtgacctttaacgacatctccagcctgagcaagcatgttgatgagggcctggacggttatcgcgactacctgatcaagtattccgaccgtgagctggtgcagttctttgagaatgcccagttgaaacgtcagtacggtgaagaaacggaaaccgttaaacgtgacaaggacgagattgaaaagccgagcattttcgcactgttgcctgcttacgccttgagcgagattaagagcgcattcaaaattggtttttacctgtacctgccgttcgttgtggtcgatctggttgtctccagcgttctgctggccctgggcatgatgatgatgtccccggttaccatcagcacgccgatcaaactggtcctgtttgtggccctggatggttggacgctgctgtctaaaggcctgatcctgcaatacatggacatcgcgacctaagagctctgggcacgcgtccattaatgaggaaaaattattagcatgaaaacgcacattctgttggcccgtgtgctggcttgcgcagctctggtgctggtcaccccaggttatagctccgagaagatcccggttacgggcagcggcttcgttgcaaaggacgattctctgcgcacctttttcgatgcgatggcactgcaattgaaggagccggtgattgtcagcaagatggcggctcgcaaaaagattaccggcaatttcgagttccacgatccaaacgcgctgctggagaaactgtccctgcaactgggtctgatctggtactttgatggtcaggcgatctacatctacgacgcgagcgaaatgcgtaatgcggttgtgagcctgcgtaatgtcagcctgaacgagttcaacaattttctgaagcgcagcggcctgtacaataagaactaccctctgcgtggtgataatcgtaaaggcaccttctatgtcagcggtccgccggtgtatgttgatatggttgtaaatgcggccaccatgatggacaaacagaatgatggcatcgagctgggtcgccaaaagatcggtgttatgcgcctgaacaacacttttgtgggcgaccgcacctacaacctgcgtgatcaaaagatggtcattccgggtattgctacggcaattgaacgcctgttgcaaggcgaagaacaaccgctgggtaacattgtaagctccgagcctccggccatgccggcctttagcgcaaacggcgagaaaggtaaggcagcgaattacgcgggtggtatgagcctgcaagaagcgctgaaacagaacgcagcggcaggcaacatcaaaattgtggcctatccggacaccaacagcctgctggtgaaaggtacggcggagcaggtgcatttcatcgagatgctggttaaagccctggacgtggcgaaacgtcacgttgaattgagcctgtggattgtggatttgaataagagcgacctggaacgcttgggcaccagctggagcggtagcatcaccatcggcgacaagctgggtgtgagcctgaaccagagcagcatctccacgctggacggtagccgctttattgcggcggtcaacgctctggaggaaaagaaacaggccactgttgtcagccgtccggttctgctgacccaggagaatgtcccggcgatttttgacaataatcgtactttctataccaaactgatcggtgaacgtaatgttgcattggaacacgtgacctatggcaccatgatccgtgtcctgccgcgtttcagcgcggacggccagattgagatgagcctggacatcgaagatggtaatgacaaaaccccgcagtctgatacgaccacctccgttgatgcgctgccagaagtgggtcgtaccctgatctcgacgattgcacgtgtcccgcatggtaaatctctgctggttggtggctacacgcgtgatgcaaacacggacacggtccaaagcatcccgttcctgggtaagctgccgctgattggctcgttgtttcgctacagcagcaaaaacaagtctaatgtcgtccgtgtctttatgattgagccgaaagaaatcgttgacccgctgaccccggatgccagcgagagcgttaacaacattctgaaacagtccggtgcgtggagcggtgacgataagctgcaaaagtgggttcgtgtgtatttggaccgtggtcaggaggccattaagtaacttgggcacgcgtccatgaaagacaggacccactagatgtccagcaacaaaaccgaaaaaccgactaagaaacgtctggaggatagcgcaaagaaaggtcagagcttcaagagcaaggacctgattatcgcgtgcctgaccctgggtggtatcgcttatttggtgagctacggcagcttcaatgagtttatgggtatcattaagattatcatcgctgataactttgatcagtcgatggcagattatagcctggccgtgtttggtattggcctgaaatacctgattccgttcatgctgctgtgtttggtttgttccgcactgccggcactgctgcaagcgggcttcgttctggcaaccgaggccctgaagccgaatctgtccgccctgaacccggttgaaggcgcgaagaaactgttttccatgcgcaccgtcaaagacacggtcaagacgctgctgtatctgtcgagctttgtggttgcggcaatcatttgctggaaaaagtataaagtcgagattttcagccaactgaacggtaatatcgtgggtattgcggttatctggcgtgaattgctgctggcgttggttctgacctgtctggcgtgcgcgctgatcgtgctgttgctggatgctattgccgagtactttctgaccatgaaagatatgaagatggacaaagaagaagttaaacgcgagatgaaagagcaggagggtaacccggaggtgaagtctaaacgtcgtgaagtccacatggaaatcctgagcgaacaagtcaagtctgacattgaaaatagccgtctgattgtggcaaaccctacgcatattaccatcggcatctacttcaaaccggaactgatgccgattccaatgattagcgtctatgaaaccaatcaacgcgcgctggcggtccgtgcgtacgccgagaaagtgggtgttccggttattgtagacatcaagctggcgcgcagcctgttcaaaacgcaccgtcgttacgacctggtgagcctggaggagatcgacgaggttttgcgcctgctggtttggttggaagaggtcgaaaacgcaggcaaggatgtgatccaaccgcaggagaatgaagtgcgtcattaactgcaggtttaaactacttgggcacgcgtccattaattaggatcaatagcatgattccgggcagcacctccggtatttcctttagccgtatcctgagccgtcagacctcccaccaggatgcaacccagcataccgacgcacaacaagcggaaattcaacaagcggcggaagatagctcgccgggtgcggaggttcagaaattcgtccagagcacggacgagatgtctgctgcgttggcgcagttccgcaatcgccgtgactatgagaaaaagagcagcaatttgtctaactccttcgagcgcgttctggaggacgaggcactgccgaaagcgaagcagattctgaaactgatcagcgtgcatggcggtgcgttggaggatttcctgcgtcaggcgcgcagcctgttcccggacccaagcgatctggtgctggttctgcgcgagctgttgcgtcgtaaggacctggaggagatcgtgcgtaagaagctggagagcctgctgaagcacgtggaggaacaaaccgacccgaaaaccctgaaggccggtattaactgcgcgctgaaggcgcgtctgtttggcaagacgctgtctctgaaacctggtctgctgcgtgccagctaccgccagttcatccaaagcgaaagccacgaagtcgagatttacagcgattggatcgccagctacggttatcagcgtcgcctggttgttctggatttcattgaaggcagcctgctgactgacatcgatgctaacgatgcaagctgctcccgtctggagtttggccaactgctgcgccgtctgacccagctgaaaatgttgcgtagcgccgacctgctgtttgtctcgacgttgctgtcttacagcttcacgaaagcatttaacgctgaggagagcagctggctgttgctgatgctgtctttgctgcaacagccgcacgaagtggatagcctgctggcggacattatcggtctgaatgcgctgctgttgtcccacaaagagcacgccagcttcctgcaaatcttctatcaggtctgtaaggcaatcccgtctagcctgttttatgaagagtactggcaagaagaactgctgatggcactgcgctccatgacggacattgcttacaaacacgaaatggccgaacaacgtcgtaccatcgaaaagctgtcctaagtttaaaccttgggcacgcgtccatgaaagacaggacccactagatgagcttgcgcgtacgccaaattgaccgccgtgaatggctgctggcccagactgcgaccgaatgtcagcgtcacggtcgtgaggccaccctggagtatccgacccgtcagggtatgtgggtccgcctgtctgatgccgaaaaacgctggtctgcgtggatcaaaccgggtgattggttggaacacgttagcccagcactggcgggtgccgcggtcagcgcaggcgcggagcacctggtggttccgtggctggcggcaaccgaacgcccgttcgagctgccggtcccgcacttgagctgccgtcgtctgtgcgtggagaacccggttccgggttccgcactgcctgagggcaagctgctgcacatcatgtcggatcgtggtggcctgtggtttgagcatctgccggagctgccggctgttggcggtggccgtccgaagatgctgcgttggccgctgcgtttcgttattggcagcagcgacacccagcgcagcctgctgggtcgtatcggtatcggtgatgttctgctgatccgcaccagccgtgctgaggtttactgttacgcgaagaaactgggccactttaatcgtgtggaaggtggcattattgtcgaaacgctggacattcaacatatcgaggaggagaacaacacgacggaaacggcggaaaccctgccgggtctgaatcaactgccggtgaagctggagttcgttctgtatcgtaaaaacgtgacgttggccgaactggaagcaatgggtcagcaacaactgctgtccttgccaaccaatgcggaactgaacgtcgaaatcatggcgaatggcgtgctgctgggtaacggcgaactggtgcagatgaatgacaccctgggtgtcgagattcatgagtggttgtccgagagcggtaatggcgagtagagatctcttgggcacgcgtccattaaaaaggaccaattaagcatgcactctctgactcgtatcaaggtcctgcaacgtcgttgtaccgtgttccattctcagtgcgagtccattctgttgcgttatcaggacgaagatcgcggcttgcaggcggaggaggaggccatcctggaacagatcgcaggtctgaaactgctgttggacaccctgcgtgctgaaaatcgtcaactgagccgtgaagaaatctatacgctgctgcgcaaacagagcattgttcgtcgccagattaaggatctggagctgcaaatcattcagattcaagaaaagcgtagcgagctggaaaagaaacgtgaggaatttcaaaagaaaagcaaatactggctgcgtaaagaaggtaactaccagcgctggattatccgtcaaaaacgcttctacattcaacgtgagatccagcaagaggaggcggagagcgaagagatcatttaacttgggcacgcgtccatgaaagacaggacccactagatgttctatgcattgtattttgagatccaccatctggtggcgtccgcggctctgggttttgcgcgtgttgctccgatctttttctttctgccgttcctgaatagcggtgtcctgagcggtgctccgcgcaacgcgatcatcattctggtggcgctgggtgtatggccgcacgccctgaatgaggcgccaccgtttctgtctgtggcaatgattccgctggtcctgcaagaggcagccgtgggtgttatgctgggttgcctgttgtcctggccgttttgggttatgcacgcgttgggctgtatcattgataaccaacgcggtgcaaccctgtccagcagcattgatcctgcgaatggcatcgacaccagcgagatggccaatttcctgaacatgttcgcggctgtcgtgtatttgcagaacggtggcttggtcacgatggtggacgtgctgaataagtcttaccagctgtgtgatccgatgaacgagtgtacgccgagcctgcctccgttgctgaccttcattaatcaagtggcccagaacgcactggtgctggcgtccccggtcgttctggttctgctgctgtcggaagttttcctgggcctgctgtctcgttttgcaccgcaaatgaacgcgttcgccattagcctgactgttaaaagcggtattgcggttttgatcatgctgctgtatttcagcccggtcctgccggacaatgttctgcgtctgagctttcaggcgaccggcctgagcagctggttctacgaacgtggcgcaacgcatgtgctggaataaggatccggcatcaaataaaacgaaaggctcagtcgaaagactgggcctttcgttttatctgttgtttgtcggtgaacgctctcctgagtaggacaaatccgccgccctagaactagtccataagaatgcggccgc

SEQ ID NO: 156 - DNA, 23 bp, synthetic construct
  misc_feature 1..23: note = synthetic Enterobacteria phage T7 promoter seed sequence
  modified_base 16..20: mod_base = OTHER; note = n = g, a, c or t
  source 1..23: mol_type = other DNA
taatacgactcactannnnnaga

SEQ ID NO: 157 - DNA, 23 bp, synthetic construct
  misc_feature 1..23: note = synthetic Enterobacteria phage T7 wild type (WT) promoter
  source 1..23: mol_type = other DNA
taatacgactcactatagggaga

SEQ ID NO: 158 - DNA, 23 bp, synthetic construct
  misc_feature 1..23: note = synthetic mutant Enterobacteria phage T7 promoter Mut1
  source 1..23: mol_type = other DNA
taatacgactcactacaggcaga

SEQ ID NO: 159 - DNA, 23 bp, synthetic construct
  misc_feature 1..23: note = synthetic mutant Enterobacteria phage T7 promoter Mut2
  source 1..23: mol_type = other DNA
taatacgactcactagagagaga

SEQ ID NO: 160 - DNA, 23 bp, synthetic construct
  misc_feature 1..23: note = synthetic mutant Enterobacteria phage T7 promoter Mut3
  source 1..23: mol_type = other DNA
taatacgactcactaatgggaga

SEQ ID NO: 161 - DNA, 23 bp, synthetic construct
  misc_feature 1..23: note = synthetic mutant Enterobacteria phage T7 promoter Mut4
  source 1..23: mol_type = other DNA
taatacgactcactataggtaga

SEQ ID NO: 162 - DNA, 23 bp, synthetic construct
  misc_feature 1..23: note = synthetic mutant Enterobacteria phage T7 promoter Mut5
  source 1..23: mol_type = other DNA
taatacgactcactaaagggaga

SEQ ID NO: 163 - DNA, 23 bp, synthetic construct
  misc_feature 1..23: note = synthetic mutant Enterobacteria phage T7 promoter Mut6
  source 1..23: mol_type = other DNA
taatacgactcactattgggaga

SEQ ID NO: 164 - DNA, 26 bp, synthetic construct
  misc_feature 1..26: note = synthetic Klebsiella oxytoca nif operon deletion mutant NF8 deletion region
  modified_base 26: mod_base = OTHER; note = c modified by Km cassette and SEQ ID NO:163
  source 1..26: mol_type = other DNA
gcaggagaactaaaggcccggcatgc

SEQ ID NO: 165 - DNA, 26 bp, synthetic construct
  misc_feature 1..26: note = synthetic Klebsiella oxytoca nif operon deletion mutant NF8 deletion region
  modified_base 1: mod_base = OTHER; note = g modified by Km cassette and SEQ ID NO:164
  source 1..26: mol_type = other DNA
gcatgcaagcgcccatggccccggca

SEQ ID NO: 166 - DNA, 46 bp, synthetic construct
  misc_feature 1..46: note = synthetic Klebsiella oxytoca nif in-frame deletion mutant UC12 deletion region
  source 1..46: mol_type = other DNA
cataaacaggcacggctggtggtaccccatcaggtgccccgcgtca

SEQ ID NO: 167 - DNA, 46 bp, synthetic construct
  misc_feature 1..46: note = synthetic Klebsiella oxytoca nif operon deletion mutant NF9 deletion region
  source 1..46: mol_type = other DNA
atggccccggcaggcgcaatgcatgcgacgctcttccccacgttac

SEQ ID NO: 168 - DNA, 46 bp, synthetic construct
  misc_feature 1..46: note = synthetic Klebsiella oxytoca nif operon deletion mutant UC14 deletion region
  source 1..46: mol_type = other DNA
gacgctcttccccacgttacgcatgcgatccggacccgcgccgcta

SEQ ID NO: 169 - DNA, 46 bp, synthetic construct
  misc_feature 1..46: note = synthetic Klebsiella oxytoca nif operon deletion mutant UC15 deletion region
  source 1..46: mol_type = other DNA
ctcttccccacgttacgctcgcatgcgatccggacccgcgccgcta

SEQ ID NO: 170 - DNA, 46 bp, synthetic construct
  misc_feature 1..46: note = synthetic Klebsiella oxytoca nif operon deletion mutant NF10 deletion region
  source 1..46: mol_type = other DNA
cggacccgcgccgctagccggcatgcatctttggcagcagagccag

SEQ ID NO: 171 - DNA, 46 bp, synthetic construct
  misc_feature 1..46: note = synthetic Klebsiella oxytoca nif operon deletion mutant NF11 deletion region
  source 1..46: mol_type = other DNA
cggacccgcgccgctagccggcatgcagcctcggcggctacccgtt

SEQ ID NO: 172 - DNA, 46 bp, synthetic construct
  misc_feature 1..46: note = synthetic Klebsiella oxytoca nif operon deletion mutant NF12 deletion region
  source 1..46: mol_type = other DNA
actggttatcctgatccagcgcatgcctttgcactaccgcggccca

SEQ ID NO: 173 - DNA, 46 bp, synthetic construct
  misc_feature 1..46: note = synthetic Klebsiella oxytoca nif operon deletion mutant NF13 deletion region
  source 1..46: mol_type = other DNA
ccgttaacgcctacagcacggcatgcctttgcactaccgcggccca

SEQ ID NO: 174 - DNA, 40 bp, synthetic construct
  misc_feature 1..40: note = synthetic Klebsiella oxytoca nif operon deletion mutant NF14 deletion region
  source 1..40: mol_type = other DNA
attcagggacgcgggttgccatgtgattatgcgacgtctt

SEQ ID NO: 175 - DNA, 46 bp, synthetic construct
  misc_feature 1..46: note = synthetic Klebsiella oxytoca nif operon deletion mutant NF24 deletion region
  source 1..46: mol_type = other DNA
gtcaaacaccagaatattgagagctctgtcgtttctgtgacaaagc

SEQ ID NO: 176 - DNA, 46 bp, synthetic construct
  misc_feature 1..46: note = synthetic Klebsiella oxytoca nif operon deletion mutant NF25 deletion region
  source 1..46: mol_type = other DNA
cggacccgcgccgctagccggcatgcctttgcactaccgcggccca

SEQ ID NO: 177 - DNA, 46 bp, synthetic construct
  misc_feature 1..46: note = synthetic Klebsiella oxytoca whole nif deletion mutant NF26 deletion region
  source 1..46: mol_type = other DNA
gtcaaacaccagaatattgactcgagatgtgattatgcgacgtctt

SEQ ID NO: 178 - DNA, 23 bp, synthetic construct
  misc_feature 1..23: note = synthetic wild type (WT) Enterobacteria phage T7 promoter part number SBa_000443
  source 1..23: mol_type = other DNA
taatacgactcactatagggaga

SEQ ID NO: 179 - DNA, 23 bp, synthetic construct
  misc_feature 1..23: note = synthetic Enterobacteria phage T7 promoter 1 part number SBa_000444
  source 1..23: mol_type = other DNA
taatacgactcactacaggcaga

SEQ ID NO: 180 - DNA, 23 bp, synthetic construct
  misc_feature 1..23: note = synthetic Enterobacteria phage T7 promoter 2 part number SBa_000445
  source 1..23: mol_type = other DNA
taatacgactcactagagagaga

SEQ ID NO: 181 - DNA, 23 bp, synthetic construct
  misc_feature 1..23: note = synthetic Enterobacteria phage T7 promoter 3 part number SBa_000446
  source 1..23: mol_type = other DNA
taatacgactcactaatgggaga

SEQ ID NO: 182 - DNA, 23 bp, synthetic construct
  misc_feature 1..23: note = synthetic Enterobacteria phage T7 promoter 4 part number SBa_000447
  source 1..23: mol_type = other DNA
taatacgactcactattgggaga

SEQ ID NO: 183 - DNA, 48 bp, synthetic construct
  misc_feature 1..48: note = synthetic Enterobacteria phage T7 wild type (WT) terminator part number SBa_000450
  source 1..48: mol_type = other DNA
tagcataaccccttggggcctctaaacgggtcttgaggggttttttgt

SEQ ID NO: 184 - DNA, 29 bp, synthetic construct
  misc_feature 1..29: note = synthetic Enterobacteria phage T7 terminator part number SBa_000451
  source 1..29: mol_type = other DNA
tacatatcgggggggtaggggttttttgt

SEQ ID NO: 185 - DNA, 37 bp, synthetic construct; identical to SEQ ID NO: 72
  misc_feature 1..37: note = synthetic Enterobacteria phage T7 terminator part number SBa_000452
  source 1..37: mol_type = other DNA

SEQ ID NO: 186 - DNA, 50 bp, synthetic construct; identical to SEQ ID NO: 55
  misc_feature 1..50: note = synthetic insulator part number SBa_000453
  source 1..50: mol_type = other DNA

SEQ ID NO: 187 - DNA, 50 bp, synthetic construct; identical to SEQ ID NO: 58
  misc_feature 1..50: note = synthetic insulator part number SBa_000454
  source 1..50: mol_type = other DNA

SEQ ID NO: 188 - DNA, 40 bp, synthetic construct; identical to SEQ ID NO: 61
  misc_feature 1..40: note = synthetic insulator part number SBa_000455
  source 1..40: mol_type = other DNA

SEQ ID NO: 189 - DNA, 40 bp, synthetic construct; identical to SEQ ID NO: 64
  misc_feature 1..40: note = synthetic insulator part number SBa_000456
  source 1..40: mol_type = other DNA

SEQ ID NO: 190 - DNA, 40 bp, synthetic construct; identical to SEQ ID NO: 67
  misc_feature 1..40: note = synthetic insulator part number SBa_000457
  source 1..40: mol_type = other DNA

SEQ ID NO: 191 - DNA, 30 bp, synthetic construct; identical to SEQ ID NO: 73
  misc_feature 1..30: note = synthetic insulator part number SBa_000458
  source 1..30: mol_type = other DNA

SEQ ID NO: 192 - DNA, 40 bp, synthetic construct; identical to SEQ ID NO: 75
  misc_feature 1..40: note = synthetic insulator part number SBa_000459
  source 1..40: mol_type = other DNA

SEQ ID NO: 193 - DNA, 40 bp, synthetic construct; identical to SEQ ID NO: 78
  misc_feature 1..40: note = synthetic insulator part number SBa_000460
  source 1..40: mol_type = other DNA

SEQ ID NO: 194 - DNA, 18 bp, synthetic construct
  misc_feature 1..18: note = synthetic insulator part number SBa_000461
  source 1..18: mol_type = other DNA
gtctgtagcacgtgcatc

SEQ ID NO: 195 - DNA, 18 bp, synthetic construct
  misc_feature 1..18: note = synthetic insulator part number SBa_000462
  source 1..18: mol_type = other DNA
ggtcattacaacggttat

SEQ ID NO: 196 - DNA, 40 bp, synthetic construct; identical to SEQ ID NO: 89
  misc_feature 1..40: note = synthetic insulator part number SBa_000463
  source 1..40: mol_type = other DNA

SEQ ID NO: 197 - DNA, 40 bp, synthetic construct; identical to SEQ ID NO: 92
  misc_feature 1..40: note = synthetic insulator part number SBa_000464
  source 1..40: mol_type = other DNA

SEQ ID NO: 198 - DNA, 40 bp, synthetic construct; identical to SEQ ID NO: 95
  misc_feature 1..40: note = synthetic insulator part number SBa_000465
  source 1..40: mol_type = other DNA

SEQ ID NO: 199 - DNA, 40 bp, synthetic construct; identical to SEQ ID NO: 98
  misc_feature 1..40: note = synthetic insulator part number SBa_000466
  source 1..40: mol_type = other DNA

SEQ ID NO: 200 - DNA, 40 bp, synthetic construct; identical to SEQ ID NO: 101
  misc_feature 1..40: note = synthetic insulator part number SBa_000467
  source 1..40: mol_type = other DNA

SEQ ID NO: 201 - DNA, 40 bp, synthetic construct; identical to SEQ ID NO: 104
  misc_feature 1..40: note = synthetic insulator part number SBa_000468
  source 1..40: mol_type = other DNA

SEQ ID NO: 202 - DNA, 40 bp, synthetic construct; identical to SEQ ID NO: 36
  misc_feature 1..40: note = synthetic insulator part number SBa_000508
  source 1..40: mol_type = other DNA

SEQ ID NO: 203 - DNA, 110 bp, synthetic construct
  misc_feature 1..110: note = synthetic ribosome binding site (RBS) part number SBa_000475
  source 1..110: mol_type = other DNA
ttaaagaggagaaattaagcatgaaaactatggacggtaacgctgcggctgcatggattagctacgcctttaccgaagtggctgcgatctacccgattacgccgagcacc

SEQ ID NO: 204 - DNA, 126 bp, synthetic construct
  misc_feature 1..126: note = synthetic ribosome binding site (RBS) part number SBa_000469
  source 1..126: mol_type = other DNA
tactagagacaataaactaacataaggaggataaatatgaccatgcgtcagtgcgcgatttatggcaaaggtggtattggcaaaagcacgacgacccagaacttggtggcggccctggccgagatg

SEQ ID NO: 205 - DNA, 174 bp, synthetic construct
  misc_feature 1..174: note = synthetic ribosome binding site (RBS) part number SBa_000470
  source 1..174: mol_type = other DNA
gcgtgcgtacaccttaatcaccgcttcatgctaaggtcctggctgcatgcaaaaattcacatccctatctagcggaggagccggatgatgactaatgctactggcgaacgtaacctggcactgattcaagaagtactggaagtgttcccggaaaccgcgcgcaaagagcgccgt

SEQ ID NO: 206 - DNA, 174 bp, synthetic construct
  misc_feature 1..174: note = synthetic ribosome binding site (RBS) part number SBa_000471
  source 1..174: mol_type = other DNA
caaacaccccatgtcgatactgaacgaatcgacgcacactcccttccttgcaatctcatactctcaaaaattaggcgaggtaacatgtctcaaactatcgataaaatcaactcttgttacccgctgttcgagcaggacgaatatcaggaactgttccgtaacaaacgtcagctg

SEQ ID NO: 207 - DNA, 156 bp, synthetic construct
  misc_feature 1..156: note = synthetic ribosome binding site (RBS) part number SBa_000472
  source 1..156: mol_type = other DNA
cctgattgtatccgcatctgatgctaccgtggttgagttaccatactcactcccggaggtacttctatgtctgacaatgataccctgttttggcgcatgctggcgctgtttcagtcgctgccggatttgcagccggctcaaatcgtcgattggctg

SEQ ID NO: 208 - DNA, 162 bp, synthetic construct
  misc_feature 1..162: note = synthetic ribosome binding site (RBS) part number SBa_000473
  source 1..162: mol_type = other DNA
catttttgccttgcgacagacctcctacttagattgccacactattcaatacatcactggaggttattacaaatgaagggtaacgagattcttgctctgctggacgaaccggcctgtgaacacaaccataaacagaaatccggctgtagcgccccaaagccg

SEQ ID NO: 209 - DNA, 161 bp, synthetic construct
  misc_feature 1..161: note = synthetic ribosome binding site (RBS) part number SBa_000474
  source 1..161: mol_type = other DNA
tgtcacgctaggaggcaattctataagaatgcacactgcacctaaacctaccacacctgaggagagtaattatggcagacattttccgcactgataagccgttggctgtgtcgccgatcaagaccggccagccgctgggtgcgatcctggcgtccctgggt

SEQ ID NO: 210 - DNA, 167 bp, synthetic construct
  misc_feature 1..167: note = synthetic ribosome binding site (RBS) part number SBa_000476
  source 1..167: mol_type = other DNA
aacatagcgttccatgagggctagaattacctaccggcctcagatactgacaaataaaccagcgaaggaggttcctaatgtggaactacagcgagaaagtcaaggaccatttcttcaatccgcgcaacgcgcgtgttgtggataacgcaaatgcggtgggcgacgtc

SEQ ID NO: 211 - DNA, 169 bp, synthetic construct
  misc_feature 1..169: note = synthetic ribosome binding site (RBS) part number SBa_000477
  source 1..169: mol_type = other DNA
cattgtaatagccaccaaaagagtgatgatagtcatgggtgatacccgtagaccattctgaaatcgaaggaggttttccatgaaacaagtgtacctggacaacaacgcgaccacccgcctggacccgatggttctggaagcgatgatgccgtttctcacggatttctat

SEQ ID NO: 212 - DNA, 164 bp, synthetic construct
  misc_feature 1..164: note = synthetic ribosome binding site (RBS) part number SBa_000478
  source 1..164: mol_type = other DNA
gagttactggccctgatttctccgcttctaataccgcacagcgactaggagcctaactcgccacaaggaaacatatggagcgcgtcttgatcaacgatactaccctgcgtgatggcgaacaatctccgggcgtagcgtttcgtacctccgagaaagttgccatc

SEQ ID NO: 213 - DNA, 165 bp, synthetic construct
  misc_feature 1..165: note = synthetic ribosome binding site (RBS) part number SBa_000479
  source 1..165: mol_type = other DNA
gactcaacacgctagggacgtgaagtcgattccttcgatgcagaaggcgagaactagatttaagggccattatagatggagtggttttaccagattccgggtgtagacgaattgcgcagcgctgaatccttctttcagttcttcgcggttccataccagccggaa

SEQ ID NO: 214 - DNA, 166 bp, synthetic construct
  misc_feature 1..166: note = synthetic ribosome binding site (RBS) part number SBa_000480
  source 1..166: mol_type = other DNA
tcgagaaacaaggcagttccgggctgaaagtagcgccgggacaagtcccgtattataaccgcctaggaggtgttggatgcgcccgaaattcaccttctctgaagaggtccgcgtagttcgcgcgattcgtaatgatggcaccgtggcgggttttgcgccaggtgcg

SEQ ID NO: 215 - DNA, 164 bp, synthetic construct
  misc_feature 1..164: note = synthetic ribosome binding site (RBS) part number SBa_000481
  source 1..164: mol_type = other DNA
acgccacgcgtagtgagacatacacgttcgttgggttcactcagagactgaagttattacccaggaggtctataatgaatccgtggcagcgctttgcccgtcaacgccttgctcgcagccgctggaaccgtgatccggctgctctcgacccagccgatacccca

SEQ ID NO: 216 - DNA, 124 bp, synthetic construct
  misc_feature 1..124: note = synthetic ribosome binding site (RBS) part number SBa_000482
  source 1..124: mol_type = other DNA
gacaagagtctcaattataaggaggctttactacatggcgaacatcggcatcttctttggtacggataccggcaaaacccgcaagattgcgaagatgattcacaaacagctgggcgagctggcc

SEQ ID NO: 217 - DNA, 169 bp, synthetic construct
  misc_feature 1..169: note = synthetic ribosome binding site (RBS) part number SBa_000483
  source 1..169: mol_type = other DNA
cgcgacttccagagaagaagactactgacttgagcgttccctctctgtaatacatcaaatcaatcataggagggctaaaatgacctcttgttcgtcgttttctggcggtaaagcgtgccgtccggccgatgactccgcgctgactccgctggtggccgacaaggcagct

SEQ ID NO: 218 - DNA, 152 bp, synthetic construct
  misc_feature 1..152: note = synthetic ribosome binding site (RBS) part number SBa_000475
  source 1..152: mol_type = other DNA
aactacgagatttgaggtaaaccaaataagcacgtagtggcattaaagaggagaaattaagcatgccgccattggactggttgcgtcgtttgtggttactctatcacgccggcaaaggcagctttccgcttcgtatgggcttgtcgccgcgt

SEQ ID NO: 219 - DNA, 1761 bp, synthetic construct
  misc_feature 1..1761: note = synthetic P-tac promoter and lacI cassette part number SBa_000561
  source 1..1761: mol_type = other DNA
caattcgcgctaacttacattaattgcgttgcgctcactgcccgctttccagtcgggaaacctgtcgtgccagctgcattaatgaatcggccaacgcgcggggagaggcggtttgcgtattgggcgccagggtggtttttcttttcaccagtgagacgggcaacagctgattgcccttcaccgcctggccctgagagagttgcagcaagcggtccacgctggtttgccccagcaggcgaaaatcctgtttgatggtggttgacggcgggatataacatgagctgtcttcggtatcgtcgtatcccactaccgagatatccgcaccaacgcgcagcccggactcggtaatggcgcgcattgcgcccagcgccatctgatcgttggcaaccagcatcgcagtgggaacgatgccctcattcagcatttgcatggtttgttgaaaaccggacatggcactccagtcgccttcccgttccgctatcggctgaatttgattgcgagtgagatatttatgccagccagccagacgcagacgcgccgagacagaacttaatgggcccgctaacagcgcgatttgctggtgacccaatgcgaccagatgctccacgcccagtcgcgtaccgtcttcatgggagaaaataatactgttgatgggtgtctggtcagagacatcaagaaataacgccggaacattagtgcaggcagcttccacagcaatggcatcctggtcatccagcggatagttaatgatcagcccactgacgcgttgcgcgagaagattgtgcaccgccgctttacaggcttcgacgccgcttcgttctaccatcgacaccaccacgctggcacccagttgatcggcgcgagatttaatcgccgcgacaatttgcgacggcgcgtgcagggccagactggaggtggcaacgccaatcagcaacgactgtttgcccgccagttgttgtgccacgcggttgggaatgtaattcagctccgccatcgccgcttccactttttcccgcgttttcgcagaaacgtggctggcctggttcaccacgcgggaaacggtctgataagagacaccggcatactctgcgacatcgtataacgttactggtttcacattcaccaccctgaattgactctcttccgggcgctatcatgccataccgcgaaaggttttgcaccattcgatggtgtcaacgtaaatgcatgccgcttcgccttcgcgcgcgaattggccgccatgccggcgataatggcctgcttctcgccgaaacgtttggtggcgggaccagtgacgaaggcttgagcgagggcgtgcaagattccgaataccgcaagcgacaggccgatcatcgtcgcgctccagcgaaagcggtcctcgccgaaaatgacccagagcgctgccggcacctgtcctacgagttgcatgataaagaagacagtcataagtgcggcgacgatagtcatgccccgcgcccaccggaaggagctgactgggttgaaggctctcaagggcatcggcggagcttatcgactgcacggtgcaccaatgcttctggcgtcaggcagccatcggaagctgtggtatggctgtgcaggtcgtaaatcactgcataattcgtgtcgctcaaggcgcactcccgttctggataatgttttttgcgccgacatcataacggttctggcaaatattctgaaatgagctgttgacaattaatcatcggctcgtataatgtgtggaattgtgagcggataacaatt

SEQ ID NO: 220 - DNA, 740 bp, synthetic construct
  misc_feature 1..740: note = synthetic P-tet promoter and tetR cassette part number SBa_000562
  source 1..740: mol_type = other DNA
ttattaggacccactttcacatttaagttgtttttctaatccgcatatgatcaattcaaggccgaataagaaggctggctctgcaccttggtgatcaaataattcgatagcttgtcgtaataatggcggcatactatcagtagtaggtgtttccctttcttctttagcgacttgatgctcttgatcttccaatacgcaacctaaagtaaaatgccccacagcgctgagtgcatataatgcattctctagtgaaaaaccttgttggcataaaaaggctaattgattttcgagagtttcatactgtttttctgtaggccgtgtacctaaatgtacttttgctccatcgcgatgacttagtaaagcacatctaaaacttttagcgttattacgtaaaaaatcttgccagctttccccttctaaagggcaaaagtgagtatggtgcctatctaacatctcaatggctaaggcgtcgagcaaagcccgcttattttttacatgccaatacaatgtaggctgctctacacctagcttctgggcgagtttacgggttgttaaaccttcgattccgacctcattaagcagctctaatgcgctgttaatcactttacttttatctaatctggacatcgaggcctttcctgtgtgagctagcactgtacctaggactgagctagccgtcaattttttccctatcagtgatagagattgacatccctatcagtgatagatataatgagcac

SEQ ID NO: 221 - DNA, 702 bp, synthetic construct
  misc_feature 1..702: note = synthetic red fluorescent protein (mRFP) fluorescsnt reporter part number SBa_000484
  source 1..702: mol_type = other DNA
atgtccagattagataaaagtaaagttgcgagctctgaagacgttatcaaagagttcatgcgtttcaaagttcgtatggaaggttccgttaacggtcacgagttcgaaatcgaaggtgaaggtgaaggtcgtccgtacgaaggtacccagaccgctaaactgaaagttaccaaaggtggtccgctgccgttcgcttgggacatcctgtccccgcagttccagtacggttccaaagcttacgttaaacacccggctgacatcccggactacctgaaactgtccttcccggaaggtttcaaatgggaacgtgttatgaacttcgaagacggtggtgttgttaccgttacccaggactcctccctgcaagacggtgagttcatctacaaagttaaactgcgtggtaccaacttcccgtccgacggtccggttatgcagaaaaaaaccatgggttgggaagcttccaccgaacgtatgtacccggaagacggtgctctgaaaggtgaaatcaaaatgcgtctgaaactgaaagacggtggtcactacgacgctgaagttaaaaccacctacatggctaaaaaaccggttcagctgccgggtgcttacaaaaccgacatcaaactggacatcacctcccacaacgaagactacaccatcgttgaacagtacgaacgtgctgaaggtcgtcactccaccggtgcttaa

SEQ ID NO: 222 - DNA, 2652 bp, synthetic construct
  misc_feature 1..2652: note = synthetic Enterobacteria phage T7* variant RNA polymerase (RNAP) part number SBa_000514
  source 1..2652: mol_type = other DNA
atgaacacgattaacatcgctaagaacgacttctctgacatcgaactggctgctatcccgttcaacactctggctgaccattacggtgagcgtttagctcgcgaacagttggcccttgagcatgagtcttacgagatgggtgaagcacgcttccgcaagatgtttgagcgtcaacttaaagctggtgaggttgcggataacgctgccgccaagcctctcatcactaccctactccctaagatgattgcacgcatcaacgactggtttgaggaagtgaaagctaagcgcggcaagcgcccgacagccttccagttcctgcaagaaatcaagccggaagccgtagcgtacatcaccattaagaccactctggcttgcctaaccagtgctgacaatacaaccgttcaggctgtagcaagcgcaatcggtcgggccattgaggacgaggctcgcttcggtcgtatccgtgaccttgaagctaagcacttcaagaaaaacgttgaggaacaactcaacaagcgcgtagggcacgtctacaagaaagcatttatgcaagttgtcgaggctgacatgctctctaagggtctactcggtggcgaggcgtggtcttcgtggcataaggaagactctattcatgtaggagtacgctgcatcgagatgctcattgagtcaaccggaatggttagcttacaccgccaaaatgctggcgtagtaggtcaagactctgagactatcgaactcgcacctgaatacgctgaggctatcgcaacccgtgcaggtgcgctggctggcatctctccgatgttccaaccttgcgtagttcctcctaagccgtggactggcattactggtggtggctattgggctaacggtcgtcgtcctctggcgctggtgcgtactcacagtaagaaagcactgatgcgctacgaagacgtttacatgcctgaggtgtacaaagcgattaacattgcgcaaaacaccgcatggaaaatcaacaagaaagtcctagcggtcgccaacgtaatcaccaagtggaagcattgtccggtcgaggacatccctgcgattgagcgtgaagaactcccgatgaaaccggaagacatcgacatgaatcctgaggctctcaccgcgtggaaacgtgctgccgctgctgtgtaccgcaaggacaaggctcgcaagtctcgccgtatcagccttgagttcatgcttgagcaagccaataagtttgctaaccataaggccatctggttcccttacaacatggactggcgcggtcgtgtttacgctgtgtcaatgttcaacccgcaaggtaacgatatgaccaaaggactgcttacgctggcgaaaggtaaaccaatcggtaaggaaggttactactggctgaaaatccacggtgcaaactgtgcgggtgtcgacaaggttccgttccctgagcgcatcaagttcattgaggaaaaccacgagaacatcatggcttgcgctaagtctccactggagaacacttggtgggctgagcaagattctccgttctgcttccttgcgttctgctttgagtacgctggggtacagcaccacggcctgagctataactgctcccttccgctggcgtttgacgggtcttgctctggcatccagcacttctccgcgatgctccgagatgaggtaggtggtcgcgcggttaacttgcttcctagtgaaaccgttcaggacatctacgggattgttgctaagaaagtcaacgagattctacaagcagacgcaatcaatgggaccgataacgaagtagttaccgtgaccgatgagaacactggtgaaatctctgagaaagtcaagctgggcactaaggcactggctggtcaatggctggcttacggtgttactcgcagtgtgactaagagttcagtcatgacgctggcttacgggtccaaagagttcggcttccgtcaacaagtgctggaagataccattcagccagctattgattccggcaagggtctgatgttcactcagccgaatcaggctgctggatacatggctaagctgatttgggaatctgtgagcgtgacggtggtagctgcggttgaagcaatgaactggcttaagtctgctgctaagctgctggctgctgaggtcaaagataagaagactggagagattcttcgcaagcgttgcgctgtgcattgggtaactcctgatggtttccctgtgtggcaggaatacaagaagcctattcagacgcgcttgaacctgatgttcctcggtcagttccgcttacagcctaccattaacaccaacaaagatagcgagattgatgcacacaaacaggagtctggtatcgctcctaactttgtacacagccaagacggtagccaccttcgtaagactgtagtgtgggcacacgagaagtacggaatcgaatcttttgcactgattcacgactccttcggtacgattccggctgacgctgcgaacctgttcaaagcagtgcgcgaaactatggttgacacatatgagtcttgtgatgtactggctgatttctacgaccagttcgctgaccagttgcacgagtctcaattggacaaaatgccagcacttccggctaaaggtaacttgaacctccgtgacatcttagagtcggacttcgcgttcgcgtaa

SEQ ID NO: 223 - DNA, 3504 bp, synthetic construct; identical to SEQ ID NO: 2
  misc_feature 1..3504: note = synthetic Klebsiella pneumoniae nifJ
  source 1..3504: mol_type = other DNA

SEQ ID NO: 224 - DNA, 882 bp, synthetic construct; identical to SEQ ID NO: 4
  misc_feature 1..882: note = synthetic Klebsiella pneumoniae nifH
  source 1..882: mol_type = other DNA

SEQ ID NO: 225 - DNA, 1452 bp, synthetic construct
  misc_feature 1..1452: note = synthetic Klebsiella pneumoniae nifI
  source 1..1452: mol_type = other DNA
atgatgactaatgctactggcgaacgtaacctggcactgattcaagaagtactggaagtgttcccggaaaccgcgcgcaaagagcgccgtaaacacatgatggtttctgacccggaaatggaatctgtgggtaaatgcatcatctctaatcgcaaatctcagccgggtgtcatgactgttcgtggctgtgcgtacgcaggttctaaaggtgtcgtattcggcccgatcaaagatatggcgcatatctctcatggcccggtaggctgtggccagtactctcgcgcgggacgtcgtaactactacacgggcgtttctggcgttgactctttcggcacgctgaacttcacctctgacttccaggaacgtgacatcgttttcggtggcgataaaaagctgtccaaactgatcgaagaaatggaactgctgttcccgctgactaaaggcattactatccaaagcgaatgtccggtgggtctgatcggtgatgacatcagcgcggtcgcaaacgcatcttccaaagccctggataagccggtgatcccggttcgttgcgagggcttccgcggcgtttctcagtctctgggtcatcacatcgcaaacgatgttgtgcgtgactggattctgaacaaccgtgaaggtcagccttttgaaaccaccccttatgacgttgcgattattggcgactataacatcggcggcgacgcctgggcatcccgcatcctgctggaggagatgggtctgcgtgttgtcgcacagtggtctggcgatggcaccctggttgaaatggaaaacaccccgtttgttaaactgaacctggttcactgctaccgctccatgaactacattgcccgtcacatggaagaaaaacatcagatcccttggatggaatacaacttcttcggtccgactaaaatcgcagaatccctgcgtaaaatcgccgatcagtttgatgataccattcgcgcgaacgctgaagcagtaattgcgcgctacgaaggccagatggcagcaatcattgctaagtaccgtccgcgcctggaaggtcgtaaagtgctgctgtacatgggtggtctgcgtccacgtcatgtgatcggtgcctacgaggacctgggcatggagatcatcgcagcgggttacgaatttgcacacaacgacgactatgatcgtacgctgccagacctgaaagaaggtacgctgctgtttgacgacgccagctcttatgaactggaagccttcgtgaaagcgctgaaaccagacctgatcggctccggcatcaaggaaaaatacattttccagaaaatgggcgtgccgttccgccagatgcactcctgggactactccggtccgtaccacggctacgacggtttcgctatcttcgctcgtgacatggatatgaccctgaataacccagcgtggaatgaactgaccgcaccgtggctgaaatctgcataa

SEQ ID NO: 226 - DNA, 1563 bp, synthetic construct
  misc_feature 1..1563: note = synthetic Klebsiella pneumoniae nifK
  source 1..1563: mol_type = other DNA
atgtctcaaactatcgataaaatcaactcttgttacccgctgttcgagcaggacgaatatcaggaactgttccgtaacaaacgtcagctggaagaagcgcacgacgcacagcgcgtgcaggaagtgttcgcatggaccaccaccgcggaatacgaagctctgaacttccagcgcgaagccctgacggttgatccggcgaaagcgtgccagcctctgggtgcggttctgtgcagcctgggttttgccaacaccctgccgtatgtccacggttcccagggctgcgtagcctacttccgtacctatttcaaccgccactttaaagaaccaatcgcgtgcgtgtccgacagcatgacggaggacgcggcagttttcggtggtaacaacaacatgaacctgggcctgcaaaatgcttccgcactgtacaaaccggaaatcatcgcagtgtctaccacctgcatggcagaggttattggtgatgatctgcaagcatttattgccaacgcaaagaaagacggtttcgttgacagctctatcgcggttccgcacgctcataccccgtccttcatcggttctcacgtaactggttgggacaacatgttcgaaggcttcgcaaaaacttttaccgcagactatcaaggccaaccgggtaaactgccgaagctgaacctggtgaccggctttgaaacctacctgggcaactttcgtgtcctgaagcgcatgatggagcagatggcggttccgtgttctctgctgtctgacccgtctgaggttctggacactccagcggacggccactatcgcatgtattctggtggcaccactcagcaggaaatgaaagaggccccagacgcgattgacaccctgctgctgcaaccgtggcagctgctgaaaagcaagaaagttgttcaggaaatgtggaaccagccggcaacggaagttgcaatcccgctgggtctggcagctactgacgaactgctgatgaccgtgtcccaactgagcggcaaaccaatcgcggatgctctgaccctggaacgcggtcgcctggtggacatgatgctggacagccacacgtggctgcatggcaagaaatttggcctgtacggtgacccggacttcgtaatgggcctgacccgtttcctgctggaactgggctgcgagccgactgttatcctgtctcacaacgctaacaaacgttggcagaaggccatgaacaaaatgctggatgcgagcccatacggccgtgatagcgaagtgttcatcaactgcgacctgtggcatttccgctctctgatgtttacgcgtcagccggatttcatgatcggtaactcttacggcaaattcatccagcgtgacactctggccaaaggcaaagcgtttgaagtgccgctgattcgtctgggctttccgctgttcgaccgtcaccacctgcaccgccagaccacctggggttacgaaggcgcgatgaacatcgtaactactctggtaaacgcagtactggaaaagctggacagcgatacttcccagctgggcaaaaccgactattctttcgatctggttcgttaa

SEQ ID NO: 227 - DNA, 663 bp, synthetic construct
  misc_feature 1..663: note = synthetic Klebsiella pneumoniae nifY
  source 1..663: mol_type = other DNA
atgtctgacaatgataccctgttttggcgcatgctggcgctgtttcagtcgctgccggatttgcagccggctcaaatcgtcgattggctggcgcaggaatccggcgaaaccctgacgccggagcgccttgccaccctgacccaaccgcaactcgcggcgtcgttcccatccgcgacggcagtgatgagcccggctcgctggagccgcgttatggcttctctgcaaggcgccctcccagcccacttgcgcatcgtacgtccggcgcagcgtaccccgcaactgctcgccgcgttttgcagccaagacggccttgttatcaatggtcatttcggccagggtcgtctgttcttcatttacgcctttgacgagcagggcggctggctgtatgacttgcgccgctatccgagcgcaccgcaccagcaggaagcgaatgaggtgcgtgctcgtctgattgaagattgccagctgctgttctgccaggagattggcggtccggcagcagcgcgtctgatccgccaccgcatccatccgatgaaggcgcagccgggtactacgattcaggcgcagtgtgaagctatcaacaccctgctggccggtcgcctgccgccgtggctcgccaaacgtttgaaccgtgataacccgctggaagagcgtgtgttttaa

SEQ ID NO: 228 - DNA, 1374 bp, synthetic construct; identical to SEQ ID NO: 12
  misc_feature 1..1374: note = synthetic Klebsiella pneumoniae nifE
  source 1..1374: mol_type = other DNA

SEQ ID NO: 229 - DNA, 1386 bp, synthetic construct; identical to SEQ ID NO: 14
  misc_feature 1..1386: note = synthetic Klebsiella pneumoniae nifN
  source 1..1386: mol_type = other DNA

SEQ ID NO: 230 - DNA, 825 bp, synthetic construct; identical to SEQ ID NO: 16
  misc_feature 1..825: note = synthetic Klebsiella pneumoniae nifU
  source 1..825: mol_type = other DNA

SEQ ID NO: 231 - DNA, 1203 bp, synthetic construct; identical to SEQ ID NO: 94
  misc_feature 1..1203: note = synthetic Klebsiella pneumoniae nifS
  source 1..1203: mol_type = other DNA

SEQ ID NO: 232 - DNA, 1143 bp, synthetic construct
  misc_feature 1..1143: note = synthetic Klebsiella pneumoniae nifV
  source 1..1143: mol_type = other DNA
atggagcgcgtcttgatcaacgatactaccctgcgtgatggcgaacaatctccgggcgtagcgtttcgtacctccgagaaagttgccatcgcggaggcactgtacgctgcgggtatcaccgcgatggaagtcggcactccggcgatgggtgatgaagagatcgcccgcattcagctggtgcgtcgtcaactgccggacgcgacgcttatgacctggtgccgtatgaacgctctggaaatccgtcagagcgcggatctgggtattgactgggtggatatctcgatcccagcatccgacaagctgcgtcagtacaagctgcgtgagccgctggccgtgctgctggagcgccttgcgatgtttatccatctggcccacacgttaggcctcaaagtatgtattggttgcgaggatgcgagccgtgcgtctggtcagaccctgcgcgccattgccgaggtggcccagcaatgcgcggctgcgcgcttgcgttacgctgacaccgtgggcctgctggacccgttcaccaccgcagcccagatcagcgccctgcgtgacgtttggtcgggcgagatcgagatgcatgctcacaatgatctgggcatggctaccgcgaacacgctggcggcagtttcggctggcgccacgtcggtgaacactaccgtcctcggtctgggtgaacgtgcaggcaacgcagccctggaaaccgttgcgctgggcctggaacgctgcctgggcgtggaaaccggcgtccatttcagcgcgctcccagcgctctgtcagcgcgtcgcggaggctgcacagcgcgcaatcgacccgcaacagccgctggtgggtgaattggttttcacccacgagtctggtgttcacgttgcggcgctgctgcgcgacagcgaatcctatcaatctattgccccaagcctcatgggccgtagctaccgtctggtgctcggcaagcattcgggtcgtcaggctgtcaacggtgttttcgaccagatgggttaccacctgaatgcggcgcagatcaatcagttgctgccggccattcgccgcttcgccgagaattggaaacgctctccgaaagactacgaactggttgcgatctatgacgaattgtgcggtgaatccgcccttcgtgctcgcggctaa

SEQ ID NO: 233 - DNA, 258 bp, synthetic construct; identical to SEQ ID NO: 22
  misc_feature 1..258: note = synthetic Klebsiella pneumoniae nifW
  source 1..258: mol_type = other DNA

SEQ ID NO: 234 - DNA, 447 bp, synthetic construct; identical to SEQ ID NO: 24
  misc_feature 1..447: note = synthetic Klebsiella pneumoniae nifZ
  source 1..447: mol_type = other DNA

SEQ ID NO: 235 - DNA, 801 bp, synthetic construct; identical to SEQ ID NO: 26
  misc_feature 1..801: note = synthetic Klebsiella pneumoniae nifM
  source 1..801: mol_type = other DNA

SEQ ID NO: 236 - DNA, 531 bp, synthetic construct; identical to SEQ ID NO: 28
  misc_feature 1..531: note = synthetic Klebsiella pneumoniae nifF
  source 1..531: mol_type = other DNA

SEQ ID NO: 237 - DNA, 1407 bp, synthetic construct; identical to SEQ ID NO: 30
  misc_feature 1..1407: note = synthetic Klebsiella pneumoniae nifB
  source 1..1407: mol_type = other DNA

SEQ ID NO: 238 - DNA, 504 bp, synthetic construct; identical to SEQ ID NO: 32
  misc_feature 1..504: note = synthetic Klebsiella pneumoniae nifQ
  source 1..504: mol_type = other DNA

SEQ ID NO: 239 - protein, 206 aa, synthetic construct
  REGION 1..206: note = synthetic chimeric sigma factor ECF11_ECF02
MRITASLRTFCHLSTPHSDSTTSRLWIDEVTAVARQRDRDSFMRIYDHFAPRLLRYLTGLNVPEGQAEELVQEVLLKLWHKAESFDPSKASLGTWLFRIARNLYIDSVRKDRGWVQVQNSLEQLERLEAISNPENLMLSEELRQIVFRTIESLPEDLRMAITLRELDGLSYEEIAAIMDCPVGTVRSRIFRAREAIDNKVQPLIRR

SEQ ID NO: 240 - protein, 187 aa, synthetic construct
  REGION 1..187: note = synthetic chimeric sigma factor ECF02_ECF11
MSEQLTDQVLVERVQKGDQKAFNLLVVRYQHKVASLVSRYVPSGDVPDVVQEAFIKAYRALDSFRGDSAFYTWLYRIAVNTAKNYLVAQGRRPPSSDVDAIEAENFEQLERLEAPVDRTLDYSQRQEQQLNSAIQNLPTDQAKVLRMSYFEALSHREISERLDMPLGTVKSCLRLAFQKLRSRIEES

SEQ ID NO: 241 - protein, 883 aa, Enterobacteria phage T7
  REGION 1..883: note = Enterobacteria phage T7 RNA polymerase (RNAP)
MNTINIAKNDFSDIELAAIPFNTLADHYGERLAREQLALEHESYEMGEARFRKMFERQLKAGEVADNAAAKPLITTLLPKMIARINDWFEEVKAKRGKRPTAFQFLQEIKPEAVAYITIKTTLACLTSADNTTVQAVASAIGRAIEDEARFGRIRDLEAKHFKKNVEEQLNKRVGHVYKKAFMQVVEADMLSKGLLGGEAWSSWHKEDSIHVGVRCIEMLIESTGMVSLHRQNAGVVGQDSETIELAPEYAEAIATRAGALAGISPMFQPCVVPPKPWTGITGGGYWANGRRPLALVRTHSKKALMRYEDVYMPEVYKAINIAQNTAWKINKKVLAVANVITKWKHCPVEDIPAIEREELPMKPEDIDMNPEALTAWKRAAAAVYRKDKARKSRRISLEFMLEQANKFANHKAIWFPYNMDWRGRVYAVSMFNPQGNDMTKGLLTLAKGKPIGKEGYYWLKIHGANCAGVDKVPFPERIKFIEENHENIMACAKSPLENTWWAEQDSPFCFLAFCFEYAGVQHHGLSYNCSLPLAFDGSCSGIQHFSAMLRDEVGGRAVNLLPSETVQDIYGIVAKKVNEILQADAINGTDNEVVTVTDENTGEISEKVKLGTKALAGQWLAYGVTRSVTKRSVMTLAYGSKEFGFRQQVLEDTIQPAIDSGKGLMFTQPNQAAGYMAKLIWESVSVTVVAAVEAMNWLKSAAKLLAAEVKDKKTGEILRKRCAVHWVTPDGFPVWQEYKKPIQTRLNLMFLGQFRLQPTINTNKDSEIDAHKQESGIAPNFVHSQDGSHLRKTVVWAHEKYGIESFALIHDSFGTIPADAANLFKAVRETMVDTYESCDVLADFYDQFADQLHESQLDKMPALPAKGNLNLRDILESDFAFA

SEQ ID NO: 242 - DNA, 48 bp, synthetic construct
  misc_feature 1..48: note = synthetic Enterobacteria phage T7 stem loop terminator seed sequence
  modified_base 3..6: mod_base = OTHER; note = n = g, a, c or t
  source 1..48: mol_type = other DNA
tannnnaaccsswwsssssstcwwwwcgsssssswwssggttttttgt

SEQ ID NO: 243 - DNA, 29 bp, synthetic construct
  misc_feature 1..29: note = synthetic Enterobacteria phage T7 terminator 52
  source 1..29: mol_type = other DNA
tataaaacggggggctaggggttttttgt

SEQ ID NO: 244 - DNA, 48 bp, synthetic construct
  misc_feature 1..48: note = synthetic Enterobacteria phage T7 terminator 23
  source 1..48: mol_type = other DNA
tactcgaacccctagcccgctcttatcgggcggctaggggttttttgt

SEQ ID NO: 245 - DNA, 37 bp, synthetic construct
  misc_feature 1..37: note = synthetic Enterobacteria phage T7 terminator 72
  source 1..37: mol_type = other DNA
tagcagaaccgctaacgggggcgaaggggttttttgt

SEQ ID NO: 246 - DNA, 48 bp, synthetic construct; identical to SEQ ID NO: 244
  misc_feature 1..48: note = synthetic Enterobacteria phage T7 terminator 48
  source 1..48: mol_type = other DNA

SEQ ID NO: 247 - DNA, 29 bp, synthetic construct
  misc_feature 1..29: note = synthetic Enterobacteria phage T7 terminator 1
  source 1..29: mol_type = other DNA
tacatatcgggggggtaggggttttttgt

SEQ ID NO: 248 - DNA, 29 bp, synthetic construct
  misc_feature 1..29: note = synthetic Enterobacteria phage T7 terminator 2
  source 1..29: mol_type = other DNA
tacatatcgggggggtaggggttttttgt

SEQ ID NO: 249 - DNA, 48 bp, synthetic construct; identical to SEQ ID NO: 183
  misc_feature 1..48: note = synthetic Enterobacteria phage T7 wild type (WT) terminator
  source 1..48: mol_type = other DNA

SEQ ID NO: 250 - DNA, 47 bp, synthetic construct
  misc_feature 1..47: note = synthetic Enterobacteria phage T7 terminator 31
  source 1..47: mol_type = other DNA
taccctaaccccttccccggtcaatcggggcggatggggttttttgt

SEQ ID NO: 251 - DNA, 47 bp, synthetic construct
  misc_feature 1..47: note = synthetic Enterobacteria phage T7 terminator 58
  source 1..47: mol_type = other DNA
tagaccaaccccttgcggcctcaatcgggggggatggggttttttgt

SEQ ID NO: 252 - DNA, 37 bp, synthetic construct; identical to SEQ ID NO: 72
  misc_feature 1..37: note = synthetic Enterobacteria phage T7 terminator 25
  source 1..37: mol_type = other DNA

SEQ ID NO: 253 - DNA, 48 bp, synthetic construct
  misc_feature 1..48: note = synthetic Enterobacteria phage T7 terminator 17
  source 1..48: mol_type = other DNA
tacctcaaccccttccgccctcatatcgcggggcatgcggttttttgt

SEQ ID NO: 254 - protein, 39 aa, synthetic construct
  REGION 1..39: note = synthetic Enterobacteria phage T7 RNA polymerase (RNAP) specificity loop sequence
VWQEYKKPIQTRLNLMFLGQFRLQPTINTNKDSEIDAHK

SEQ ID NO: 255 - protein, 39 aa, synthetic construct
  REGION 1..39: note = synthetic Enterobacteria phage T3 RNA polymerase (RNAP) specificity loop sequence
VWQEYKKPIQKRLDMIFLGQFRLQPTINTNKDSEIDAHK

SEQ ID NO: 256 - DNA, 23 bp, synthetic construct
  misc_feature 1..23: note = synthetic Enterobacteria phage T3 RNA polymerase (RNAP) promoter sequence
  source 1..23: mol_type = other DNA
taataaccctcactatagggaga

SEQ ID NO: 257 - protein, 39 aa, synthetic construct
  REGION 1..39: note = synthetic Enterobacteria phage K1F RNA polymerase (RNAP) specificity loop sequence
VWQEYKKPIQTRLNLMFLGSFNLQPTVNTNKDSEIDAHK

SEQ ID NO: 258 - DNA, 23 bp, synthetic construct
  misc_feature 1..23: note = synthetic Enterobacteria phage K1F RNA polymerase (RNAP) promoter sequence
  source 1..23: mol_type = other DNA
taataactatcactatagggaga

SEQ ID NO: 259 - protein, 39 aa, synthetic construct
  REGION 1..39: note = synthetic Enterobacteria phage N4 RNA polymerase (RNAP) specificity loop sequence
VWQEYKKPIQTRIDCVILGTHRMALTINTNKDSEIDAHK

SEQ ID NO: 260 - DNA, 23 bp, synthetic construct
  misc_feature 1..23: note = synthetic Enterobacteria phage N4 RNA polymerase (RNAP) promoter sequence
  source 1..23: mol_type = other DNA
taataacccacactatagggaga

SEQ ID NO: 261 - DNA, 498 bp, Salmonella typhimurium
  misc_feature 1..498: note = transcriptional activator sicA
  source 1..498: mol_type = other DNA
atggattatcaaaataatgtcagcgaagaacgtgttgcggaaatgatttgggatgccgttagtgaaggcgccacgctaaaagacgttcatgggatccctcaagatatgatggacggtttatatgctcatgcttatgagttttataaccagggacgactggatgaagctgagacgttctttcgtttcttatgcatttatgatttttacaatcccgattacaccatgggactggcggcagtatgccaactgaaaaaacaatttcagaaagcatgtgacctttatgcagtagcgtttacgttacttaaaaatgattatcgccccgttttttttaccgggcagtgtcaattattaatgcgtaaggcagcaaaagccagacagtgttttgaacttgtcaatgaacgtactgaagatgagtctctgcgggcaaaagcgttggtctatctggaggcgctaaaaacggcggagacagagcagcacagtgaacaagaaaaggaataa

SEQ ID NO: 262 - DNA, 498 bp, synthetic construct
  misc_feature 1..498: note = synthetic Salmonella typhimurium mutant transcriptional activator sicA*
  source 1..498: mol_type = other DNA
atggattatcaaaataatgtcagcgaagaacgtgttgcggaaatgatttgggatgccgttagtgaaggcgccacgctaaaagacgttcatgggatccctcaagatatgatggacggtttatatgctcatgcttatgagttttataaccagggacgactggatgaagctgagacgttctttcgttacttatgcatttatgatttttacaatcccgattacaccatgggactggcggcagtatgccaactgaaaaaacaatttcagaaagcatgtgacctttatgcagtagcgtttacgttacttaaaaatgattatcgccccgttttttttaccgggcagtgtcaattattaatgcgtaaggcagcaaaagccagacagtgttttgaacttgtcaatgaacgtactgaagatgagtctctgcgggcaaaagcgttggtctatctggaggcgctaaaaacggcggagacagagcagcacagtgaacaagaaaaggaataa

SEQ ID NO: 263 - DNA, 750 bp, Salmonella typhimurium
  misc_feature 1..750: note = transcriptional activator invF with new start codon
  source 1..750: mol_type = other DNA
atgctaaatacgcaggaagtacttaaagaaggagagaagcggaaaatccgcagcccggaagcatggtttatacagacgtgttccgcgcaaaagctgcatatgtcattttctgaaagccgacacaatgaaaattgcctgattcaggaaggcgcgctgcttttttgcgagcaggccgttgtcgcaccagtatcaggagacctggtttttcgaccgttaaaaattgaagtactcagcaaattactggcatttatcgatggcgcaggattagtggacacgacatatgctgaatccgataaatgggttttgctgagtcctgagtttcgcgctatttggcaagatcgtaaacgctgcgagtactggtttttgcagcaaattattacgccttctccggccttcaataaggtactggcgctgttacgaaaaagcgagagttactggttggttggctatttactcgctcagtcaaccagcggcaacacgatgagaatgctgggagaagactatggcgtttcttatacccattttcgtcgtttgtgcagcagagcgttgggcggaaaagcgaagagtgaattacgaaactggcgtatggcgcaatcgctgctgaatagtgtagaaggccacgagaacatcacccaattagccgttaatcatggttactcatcgccttcacatttttctagtgagatcaaagagctgatcggcgtttcgccgcggaaattatcaaatattattcaattggcagacaaatga

SEQ ID NO: 264 - DNA, 163 bp, synthetic construct
  misc_feature 1..163: note = synthetic promoter psicA
  source 1..163: mol_type = other DNA
ccacaagaaacgaggtacggcattgagccgcgtaaggcagtagcgatgtattcattgggcgttttttgaatgttcactaaccaccgtcggggtttaataactgcatcagataaacgcagtcgttaagttctacaaagtcggtgacagataacaggagtaagta

SEQ ID NO: 265 - DNA, 468 bp, Shigella flexneri
  misc_feature 1..468: note = transcriptional activator ipgC
  source 1..468: mol_type = other DNA
atgtctttaaatatcaccgaaaatgaaagcatctctactgcagtaattgatgcaattaactctggcgctacactgaaagatattaatgcaattcctgatgatatgatggatgacatttattcatatgcttatgacttttacaacaaaggaagaatagaggaagctgaagttttcttcaggtttttatgtatatacgacttttacaatgtagactacattatgggactcgcagctatttatcagataaaagaacagttccaacaagcagcagacctttatgctgtcgcttttgcattaggaaaaaatgactatacaccagtattccatactggacaatgtcagcttcggttgaaagcccccttaaaagctaaagagtgcttcgaactcgtaattcaacacagcaatgatgaaaaattaaaaataaaagcacaatcatacttggacgcaattcaggatatcaaggagtaa

SEQ ID NO: 266 - DNA, 756 bp, synthetic construct
  misc_feature 1..756: note = synthetic codon optimized Shigella flexneri mxiE
  source 1..756: mol_type = other DNA
atgagtaaatataaaggcctgaacaccagcaacatgttctacatctacagctctggtcatgaaccggtgaacgttgaactggtgaaagataaagaacgtaacatcatcgaactggcaccggcgtggaaaggctttttctttgtgcgtaaccagaacatcaaattcagcgataacgttaactaccactaccgcttcaacatcaactcttgcgcaaaattcctggcgttttgggattattttagcggcgccctggttgaacattctcacgcagaaaaatgcatccatttctaccacgaaaacgatctgcgtgatagctgtaatacggaatctatgctggataaactgatgctgcgcttcatttttagtagcgatcagaacgtgtctaatgccctggcaatgatccgtatgaccgaaagttatcatctggttctgtacctgctgcgtacgattgaaaaagaaaaagaagtgcgcatcaaaagcctgaccgaacactatggcgtttctgaagcgtactttcgtagtctgtgtcgcaaagcgctgggtgccaaagtgaaagaacagctgaacacgtggcgcctggtgaatggcctgctggatgttttcctgcataaccagaccattacgagcgcggccatgaacaatggttatgcgtctaccagtcacttcagcaatgaaattaaaacgcgtctgggctttagtgcccgcgaactgagcaacatcaccttcctggtgaagaaaattaatgaaaaaatctaa

SEQ ID NO: 267 - DNA, 350 bp, synthetic construct
  misc_feature 1..350: note = synthetic promoter pipaH9.8
  source 1..350: mol_type = other DNA
gcgaaaatgacatcaaaaacgccattaacctgatgttctggggaatataaatgtcaggctagggtcaaaaatcgtggcgttgacaaaatggctgcgttacgtcattgagcatatccaggactggccggcaaaccgggtacgcgatctgttgccttggaaagttgatctgacctctcagtaaatatcaatacggttctgacgagccgcttaccgttcaaatatgaagtacgatgtttaactaaccgaaaaacaagaacaatacggtgcaaacaggccattcacggttaactgaaacagtatcgtttttttacagccaattttgtttatccttattataataaaaaagtgct

SEQ ID NO: 268 - DNA, 350 bp, synthetic construct
  misc_feature 1..350: note = synthetic promoter pipaH9.8* with mutation
  source 1..350: mol_type = other DNA
gcgaaaatgacatcaaaaacgccattaacctgatgttctggggaatataaatgtcaggctagggtcaaaaatcgtggcgttgacaaaatggctgcgttacgtcattgagcatatccaggactggccggcaaaccgggtacgcgatctgttgccttggaaagttgatctgacctctcagtaaatatcaatacggttctgacgagccgcttaccgttcaaatatgaagtacgatgtttaactaaccgaaaaacaagaacaatacggtgcaaacaggccattcacggttaactgaaacagtatcgtttttttacagccaattttgtttatccttattaagataaaaaagtgct

SEQ ID NO: 269 - DNA, 438 bp, Pseudomonas aeruginosa
  misc_feature 1..438: note = transcriptional activator exsC
  source 1..438: mol_type = other DNA
atggatttaacgagcaaggtcaaccgactgcttgccgagttcgcaggccgtatcggtttgccttccctgtccctcgacgaggagggcatggcgagcctcctgttcgacgaacaggtgggcgtcaccctgttgctgctcgccgagcgcgagcgtctgttgctggaggccgatgtggcgggcatcgatgtgctgggcgaggggatctttcgccagctcgccagcttcaaccgccattggcaccgtttcgatctgcatttcggcttcgacgagctgaccggcaaggtccagttgtatgcgcagattctcgcagcgcaactgaccctcgaatgcttcgaggcgaccttggccaatctgctcgatcacgccgagttctggcagcgcctgctgccgtgcgacagtgatcgcgaggcggtcgctgcggtcggcatgagggtttga

SEQ ID NO: 270 - DNA, 831 bp, Pseudomonas aeruginosa
  misc_feature 1..831: note = transcriptional activator exsD
  source 1..831: mol_type = other DNA
atggagcaggaagacgataagcagtactcccgagaagcggtgttcgctggcaggcgggtatccgtggtgggctcggacgcccgctcgcggggtcgggtgccgggttacgcatcgagcagtttgtatcgtgagtccggaatcatcagtgcgcggcaactggcgttgctgcagcggatgctgccgcgcctgcggctggagcaactgttccgctgcgagtggttgcagcagcgcctggcgcgcggcctggcgctggggcgcgaagaggtgcggcagattctcctctgcgcggcgcaggacgacgacggctggtgctccgaactgggcgaccgggtcaacctcgccgtgccgcagtcgatgatcgactgggtcctgctgccggtctatggctggtgggaaagcctgctcgaccaggcgatccccggctggcgcctgtcgctggtggagctggagacccagtcccggcaactgcgagtcaagtccgaattctggtcccgcgtggccgagctggagccggagcaggcccgcgaggaactggccagggtcgccaagtgccaggcgcgcacccaggaacaggtggccgaactggccggcaagctggagacggcttcggcactggcgaagagcgcctggccgaactggcagcggggcatggcgacgctgctcgccagcggcgggctggccggcttcgagccgatccccgaggtcctcgaatgcctctggcaacctctctgccggctggacgacgacgtcggcgcggcggacgccgtccaggcctggctgcacgaacgcaacctgtgccaggcacaggatcacttctactggcagagctga

SEQ ID NO: 271 - DNA, 837 bp, Pseudomonas aeruginosa
  misc_feature 1..837: note = transcriptional activator exsA
  source 1..837: mol_type = other DNA
atgcaaggagccaaatctcttggccgaaagcagataacgtcttgtcattggaacattccaactttcgaatacagggtaaacaaggaagagggcgtatatgttctgctcgagggcgaactgaccgtccaggacatcgattccactttttgcctggcgcctggcgagttgcttttcgtccgccgcggaagctatgtcgtaagtaccaagggaaaggacagccgaatactctggattccattatctgcccagtttctacaaggcttcgtccagcgcttcggcgcgctgttgagtgaagtcgagcgttgcgacgagcccgtgccgggcatcatcgcgttcgctgccacgcctctgctggccggttgcgtcaaggggttgaaggaattgcttgtgcatgagcatccgccgatgctcgcctgcctgaagatcgaggagttgctgatgctcttcgcgttcagtccgcaggggccgctgctgatgtcggtcctgcggcaactgagcaaccggcatgtcgagcgtctgcagctattcatggagaagcactacctcaacgagtggaagctgtccgacttctcccgcgagttcggcatggggctgaccaccttcaaggagctgttcggcagtgtctatggggtttcgccgcgcgcctggatcagcgagcggagaatcctctatgcccatcagttgctgctcaacagcgacatgagcatcgtcgacatcgccatggaggcgggcttttccagtcagtcctatttcacccagagctatcgccgccgtttcggctgcacgccgagccgctcgcggcaggggaaggacgaatgccgggctaaaaataactga

SEQ ID NO: 272 - DNA, 80 bp, synthetic construct
  misc_feature 1..80: note = synthetic pesxD promoter
  source 1..80: mol_type = other DNA
gaaggacgaatgccgggctaaaaataactgacgttttttgaaagcccggtagcggctgcatgagtagaatcggcccaaat

SEQ ID NO: 273 - DNA, 80 bp, synthetic construct
  misc_feature 1..80: note = synthetic pexsC promoter
  source 1..80: mol_type = other DNA
gatgtggcttttttcttaaaagaaaagtctctcagtgacaaaagcgatgcatagcccggtgctagcatgcgctgagcttt

SEQ ID NO: 274 - DNA, 702 bp, synthetic construct
  misc_feature 1..702: note = synthetic red fluorescence protein (rfp, RFP)
  source 1..702: mol_type = other DNA
atggcttcctccgaagacgttatcaaagagttcatgcgtttcaaagttcgtatggaaggttccgttaacggtcacgagttcgaaatcgaaggtgaaggtgaaggtcgtccgtacgaaggtacgcagaccgctaaactgaaagttaccaaaggtggtccgctgccgttcgcttgggacatcctgtccccgcagttccagtacggttccaaagcttacgttaaacacccggctgacatcccggactacctgaaactgtccttcccggaaggtttcaaatgggaacgtgttatgaacttcgaagacggtggtgttgttaccgttacccaggactcctccctgcaagacggtgagttcatctacaaagttaaactgcgtggtactaacttcccgtccgacggtccggttatgcagaaaaaaaccatgggttgggaagcttccaccgaacgtatgtacccggaagacggtgctctgaaaggtgaaatcaaaatgcgtctgaaactgaaagacggtggtcactacgacgctgaagttaaaaccacctacatggctaaaaaaccggttcagctgccgggtgcttacaaaaccgacatcaaactggacatcacctcccacaacgaagactacaccatcgttgaacagtacgaacgtgctgaaggtcgtcactccaccggtgctgcagcaaacgacgaaaactacgcttaa

SEQ ID NO: 275 - DNA, 43 bp, synthetic construct
  misc_feature 1..43: note = synthetic T5 phage buffer sequence
  source 1..43: mol_type = other DNA
agttcgatgagagcgataaccctctacaaataattttgtttaa

SEQ ID NO: 276 - DNA, 42 bp, synthetic construct
  misc_feature 1..42: note = synthetic T5 phage buffer sequence
  source 1..42: mol_type = other DNA
ataaattgataaacaaaaacctctacaaataattttgtttaa

SEQ ID NO: 277 - DNA, 43 bp, synthetic construct
  misc_feature 1..43: note = synthetic T5 phage buffer sequence
  source 1..43: mol_type = other DNA
ataaatttgagagaggagttcctctacaaataattttgtttaa

SEQ ID NO: 278 - DNA, 43 bp, synthetic construct
  misc_feature 1..43: note = synthetic T5 phage buffer sequence
  source 1..43: mol_type = other DNA
attaaagaggagaaattaaccctctacaaataattttgtttaa

SEQ ID NO: 279 - DNA, 43 bp, synthetic construct
  misc_feature 1..43: note = synthetic T7 phage buffer sequence
  source 1..43: mol_type = other DNA
aaacctaatggatcgaccttcctctacaaataattttgtttaa

SEQ ID NO: 280 - DNA, 42 bp, synthetic construct
  misc_feature 1..42: note = synthetic T7 phage buffer sequence
  source 1..42: mol_type = other DNA
atcgagagggacacggcgacctctacaaataattttgtttaa

SEQ ID NO: 281 - DNA, 42 bp, synthetic construct
  misc_feature 1..42: note = synthetic T7 phage buffer sequence
  source 1..42: mol_type = other DNA
gctaggtaacactagcagccctctacaaataattttgtttaa

SEQ ID NO: 282 - DNA, 42 bp, synthetic construct
  misc_feature 1..42: note = synthetic T7 phage buffer sequence
  source 1..42: mol_type = other DNA
atgaaacgacagtgagtcacctctacaaataattttgtttaa

SEQ ID NO: 283 - DNA, 43 bp, synthetic construct
  misc_feature 1..43: note = synthetic T7 phage buffer sequence
  source 1..43: mol_type = other DNA
agggagaccacaacggtttccctctacaaataattttgtttaa

SEQ ID NO: 284 - DNA, 43 bp, synthetic construct
  misc_feature 1..43: note = synthetic high-transcription escape buffer sequence
  source 1..43: mol_type = other DNA
attaaaaaacctgctaggatcctctacaaataattttgtttaa

SEQ ID NO: 285 - DNA, 43 bp, synthetic construct
  misc_feature 1..43: note = synthetic high-transcription escape buffer sequence
  source 1..43: mol_type = other DNA
ataaaggaaaacggtcaggtcctctacaaataattttgtttaa

SEQ ID NO: 286 - DNA, 43 bp, synthetic construct
  misc_feature 1..43: note = synthetic high-transcription escape buffer sequence
  source 1..43: mol_type = other DNA
ataggttaaaagcctgtcatcctctacaaataattttgtttaa

SEQ ID NO: 287 - DNA, 48 bp, synthetic construct
  misc_feature 1..48: note = synthetic carbon utilization buffer sequence
  source 1..48: mol_type = other DNA
acaataaaaaatcatttacatgtttcctctacaaataattttgtttaa

SEQ ID NO: 288 - DNA, 48 bp, synthetic construct
  misc_feature 1..48: note = synthetic carbon utilization buffer sequence
  source 1..48: mol_type = other DNA
agaagcagcgcgcaaaaatcagctgcctctacaaataattttgtttaa

SEQ ID NO: 289 - DNA, 48 bp, synthetic construct
  misc_feature 1..48: note = synthetic carbon utilization buffer sequence
  source 1..48: mol_type = other DNA
atgagttcatttcagacaggcaaatcctctacaaataattttgtttaa

SEQ ID NO: 290 - DNA, 48 bp, synthetic construct
  misc_feature 1..48: note = synthetic carbon utilization buffer sequence
  source 1..48: mol_type = other DNA
aacttgcagttatttactgtgattacctctacaaataattttgtttaa

SEQ ID NO: 291 - DNA, 48 bp, synthetic construct
  misc_feature 1..48: note = synthetic carbon utilization buffer sequence
  source 1..48: mol_type = other DNA
agccacaaaaaaagtcatgttggttcctctacaaataattttgtttaa

SEQ ID NO: 292 - DNA, 53 bp, synthetic construct
  misc_feature 1..53: note = synthetic carbon utilization buffer sequence
  source 1..53: mol_type = other DNA
acacagtcacttatcttttagttaaaaggtcctctacaaataattttgtttaa

SEQ ID NO: 293 - DNA, 43 bp, synthetic construct
  misc_feature 1..43: note = synthetic anti-escaping buffer sequence
  source 1..43: mol_type = other DNA
atccggaatcctcttcccggcctctacaaataattttgtttaa

SEQ ID NO: 294 - DNA, 48 bp, synthetic construct
  misc_feature 1..48: note = synthetic anti-escaping buffer sequence
  source 1..48: mol_type = other DNA
aacaaaataaaaaggagtcgctcaccctctacaaataattttgtttaa

SEQ ID NO: 295 - DNA, 43 bp, synthetic construct
  misc_feature 1..43: note = synthetic T5 phage buffer sequence
  source 1..43: mol_type = other DNA
agttcgatgagagcgataacagttccagattcaggaactataa

SEQ ID NO: 296 - DNA, 42 bp, synthetic construct
  misc_feature 1..42: note = synthetic T5 phage buffer sequence
  source 1..42: mol_type = other DNA
ataaattgataaacaaaaaagttccagattcaggaactataa

SEQ ID NO: 297 - DNA, 43 bp, synthetic construct
  misc_feature 1..43: note = synthetic T5 phage buffer sequence
  source 1..43: mol_type = other DNA
ataaatttgagagaggagttagttccagattcaggaactataa

SEQ ID NO: 298 - DNA, 43 bp, synthetic construct
  misc_feature 1..43: note = synthetic T5 phage buffer sequence
  source 1..43: mol_type = other DNA
attaaagaggagaaattaacagttccagattcaggaactataa

SEQ ID NO: 299 - DNA, 43 bp, synthetic construct
  misc_feature 1..43: note = synthetic T5 phage buffer sequence
  source 1..43: mol_type = other DNA
aaacctaatggatcgaccttagttccagattcaggaactataa

SEQ ID NO: 300 - DNA, 42 bp, synthetic construct
  misc_feature 1..42: note = synthetic T7 phage buffer sequence
  source 1..42: mol_type = other DNA
atcgagagggacacggcgaagttccagattcaggaactataa

SEQ ID NO: 301 - DNA, 42 bp, synthetic construct
  misc_feature 1..42: note = synthetic T7 phage buffer sequence
  source 1..42: mol_type = other DNA
gctaggtaacactagcagcagttccagattcaggaactataa

SEQ ID NO: 302 - DNA, 42 bp, synthetic construct
  misc_feature 1..42: note = synthetic T7 phage buffer sequence
  source 1..42: mol_type = other DNA
atgaaacgacagtgagtcaagttccagattcaggaactataa

SEQ ID NO: 303 - DNA, 43 bp, synthetic construct
  misc_feature 1..43: note = synthetic T7 phage buffer sequence
  source 1..43: mol_type = other DNA
agggagaccacaacggtttcagttccagattcaggaactataa

SEQ ID NO: 304 - DNA, 43 bp, synthetic construct
  misc_feature 1..43: note = synthetic high-transcription escape buffer sequence
  source 1..43: mol_type = other DNA
attaaaaaacctgctaggatagttccagattcaggaactataa

SEQ ID NO: 305 - DNA, 43 bp, synthetic construct
  misc_feature 1..43: note = synthetic high-transcription escape buffer sequence
  source 1..43: mol_type = other DNA
ataaaggaaaacggtcaggtagttccagattcaggaactataa

SEQ ID NO: 306 - DNA, 43 bp, synthetic construct
  misc_feature 1..43: note = synthetic high-transcription escape buffer sequence
  source 1..43: mol_type = other DNA
ataggttaaaagcctgtcatagttccagattcaggaactataa

SEQ ID NO: 307 - DNA, 48 bp, synthetic construct
  misc_feature 1..48: note = synthetic carbon utilization buffer sequence
  source 1..48: mol_type = other DNA
acaataaaaaatcatttacatgtttagttccagattcaggaactataa

SEQ ID NO: 308 - DNA, 48 bp, synthetic construct
  misc_feature 1..48: note = synthetic carbon utilization buffer sequence
  source 1..48: mol_type = other DNA
agaagcagcgcgcaaaaatcagctgagttccagattcaggaactataa

SEQ ID NO: 309 - DNA, 48 bp, synthetic construct
  misc_feature 1..48: note = synthetic carbon utilization buffer sequence
  source 1..48: mol_type = other DNA
atgagttcatttcagacaggcaaatagttccagattcaggaactataa

SEQ ID NO: 310 - DNA, 48 bp, synthetic construct
  misc_feature 1..48: note = synthetic carbon utilization buffer sequence
  source 1..48: mol_type = other DNA
aacttgcagttatttactgtgattaagttccagattcaggaactataa

SEQ ID NO: 311 - DNA, 48 bp, synthetic construct
  misc_feature 1..48: note = synthetic carbon utilization buffer sequence
  source 1..48: mol_type = other DNA
agccacaaaaaaagtcatgttggttagttccagattcaggaactataa

SEQ ID NO: 312 - DNA, 53 bp, synthetic construct
  misc_feature 1..53: note = synthetic carbon utilization buffer sequence
  source 1..53: mol_type = other DNA
acacagtcacttatcttttagttaaaaggtagttccagattcaggaactataa

SEQ ID NO: 313 - DNA, 43 bp, synthetic construct
  misc_feature 1..43: note = synthetic anti-escaping buffer sequence
  source 1..43: mol_type = other DNA
atccggaatcctcttcccggagttccagattcaggaactataa

SEQ ID NO: 314 - DNA, 48 bp, synthetic construct
  misc_feature 1..48: note = synthetic anti-escaping buffer sequence
  source 1..48: mol_type = other DNA
aacaaaataaaaaggagtcgctcacagttccagattcaggaactataa

SEQ ID NO: 315 - DNA, 30 bp, synthetic construct
  misc_feature 1..30: note = synthetic stem loops buffer sequence
  source 1..30: mol_type = other DNA
gatcaccagggggatcccccggtgaaggat

SEQ ID NO: 316 - DNA, 38 bp, synthetic construct
  misc_feature 1..38: note = synthetic stem loops buffer sequence
  source 1..38: mol_type = other DNA
gatcgcccaccggcagctgccggtgggcgatcaaggat

SEQ ID NO: 317 - DNA, 45 bp, synthetic construct
  misc_feature 1..45: note = synthetic stem loops buffer sequence
  source 1..45: mol_type = other DNA
gatcatcggtagagttaatattgagcagatcccccggtgaaggat

SEQ ID NO: 318 - DNA, 36 bp, synthetic construct
  misc_feature 1..36: note = synthetic stem loops buffer sequence
  source 1..36: mol_type = other DNA
attgatctggttattaaaggtaatcgggtcatttta

SEQ ID NO: 319 - DNA, 41 bp, synthetic construct
  misc_feature 1..41: note = synthetic stem loops buffer sequence
  source 1..41: mol_type = other DNA
gttctccacgggtgggatgagcccctcgtggtggaaatgcg

SEQ ID NO: 320 - DNA, 27 bp, synthetic construct
  misc_feature 1..27: note = synthetic stem loops buffer sequence
  source 1..27: mol_type = other DNA
agcatgaggtaaagtgtcatgcaccaa

SEQ ID NO: 321 - DNA, 38 bp, synthetic construct
  misc_feature 1..38: note = synthetic stem loops buffer sequence
  source 1..38: mol_type = other DNA
acgtcgacttatctcgagtgagatattgttgacggtac

SEQ ID NO: 322 - DNA, 37 bp, synthetic construct
  misc_feature 1..37: note = synthetic stem loops buffer sequence
  source 1..37: mol_type = other DNA
acgtcgacttatctcgagtgagataagttgacggtac

SEQ ID NO: 323 - DNA, 51 bp, synthetic construct
  misc_feature 1..51: note = synthetic stem loops buffer sequence
  source 1..51: mol_type = other DNA
acgtcgacttatctcgagactgcagttcaatagagatattgttgacggtac

SEQ ID NO: 324 - DNA, 52 bp, synthetic construct
  misc_feature 1..52: note = synthetic stem loops (ribozyme) buffer sequence
  source 1..52: mol_type = other DNA
gactgtcaccggatgtgctttccggtctgatgagtccgtgaggacgaaacag

SEQ ID NO: 325 - DNA, 53 bp, synthetic construct
  misc_feature 1..53: note = synthetic stem loops buffer sequence
  source 1..53: mol_type = other DNA
gatcaccagggggatcccccggtgaaggatcctctacaaataattttgtttaa

SEQ ID NO: 326 - DNA, 61 bp, synthetic construct
  misc_feature 1..61: note = synthetic stem loops buffer sequence
  source 1..61: mol_type = other DNA
gatcgcccaccggcagctgccggtgggcgatcaaggatcctctacaaataattttgtttaa

SEQ ID NO: 327 - DNA, 68 bp, synthetic construct
  misc_feature 1..68: note = synthetic stem loops buffer sequence
  source 1..68: mol_type = other DNA
gatcatcggtagagttaatattgagcagatcccccggtgaaggatcctctacaaataattttgtttaa

SEQ ID NO: 328 - DNA, 59 bp, synthetic construct
  misc_feature 1..59: note = synthetic stem loops buffer sequence
  source 1..59: mol_type = other DNA
attgatctggttattaaaggtaatcgggtcattttacctctacaaataattttgtttaa

SEQ ID NO: 329 - DNA, 64 bp, synthetic construct
  misc_feature 1..64: note = synthetic stem loops buffer sequence
  source 1..64: mol_type = other DNA
gttctccacgggtgggatgagcccctcgtggtggaaatgcgcctctacaaataattttgtttaa

SEQ ID NO: 330 - DNA, 50 bp, synthetic construct
  misc_feature 1..50: note = synthetic stem loops buffer sequence
  source 1..50: mol_type = other DNA
agcatgaggtaaagtgtcatgcaccaacctctacaaataattttgtttaa

SEQ ID NO: 331 - DNA, 61 bp, synthetic construct
  misc_feature 1..61: note = synthetic stem loops buffer sequence
  source 1..61: mol_type = other DNA
acgtcgacttatctcgagtgagatattgttgacggtaccctctacaaataattttgtttaa

SEQ ID NO: 332 - DNA, 60 bp, synthetic construct
  misc_feature 1..60: note = synthetic stem loops buffer sequence
  source 1..60: mol_type = other DNA
acgtcgacttatctcgagtgagataagttgacggtaccctctacaaataattttgtttaa

SEQ ID NO: 333 - DNA, 74 bp, synthetic construct
  misc_feature 1..74: note = synthetic stem loops buffer sequence
  source 1..74: mol_type = other DNA
acgtcgacttatctcgagactgcagttcaatagagatattgttgacggtaccctctacaaataattttgtttaa

SEQ ID NO: 334 - DNA, 75 bp, synthetic construct
  misc_feature 1..75: note = synthetic stem loops (ribozyme) buffer sequence
  source 1..75: mol_type = other DNA
gactgtcaccggatgtgctttccggtctgatgagtccgtgaggacgaaacagcctctacaaataattttgtttaa

SEQ ID NO: 335 - DNA, 72 bp, synthetic construct
  misc_feature 1..72: note = synthetic Ptac controller #1 promoter sequence, Ptac (SBa_00512 sequence
  source 1..72: mol_type = other DNA
tattctgaaatgagctgttgacaattaatcatcggctcgtataatgtgtggaattgtgagcggataacaatt

SEQ ID NO: 336 - DNA, 75 bp, synthetic construct
  misc_feature 1..75: note = synthetic controller #3 promoter sequence, Ptac plus OR1 and OR2 (SBa_000506) sequence
  source 1..75: mol_type = other DNA
tattaacaccgtgcgtgttgacagctatacctctggcggttataatgctagcggaattgtgagcggataacaatt

SEQ ID NO: 337 - DNA, 36 bp, synthetic construct
  misc_feature 1..36: note = synthetic randomized sequence
  modified_base 21..28: mod_base = OTHER; note = n = g, a, c or t
  source 1..36: mol_type = other DNA
cttgggcacgcgtccattaannaggannaattaagc

SEQ ID NO: 338 - DNA, 36 bp, synthetic construct
  misc_feature 1..36: note = synthetic randomized sequence
  modified_base 19..26: mod_base = OTHER; note = n = g, a, c or t
  source 1..36: mol_type = other DNA
tgggcacgcgtccattaannaggannaattattagc

SEQ ID NO: 339 - DNA, 36 bp, synthetic construct
  misc_feature 1..36: note = synthetic randomized sequence
  modified_base 23..30: mod_base = OTHER; note = n = g, a, c or t
  source 1..36: mol_type = other DNA
tacttgggcacgcgtccattaannaggannaatagc

SEQ ID NO: 340 - DNA, 36 bp, synthetic construct
  misc_feature 1..36: note = synthetic randomized sequence
  modified_base 21..28: mod_base = OTHER; note = n = g, a, c or t
  source 1..36: mol_type = other DNA
cttgggcacgcgtccattaanaaggagnaattaagc

SEQ ID NO: 341 - DNA, 36 bp, synthetic construct
  misc_feature 1..36: note = synthetic randomized sequence
  modified_base 20..29: mod_base = OTHER; note = n = g, a, c or t
  source 1..36: mol_type = other DNA
cttgggcacgcgtccattantaaggaggnattaagc

SEQ ID NO: 342 - DNA, 34 bp, synthetic construct; identical to SEQ ID NO: 37
  misc_feature 1..34: note = synthetic weak ribosome binding site (RBS) (SBa_000507)
  source 1..34: mol_type = other DNA

SEQ ID NO: 343 - DNA, 123 bp, synthetic construct
  misc_feature 1..123: note = synthetic N-terminal degradation tag (SBa_000509)
  source 1..123: mol_type = other DNA
ttgtttatcaagcctgcggatctccgcgaaattgtgacttttccgctatttagcgatcttgttcagtgtggctttccttcaccggcagcagattacgttgaacagcgcatcgatctgggtggc

SEQ ID NO: 344 - DNA, 41 bp, synthetic construct
  misc_feature 1..41: note = synthetic Enterobacteria phage T7 terminator seed sequence
  modified_base 3..16: mod_base = OTHER; note = n = g, a, c or t
  source 1..41: mol_type = other DNA
tannnaaccsswwssnsssstcwwwcgsssssswwssgttt

SEQ ID NO: 345 - skipped